European Patent Application EP 4 321 611 A1, published February 14, 2024. Title: CHIMERIC ANTIGEN RECEPTOR TARGETING ONCOLYTIC VIRUS-DERIVED PROTEIN, CELL EXPRESSING THE SAME, AND USE THEREOF. Applicant: BIONOXX INC. The sequence listing filed with the application follows.

SEQUENCE LISTING (1097 sequences)

SEQ ID NO: 1 - protein, 8 aa, Artificial Sequence
  H-CDR1 of A56-01A02
GGTFSSYA

SEQ ID NO: 2 - protein, 8 aa, Artificial Sequence
  H-CDR2 of A56-01A02
IIPIFGTA

SEQ ID NO: 3 - protein, 13 aa, Artificial Sequence
  H-CDR3 of A56-01A02
ARFVFGSGTYLDS

SEQ ID NO: 4 - protein, 11 aa, Artificial Sequence
  L-CDR1 of A56-01A02
QSLLYSNGNNY

SEQ ID NO: 5 - protein, 3 aa, Artificial Sequence
  L-CDR2 of A56-01A02
LGS

SEQ ID NO: 6 - protein, 9 aa, Artificial Sequence
  L-CDR3 of A56-01A02
MQALQTPLT

SEQ ID NO: 7 - DNA, 765 bp, Artificial Sequence
  SCFV of A56-01A02
cagatgcagctggtgcagtctggggctgaggtgaagaagcctgggtcctcggtgaaggtctcctgcaaggcttctggaggcaccttcagcagctatgctatcagctgggtgcgacaggcccctggacaagggcttgagtggatgggagggatcatccctatctttggtacagcaaactacgcacagaagttccagggcagagtcaccatgaccagggacacgtccacgagcacagtctacatggagctgagcagcctgaaatctgaggacacggccgtgtattactgtgcgagattcgtctttggttcggggacttatcttgactcctggggccagggaaccctggtcaccgtctcctcaggcctcgggggcctcggaggaggaggtagtggcggaggaggctccggtggatccagcggtgtgggttccgatattgtgatgacccagactccactctccctgcccgtcacccctggagagtcggcctccatctcctgcaggtctagtcagagcctcctgtatagtaatgggaacaactatttggattggtacctgcagaagccagggcagtccccacagctcctgatctatttgggttctaatcgggcctccggggtccctgacaggttcagtggcagtggatcaggcacagattttacactgaaaatcagcagagtggaggctgaggatgttggggtttattactgcatgcaagctctacaaactcctctcactttcggcggagggaccaaggtggatatcaaa

SEQ ID NO: 8 - protein, 120 aa, Artificial Sequence
  VH2 of A56-01A02
QMQLVQSGAEVKKPGSSVKVSCKASGGTFSSYAISWVRQAPGQGLEWMGGIIPIFGTANYAQKFQGRVTMTRDTSTSTVYMELSSLKSEDTAVYYCARFVFGSGTYLDSWGQGTLVTVSS

SEQ ID NO: 9 - protein, 112 aa, Artificial Sequence
  VL2 of A56-01A02
DIVMTQTPLSLPVTPGESASISCRSSQSLLYSNGNNYLDWYLQKPGQSPQLLIYLGSNRASGVPDRFSGSGSGTDFTLKISRVEAEDVGVYYCMQALQTPLTFGGGTKVDIK

SEQ ID NO: 10 - protein, 25 aa, Artificial Sequence
  H-FR1 of A56-01A02
QMQLVQSGAEVKKPGSSVKVSCKAS

SEQ ID NO: 11 - protein, 17 aa, Artificial Sequence
  H-FR2 of A56-01A02
ISWVRQAPGQGLEWMGG

SEQ ID NO: 12 - protein, 38 aa, Artificial Sequence
  H-FR3 of A56-01A02
NYAQKFQGRVTMTRDTSTSTVYMELSSLKSEDTAVYYC

SEQ ID NO: 13 - protein, 11 aa, Artificial Sequence
  H-FR4 of A56-01A02
WGQGTLVTVSS

SEQ ID NO: 14 - protein, 26 aa, Artificial Sequence
  L-FR1 of A56-01A02
DIVMTQTPLSLPVTPGESASISCRSS

SEQ ID NO: 15 - protein, 17 aa, Artificial Sequence
  L-FR2 of A56-01A02
LDWYLQKPGQSPQLLIY

SEQ ID NO: 16 - protein, 36 aa, Artificial Sequence
  L-FR3 of A56-01A02
IYLGSNRASGVPDRFSGSGSGTDFTLKISRVEAEDV

SEQ ID NO: 17 - protein, 10 aa, Artificial Sequence
  L-FR4 of A56-01A02
FGGGTKVDIK

SEQ ID NO: 18 - protein, 8 aa, Artificial Sequence
  H-CDR1 of A56-01A03
GYTFTPYY

SEQ ID NO: 19 - protein, 8 aa, Artificial Sequence
  H-CDR2 of A56-01A03
IIPLLGKA

SEQ ID NO: 20 - protein, 14 aa, Artificial Sequence
  H-CDR3 of A56-01A03
AREARGVNYYGMDV

SEQ ID NO: 21 - protein, 6 aa, Artificial Sequence
  L-CDR1 of A56-01A03
QGISHS

SEQ ID NO: 22 - protein, 3 aa, Artificial Sequence
  L-CDR2 of A56-01A03
VAS

SEQ ID NO: 23 - protein, 9 aa, Artificial Sequence
  L-CDR3 of A56-01A03
QQTNNFPYT

SEQ ID NO: 24 - DNA, 753 bp, Artificial Sequence
  SCFV of A56-01A03
caggtgcagctggtgcagtctggggctgaggttaggaagcctggggcctccgtgaagatttcctgcatggcatctggatacaccttcaccccctactatatccactgggtgcggcaggcccctggccaagggcttgagtggatgggagggatcatccctctccttggtaaagcgacctacgcacagaagttccagggcagaatcacggttaccgcggacgaatccacgagcacagcctacatggaactgagcagtctaagatctgaggacacggccgtgtattactgtgcgagagaagcccggggagttaactactacggtatggacgtctggggccaagggaccacggtcaccgtctcctcaggcctcgggggcctcggaggaggaggtagtggcggaggaggctccggtggatccagcggtgtgggttccgacatccagatgacccagtctccatcttctgtgtctgcatctgtgggagacagagtcaccatcagttgtcgggcgagtcaggggatcagccactcgttagcctggtatcagcagaaaccagggaaagcccctaaactcctgatcgatgttgcatccagattgcaaagtggggtcccgttaagattcagcggcagtggatctgggacagatttcactctcactatcaacagcctgcagcctgaagattctgcaacttattactgtcaacagactaacaatttcccgtacacttttggccaggggaccaagctggaaatcaaa

SEQ ID NO: 25 - protein, 121 aa, Artificial Sequence
  VH2 of A56-01A03
QVQLVQSGAEVRKPGASVKISCMASGYTFTPYYIHWVRQAPGQGLEWMGGIIPLLGKATYAQKFQGRITVTADESTSTAYMELSSLRSEDTAVYYCAREARGVNYYGMDVWGQGTTVTVSS

SEQ ID NO: 26 - protein, 107 aa, Artificial Sequence
  VL2 of A56-01A03
DIQMTQSPSSVSASVGDRVTISCRASQGISHSLAWYQQKPGKAPKLLIDVASRLQSGVPLRFSGSGSGTDFTLTINSLQPEDSATYYCQQTNNFPYTFGQGTKLEIK

SEQ ID NO: 27 - protein, 25 aa, Artificial Sequence
  H-FR1 of A56-01A03
QVQLVQSGAEVRKPGASVKISCMAS

SEQ ID NO: 28 - protein, 17 aa, Artificial Sequence
  H-FR2 of A56-01A03
IHWVRQAPGQGLEWMGG

SEQ ID NO: 29 - protein, 38 aa, Artificial Sequence
  H-FR3 of A56-01A03
TYAQKFQGRITVTADESTSTAYMELSSLRSEDTAVYYC

SEQ ID NO: 30 - protein, 11 aa, Artificial Sequence
  H-FR4 of A56-01A03
WGQGTTVTVSS

SEQ ID NO: 31 - protein, 26 aa, Artificial Sequence
  L-FR1 of A56-01A03
DIQMTQSPSSVSASVGDRVTISCRAS

SEQ ID NO: 32 - protein, 17 aa, Artificial Sequence
  L-FR2 of A56-01A03
LAWYQQKPGKAPKLLID

SEQ ID NO: 33 - protein, 36 aa, Artificial Sequence
  L-FR3 of A56-01A03
IDVASRLQSGVPLRFSGSGSGTDFTLTINSLQPEDS

SEQ ID NO: 34 - protein, 10 aa, Artificial Sequence
  L-FR4 of A56-01A03
FGQGTKLEIK

SEQ ID NO: 35 - protein, 8 aa, Artificial Sequence
  H-CDR1 of A56-01A04
GGTFSYRY

SEQ ID NO: 36 - protein, 8 aa, Artificial Sequence
  H-CDR2 of A56-01A04
ITPFNGYT

SEQ ID NO: 37 - protein, 11 aa, Artificial Sequence
  H-CDR3 of A56-01A04
VTGLGKTNLDS

SEQ ID NO: 38 - protein, 11 aa, Artificial Sequence
  L-CDR1 of A56-01A04
QSLVHSNGNTY

SEQ ID NO: 39 - protein, 3 aa, Artificial Sequence
  L-CDR2 of A56-01A04
QIS

SEQ ID NO: 40 - protein, 9 aa, Artificial Sequence
  L-CDR3 of A56-01A04
MQLTQFPLT

SEQ ID NO: 41 - DNA, 759 bp, Artificial Sequence
  SCFV of A56-01A04
caggtgcagctggtggagtctggggctgaggtgaagaagcctgggtcctcggtgaaggtctcctgcaaggcttctggaggcaccttcagttaccgctacctgcactgggtgcgacaggcctccggacaggcgcttgagtggatggggtggatcacacctttcaatggttacaccaactacgcacagaaattccaggacagagtcaccattaccagggacaggtctatgagcacagcctacatggagctgagcagcctgagatctgaggacacggccgtgtattactgtgtcacaggcctcggaaaaacgaaccttgactcctggggccagggaaccctggtcaccgtctcctcaggcctcgggggcctcggaggaggaggtagtggcggaggaggctccggtggatccagcggtgtgggttccgatattgtgatgacccagactccactctcctcacctgtcacccttggacagccggcctccatctcctgcaggtctagtcagagcctcgtacacagtaatggaaacacctacttgagttggcttcagcagaggccaggccagcctccaagactcctaatttatcagatttctaagcggttctctggggtcccagacagattcagtggcagtggggcagggacagatttcacactgaaaatcagcagggtggaagctgaggatgtcggggtttattactgcatgcaacttacacaatttcctctcactttcggcggagggaccaaggtggagatcaaa

SEQ ID NO: 42 - protein, 118 aa, Artificial Sequence
  VH2 of A56-01A04
QVQLVESGAEVKKPGSSVKVSCKASGGTFSYRYLHWVRQASGQALEWMGWITPFNGYTNYAQKFQDRVTITRDRSMSTAYMELSSLRSEDTAVYYCVTGLGKTNLDSWGQGTLVTVSS

SEQ ID NO: 43 - protein, 112 aa, Artificial Sequence
  VL2 of A56-01A04
DIVMTQTPLSSPVTLGQPASISCRSSQSLVHSNGNTYLSWLQQRPGQPPRLLIYQISKRFSGVPDRFSGSGAGTDFTLKISRVEAEDVGVYYCMQLTQFPLTFGGGTKVEIK

SEQ ID NO: 44 - protein, 25 aa, Artificial Sequence
  H-FR1 of A56-01A04
QVQLVESGAEVKKPGSSVKVSCKAS

SEQ ID NO: 45 - protein, 17 aa, Artificial Sequence
  H-FR2 of A56-01A04
LHWVRQASGQALEWMGW

SEQ ID NO: 46 - protein, 38 aa, Artificial Sequence
  H-FR3 of A56-01A04
NYAQKFQDRVTITRDRSMSTAYMELSSLRSEDTAVYYC

SEQ ID NO: 47 - protein, 11 aa, Artificial Sequence
  H-FR4 of A56-01A04
WGQGTLVTVSS

SEQ ID NO: 48 - protein, 26 aa, Artificial Sequence
  L-FR1 of A56-01A04
DIVMTQTPLSSPVTLGQPASISCRSS

SEQ ID NO: 49 - protein, 17 aa, Artificial Sequence
  L-FR2 of A56-01A04
LSWLQQRPGQPPRLLIY

SEQ ID NO: 50 - protein, 36 aa, Artificial Sequence
  L-FR3 of A56-01A04
IYQISKRFSGVPDRFSGSGAGTDFTLKISRVEAEDV

SEQ ID NO: 51 - protein, 10 aa, Artificial Sequence
  L-FR4 of A56-01A04
FGGGTKVEIK

SEQ ID NO: 52 - protein, 8 aa, Artificial Sequence
  H-CDR1 of A56-01A05
GDTLTYRF

SEQ ID NO: 53 - protein, 8 aa, Artificial Sequence
  H-CDR2 of A56-01A05
ITPFNGNT

SEQ ID NO: 54 - protein, 13 aa, Artificial Sequence
  H-CDR3 of A56-01A05
ATGGGNNYYGMEV

SEQ ID NO: 55 - protein, 6 aa, Artificial Sequence
  L-CDR1 of A56-01A05
QGIGSW

SEQ ID NO: 56 - protein, 3 aa, Artificial Sequence
  L-CDR2 of A56-01A05
GAS

SEQ ID NO: 57 - protein, 9 aa, Artificial Sequence
  L-CDR3 of A56-01A05
QKANNFPYT

SEQ ID NO: 58 - DNA, 750 bp, Artificial Sequence
  SCFV of A56-01A05
caggtgcagctggtacagtctggggctgaggtgaagaagactgggtcctcagtgaaggtttcgtgcaaggcttccggagacacccttacctaccgcttcctgcactgggtgcgacaggcccccggacaagcgcctgagtggattggatggatcacacctttcaatggtaacaccaactacgcacagaaattccaggacagagtcaccattaccagggacaggtctatgagcacagcctacatggagctgagcagcctgagatctgaggacacggccgtgtattactgtgcgactggaggtgggaacaattattacggcatggaggtctggggccaagggaccccgatcaccgtctcctcaggcctcgggggcctcggaggaggaggtagtggcggaggaggctccggtggatccagcggtgtgggttccgacatccagatgacccagtctccatcttccgtgtctgcatctgtaggagacagagtcaccatcacttgtcgggcgagtcagggtattggcagctggttagcctggtatcagcagaaaccaggggaagcccctaacctcctgatctatggtgcatccaatttggcaagtggggtcccatcaaggttcagtggcggtggatctgggacagatttcagtctcaccatcagcagcctgcagcctgaagattttgcaacttactattgtcaaaaggcaaataatttcccgtacacttttggccaggggaccaagctggatatcaaa

SEQ ID NO: 59 - protein, 120 aa, Artificial Sequence
  VH2 of A56-01A05
QVQLVQSGAEVKKTGSSVKVSCKASGDTLTYRFLHWVRQAPGQAPEWIGWITPFNGNTNYAQKFQDRVTITRDRSMSTAYMELSSLRSEDTAVYYCATGGGNNYYGMEVWGQGTPITVSS

SEQ ID NO: 60 - protein, 107 aa, Artificial Sequence
  VL2 of A56-01A05
DIQMTQSPSSVSASVGDRVTITCRASQGIGSWLAWYQQKPGEAPNLLIYGASNLASGVPSRFSGGGSGTDFSLTISSLQPEDFATYYCQKANNFPYTFGQGTKLDIK

SEQ ID NO: 61 - protein, 25 aa, Artificial Sequence
  H-FR1 of A56-01A05
QVQLVQSGAEVKKTGSSVKVSCKAS

SEQ ID NO: 62 - protein, 17 aa, Artificial Sequence
  H-FR2 of A56-01A05
LHWVRQAPGQAPEWIGW

SEQ ID NO: 63 - protein, 38 aa, Artificial Sequence; identical to SEQ ID NO: 46
  H-FR3 of A56-01A05

SEQ ID NO: 64 - protein, 11 aa, Artificial Sequence
  H-FR4 of A56-01A05
WGQGTPITVSS

SEQ ID NO: 65 - protein, 26 aa, Artificial Sequence [sequence omitted]

SEQ ID NO: 66 - protein, 17 aa, Artificial Sequence
  L-FR2 of A56-01A05
LAWYQQKPGEAPNLLIY

SEQ ID NO: 67 - protein, 36 aa, Artificial Sequence
  L-FR3 of A56-01A05
IYGASNLASGVPSRFSGGGSGTDFSLTISSLQPEDF

SEQ ID NO: 68 - protein, 10 aa, Artificial Sequence
  L-FR4 of A56-01A05
FGQGTKLDIK

SEQ ID NO: 69 - protein, 8 aa, Artificial Sequence
  H-CDR1 of A56-01B01
GFTISNYA

SEQ ID NO: 70 - protein, 8 aa, Artificial Sequence
  H-CDR2 of A56-01B01
VSGSGVTT

SEQ ID NO: 71 - protein, 8 aa, Artificial Sequence
  H-CDR3 of A56-01B01
VRMTGGPL

SEQ ID NO: 72 - protein, 6 aa, Artificial Sequence
  L-CDR1 of A56-01B01
QGVRND

SEQ ID NO: 73 - protein, 3 aa, Artificial Sequence
  L-CDR2 of A56-01B01
GAS

SEQ ID NO: 74 - protein, 9 aa, Artificial Sequence
  L-CDR3 of A56-01B01
LQDFIYPYT

SEQ ID NO: 75 - DNA, 735 bp, Artificial Sequence
  SCFV of A56-01B01
cagatgcagctggtggagtctgggggaggcttggtccagcctggggggtccctgagactctcctgtacagcctctggattcaccattagcaactacgccatgagctgggtccgccaggctccagggaaggggctggagtgggtcgcaactgttagtggtagtggtgttaccacacactacgcagcctccgtgaaggaccggttcaccgtctccagtgacagttccaagaacacactttttctgcaaatgaacagtctgagagccgaggacacggccgtgtattactgtgtaaggatgactgggggcccactttggggccagggaaccctgatcaccgtctcctcaggcctcgggggcctcggaggaggaggtagtggcggaggaggctccggtggatccagcggtgtgggttccgacatccagatgacccagtctccatcctccctgtctgcatctgtaggagacagagtcaccatcacttgccgggcaagtcagggcgttagaaatgatttaggctggtatcagcagaaaccagggaaagccccgaagctcctgatctatggtgcatccactttacaaagtggggtcccatcaaggttcagcggcagtggatctggcacagatttcactctcaccatcagcagtctgcagcctgaagattttgcaacttattactgtctacaagatttcatttacccgtacacttttggccaggggaccaagctggagatcaaa

SEQ ID NO: 76 - protein, 115 aa, Artificial Sequence
  VH2 of A56-01B01
QMQLVESGGGLVQPGGSLRLSCTASGFTISNYAMSWVRQAPGKGLEWVATVSGSGVTTHYAASVKDRFTVSSDSSKNTLFLQMNSLRAEDTAVYYCVRMTGGPLWGQGTLITVSS

SEQ ID NO: 77 - protein, 107 aa, Artificial Sequence
  VL2 of A56-01B01
DIQMTQSPSSLSASVGDRVTITCRASQGVRNDLGWYQQKPGKAPKLLIYGASTLQSGVPSRFSGSGSGTDFTLTISSLQPEDFATYYCLQDFIYPYTFGQGTKLEIK

SEQ ID NO: 78 - protein, 25 aa, Artificial Sequence
  H-FR1 of A56-01B01
QMQLVESGGGLVQPGGSLRLSCTAS

SEQ ID NO: 79 - protein, 17 aa, Artificial Sequence
  H-FR2 of A56-01B01
MSWVRQAPGKGLEWVAT

SEQ ID NO: 80 - protein, 38 aa, Artificial Sequence
  H-FR3 of A56-01B01
HYAASVKDRFTVSSDSSKNTLFLQMNSLRAEDTAVYYC

SEQ ID NO: 81 - protein, 11 aa, Artificial Sequence
  H-FR4 of A56-01B01
WGQGTLITVSS

SEQ ID NO: 82 - protein, 26 aa, Artificial Sequence [sequence omitted]

SEQ ID NO: 83 - protein, 17 aa, Artificial Sequence
  L-FR2 of A56-01B01
LGWYQQKPGKAPKLLIY

SEQ ID NO: 84 - protein, 36 aa, Artificial Sequence
  L-FR3 of A56-01B01
IYGASTLQSGVPSRFSGSGSGTDFTLTISSLQPEDF

SEQ ID NO: 85 - protein, 10 aa, Artificial Sequence
  L-FR4 of A56-01B01
FGQGTKLEIK

SEQ ID NO: 86 - protein, 8 aa, Artificial Sequence
  H-CDR1 of A56-01C08
GFTFSNNW

SEQ ID NO: 87 - protein, 8 aa, Artificial Sequence
  H-CDR2 of A56-01C08
INRDGSER

SEQ ID NO: 88 - protein, 21 aa, Artificial Sequence
  H-CDR3 of A56-01C08
VRDSLIIYDNSWYPYYHGMAV

SEQ ID NO: 89 - protein, 6 aa, Artificial Sequence
  L-CDR1 of A56-01C08
SLRKYH

SEQ ID NO: 90 - protein, 3 aa, Artificial Sequence
  L-CDR2 of A56-01C08
GKN

SEQ ID NO: 91 - protein, 11 aa, Artificial Sequence
  L-CDR3 of A56-01C08
NSRDSSPNHLV

SEQ ID NO: 92 - DNA, 777 bp, Artificial Sequence
  SCFV of A56-01C08
caggtgcagctggtagagtctgggggacggttggtccagcctgggggatccctgagactctcctgcgtaacttctggattcacttttagtaacaattggatgacttgggtccgccaggctccagggaaggggctggagtgggtggccaccataaaccgagatggaagtgagaggtattatgtggactctgtgaaggaccggttcaccatctccagagaaaacagcaaaaactccctgtatctgcaaatgaacagtctgagagccgaggacacggccgtgtattactgtgtgagagacagtctaataatatacgataatagttggtatccctattaccacggtatggccgtctggggccaagggaccacggtcaccgtctcctcaggcctcgggggcctcggaggaggaggtagtggcggaggaggctccggtggatccagcggtgtgggttcctcctatgagctgacacaggaccctgctgtgtctgtggccttgggacagacagtcaggatcacatgccaaggagacagcctcagaaaatatcatgcaagctggtaccagcagaagccaggacaggcccctgtacttgtcatctatggtaaaaacaaccggccctcagggatcccaggccgattctctggctccagctcaggaaacacagcttccttgaccatcactgaagctcaggcggaagatgaggctgactattactgtaactcccgggacagcagtcctaaccatctggttttcggcggagggaccaagctgaccgtccta

SEQ ID NO: 93 - protein, 128 aa, Artificial Sequence
  VH2 of A56-01C08
QVQLVESGGRLVQPGGSLRLSCVTSGFTFSNNWMTWVRQAPGKGLEWVATINRDGSERYYVDSVKDRFTISRENSKNSLYLQMNSLRAEDTAVYYCVRDSLIIYDNSWYPYYHGMAVWGQGTTVTVSS

SEQ ID NO: 94 - protein, 108 aa, Artificial Sequence
  VL2 of A56-01C08
SYELTQDPAVSVALGQTVRITCQGDSLRKYHASWYQQKPGQAPVLVIYGKNNRPSGIPGRFSGSSSGNTASLTITEAQAEDEADYYCNSRDSSPNHLVFGGGTKLTVL

SEQ ID NO: 95 - protein, 25 aa, Artificial Sequence
  H-FR1 of A56-01C08
QVQLVESGGRLVQPGGSLRLSCVTS

SEQ ID NO: 96 - protein, 17 aa, Artificial Sequence
  H-FR2 of A56-01C08
MTWVRQAPGKGLEWVAT

SEQ ID NO: 97 - protein, 38 aa, Artificial Sequence
  H-FR3 of A56-01C08
YYVDSVKDRFTISRENSKNSLYLQMNSLRAEDTAVYYC

SEQ ID NO: 98 - protein, 11 aa, Artificial Sequence
  H-FR4 of A56-01C08
WGQGTTVTVSS

SEQ ID NO: 99 - protein, 25 aa, Artificial Sequence
  L-FR1 of A56-01C08
SYELTQDPAVSVALGQTVRITCQGD

SEQ ID NO: 100 - protein, 17 aa, Artificial Sequence
  L-FR2 of A56-01C08
ASWYQQKPGQAPVLVIY

SEQ ID NO: 101 - protein, 36 aa, Artificial Sequence
  L-FR3 of A56-01C08
IYGKNNRPSGIPGRFSGSSSGNTASLTITEAQAEDE

SEQ ID NO: 102 - protein, 10 aa, Artificial Sequence
  L-FR4 of A56-01C08
FGGGTKLTVL

SEQ ID NO: 103 - protein, 8 aa, Artificial Sequence
  H-CDR1 of A56-01C12
GFRSSTFW

SEQ ID NO: 104 - protein, 8 aa, Artificial Sequence
  H-CDR2 of A56-01C12
IKQDGSEI

SEQ ID NO: 105 - protein, 17 aa, Artificial Sequence
  H-CDR3 of A56-01C12
ARTRGATIYDHYYGMDV

SEQ ID NO: 106 - protein, 8 aa, Artificial Sequence
  L-CDR1 of A56-01C12
SSNIGSYS

SEQ ID NO: 107 - protein, 3 aa, Artificial Sequence
  L-CDR2 of A56-01C12
GHN

SEQ ID NO: 108 - protein, 11 aa, Artificial Sequence
  L-CDR3 of A56-01C12
AAWDDSVDGWV

SEQ ID NO: 109 - DNA, 771 bp, Artificial Sequence
  SCFV of A56-01C12
caggtgcagctggtggagtctgggggaggcttggtccagcctggggggtccctgagactctcctgtgtagcctctggattcaggtctagtactttttggatgagttggatccgccaggctccagggaaggggctggagtgggtggcccacataaagcaagatggaagtgagatatactatgtggactctgtgaagggccgattcaccatctccagagacaacagcaaaaactccctgtatctgcaaatgaacagtctgagagccgaggacacggccgtgtattactgtgcgagaacgaggggggctacgatttacgaccactactatggtatggacgtctggggccaagggaccgcggtcaccgtctcctcaggcctcgggggcctcggaggaggaggtagtggcggaggaggctccggtggatccagcggtgtgggttcccagtctgccctgactcagcctccctcaaggtctgtgacccccgggcagagggtcaccatttcttgttctggaagcagctcaaatatcggaagttactctgtaaattggtaccagcaactcccaggaacggcccccaagctcctcatctacgggcataatcagcggccctcaggggtccctgaccgattctctggctccaagtctggcacctcagcctccctggccatcagtgggctccagtctgcggatgagggtgattattactgtgcagcatgggatgacagtgtggatggttgggtgttcggcggagggaccaagctgaccgtccta

SEQ ID NO: 110 - protein, 124 aa, Artificial Sequence
  VH2 of A56-01C12
QVQLVESGGGLVQPGGSLRLSCVASGFRSSTFWMSWIRQAPGKGLEWVAHIKQDGSEIYYVDSVKGRFTISRDNSKNSLYLQMNSLRAEDTAVYYCARTRGATIYDHYYGMDVWGQGTAVTVSS

SEQ ID NO: 111 - protein, 110 aa, Artificial Sequence
  VL2 of A56-01C12
QSALTQPPSRSVTPGQRVTISCSGSSSNIGSYSVNWYQQLPGTAPKLLIYGHNQRPSGVPDRFSGSKSGTSASLAISGLQSADEGDYYCAAWDDSVDGWVFGGGTKLTVL

SEQ ID NO: 112 - protein, 25 aa, Artificial Sequence
  H-FR1 of A56-01C12
QVQLVESGGGLVQPGGSLRLSCVAS

SEQ ID NO: 113 - protein, 17 aa, Artificial Sequence
  H-FR2 of A56-01C12
MSWIRQAPGKGLEWVAH

SEQ ID NO: 114 - protein, 38 aa, Artificial Sequence
  H-FR3 of A56-01C12
YYVDSVKGRFTISRDNSKNSLYLQMNSLRAEDTAVYYC

SEQ ID NO: 115 - protein, 11 aa, Artificial Sequence
  H-FR4 of A56-01C12
WGQGTAVTVSS

SEQ ID NO: 116 - protein, 25 aa, Artificial Sequence
  L-FR1 of A56-01C12
QSALTQPPSRSVTPGQRVTISCSGS

SEQ ID NO: 117 - protein, 17 aa, Artificial Sequence
  L-FR2 of A56-01C12
VNWYQQLPGTAPKLLIY

SEQ ID NO: 118 - protein, 36 aa, Artificial Sequence
  L-FR3 of A56-01C12
IYGHNQRPSGVPDRFSGSKSGTSASLAISGLQSADE

SEQ ID NO: 119 - protein, 10 aa, Artificial Sequence
  L-FR4 of A56-01C12
FGGGTKLTVL

SEQ ID NO: 120 - protein, 8 aa, Artificial Sequence
  H-CDR1 of A56-01F12
GGSFSTYA

SEQ ID NO: 121 - protein, 8 aa, Artificial Sequence
  H-CDR2 of A56-01F12
IIPISDIR

SEQ ID NO: 122 - protein, 13 aa, Artificial Sequence
  H-CDR3 of A56-01F12
AKGGRLLSTHFDY

SEQ ID NO: 123 - protein, 8 aa, Artificial Sequence
  L-CDR1 of A56-01F12
SSNIGNNY

SEQ ID NO: 124 - protein, 3 aa, Artificial Sequence
  L-CDR2 of A56-01F12
DDD

SEQ ID NO: 125 - protein, 12 aa, Artificial Sequence
  L-CDR3 of A56-01F12
GTWHSGLSAGVV

SEQ ID NO: 126 - DNA, 763 bp, Artificial Sequence
  SCFV of A56-01F12
caggtgcagctggtggagtctgggggtgaggtgaagaagcctgggtcctcggtgaaggtctcctgcaaggcttctggaggcagcttcagcacctatgctatcagctgggtgcgacaggcccctggacaagggcttgagtggatgggaaggatcatccccatctctgatatcagaaactacgcacagaaattccagggcagagtcacgttaaccgcggacagagccacgagcacagcctacatggagctgagcagcctgagatctgaggacacggccgtgtattactgtgcgaaagggggacgactgctatctactcactttgactactggggccagggaaccctggtcaccgtctcctcaggcctcgggggcctcggaggaggaggtagtggcggaggaggctccggtggatccagcggtgtgggttcccagctcgtgctgactcagccgccctcagtgtctgcggcccccggacagaaggtcaccatctcctgctctggaagcagctccaacattgggaataattatgtatcctggtaccagcaactcccaggaacagcccccaaactcctcatttatgacgatgataagcgaccctcagggattcctgaccgattctctggctccaagtctggcacgtcagccaccctgggcatcaccggactccagactggggacgaggccgattattactgcggaacatggcatagcggcctgagtgctggcgtggttttcggcggagggaccaagctgaccgtcctaa

SEQ ID NO: 127 - protein, 120 aa, Artificial Sequence
  VH2 of A56-01F12
QVQLVESGGEVKKPGSSVKVSCKASGGSFSTYAISWVRQAPGQGLEWMGRIIPISDIRNYAQKFQGRVTLTADRATSTAYMELSSLRSEDTAVYYCAKGGRLLSTHFDYWGQGTLVTVSS

SEQ ID NO: 128 - protein, 111 aa, Artificial Sequence
  VL2 of A56-01F12
QLVLTQPPSVSAAPGQKVTISCSGSSSNIGNNYVSWYQQLPGTAPKLLIYDDDKRPSGIPDRFSGSKSGTSATLGITGLQTGDEADYYCGTWHSGLSAGVVFGGGTKLTVL

SEQ ID NO: 129 - protein, 25 aa, Artificial Sequence
  H-FR1 of A56-01F12
QVQLVESGGEVKKPGSSVKVSCKAS

SEQ ID NO: 130 - protein, 17 aa, Artificial Sequence
  H-FR2 of A56-01F12
ISWVRQAPGQGLEWMGR

SEQ ID NO: 131 - protein, 38 aa, Artificial Sequence
  H-FR3 of A56-01F12
NYAQKFQGRVTLTADRATSTAYMELSSLRSEDTAVYYC

SEQ ID NO: 132 - protein, 11 aa, Artificial Sequence
  H-FR4 of A56-01F12
WGQGTLVTVSS

SEQ ID NO: 133 - protein, 25 aa, Artificial Sequence
  L-FR1 of A56-01F12
QLVLTQPPSVSAAPGQKVTISCSGS

SEQ ID NO: 134 - protein, 17 aa, Artificial Sequence
  L-FR2 of A56-01F12
VSWYQQLPGTAPKLLIY

SEQ ID NO: 135 - protein, 36 aa, Artificial Sequence
  L-FR3 of A56-01F12
IYDDDKRPSGIPDRFSGSKSGTSATLGITGLQTGDE

SEQ ID NO: 136 - protein, 10 aa, Artificial Sequence
  L-FR4 of A56-01F12
FGGGTKLTVL

SEQ ID NO: 137 - protein, 8 aa, Artificial Sequence
  H-CDR1 of A56-01G06
GGTLSSYP

SEQ ID NO: 138 - protein, 8 aa, Artificial Sequence
  H-CDR2 of A56-01G06
IIPIVGRA

SEQ ID NO: 139 - protein, 15 aa, Artificial Sequence
  H-CDR3 of A56-01G06
ARENPSSYAPFALDI

SEQ ID NO: 140 - protein, 9 aa, Artificial Sequence
  L-CDR1 of A56-01G06
SSDVGGYNY

SEQ ID NO: 141 - protein, 3 aa, Artificial Sequence
  L-CDR2 of A56-01G06
DVT

SEQ ID NO: 142 - protein, 10 aa, Artificial Sequence
  L-CDR3 of A56-01G06
SSYSSSTFYV

SEQ ID NO: 143 - DNA, 766 bp, Artificial Sequence
  SCFV of A56-01G06
caggtgcagctggtacagtctggggctgaagtgaagaagcctgggtcctcggtgaaggtctcgtgcaaggcttctggaggcaccctcagcagctatcccatcagctgggtgcgacaggcccctggacaagggcttgagtggatgggaaggatcattcctattgttggtagagcaaactacgcacagaagttccagggcagagtcacgattaacgcggacacatccacgaacacagtccacatggagttgagtagcctgagatctgaggacacggccgtgtattactgcgcgagagagaacccctccagttatgctccctttgctcttgatatctggggccaagggacagcggtcaccgtctcctcaggcctcgggggcctcggaggaggaggtagtggcggaggaggctccggtggatccagcggtgtgggttccaattttatgctgactcagcccgcctccgtgtctgggtcccctggacagtcgatcaccatctcctgcactggaagcagcagcgacgttggtggttataactatgtctcctggtaccaacagcaccaaggcaaagccccccaactcatcatttatgatgtcactaagcggccctcaggggtttctaatcgcttctccggctccaagtctggcaactcggcctccctgaccatctctggactccaggctgaggacgaggctgattattactgcagctcatacagcagcagcactttttacgtcttcggaactgggaccaaggtcaccgtcctaa

SEQ ID NO: 144 - protein, 122 aa, Artificial Sequence
  VH2 of A56-01G06
QVQLVQSGAEVKKPGSSVKVSCKASGGTLSSYPISWVRQAPGQGLEWMGRIIPIVGRANYAQKFQGRVTINADTSTNTVHMELSSLRSEDTAVYYCARENPSSYAPFALDIWGQGTAVTVSS

SEQ ID NO: 145 - protein, 110 aa, Artificial Sequence
  VL2 of A56-01G06
NFMLTQPASVSGSPGQSITISCTGSSSDVGGYNYVSWYQQHQGKAPQLIIYDVTKRPSGVSNRFSGSKSGNSASLTISGLQAEDEADYYCSSYSSSTFYVFGTGTKVTVL

SEQ ID NO: 146 - protein, 25 aa, Artificial Sequence [sequence omitted]

SEQ ID NO: 147 - protein, 17 aa, Artificial Sequence
  H-FR2 of A56-01G06
ISWVRQAPGQGLEWMGR

SEQ ID NO: 148 - protein, 38 aa, Artificial Sequence
  H-FR3 of A56-01G06
NYAQKFQGRVTINADTSTNTVHMELSSLRSEDTAVYYC

SEQ ID NO: 149 - protein, 11 aa, Artificial Sequence
  H-FR4 of A56-01G06
WGQGTAVTVSS

SEQ ID NO: 150 - protein, 25 aa, Artificial Sequence
  L-FR1 of A56-01G06
NFMLTQPASVSGSPGQSITISCTGS

SEQ ID NO: 151 - protein, 17 aa, Artificial Sequence
  L-FR2 of A56-01G06
VSWYQQHQGKAPQLIIY

SEQ ID NO: 152 - protein, 36 aa, Artificial Sequence
  L-FR3 of A56-01G06
IYDVTKRPSGVSNRFSGSKSGNSASLTISGLQAEDE

SEQ ID NO: 153 - protein, 10 aa, Artificial Sequence
  L-FR4 of A56-01G06
FGTGTKVTVL

SEQ ID NO: 154 - protein, 8 aa, Artificial Sequence
  H-CDR1 of A56-01G11
GFNFDDHA

SEQ ID NO: 155 - protein, 8 aa, Artificial Sequence
  H-CDR2 of A56-01G11
ISWNGRSI

SEQ ID NO: 156 - protein, 18 aa, Artificial Sequence
  H-CDR3 of A56-01G11
ARDLAHASGSLRRPFFDY

SEQ ID NO: 157 - protein, 6 aa, Artificial Sequence
  L-CDR1 of A56-01G11
QDISTY

SEQ ID NO: 158 - protein, 3 aa, Artificial Sequence
  L-CDR2 of A56-01G11
STS

SEQ ID NO: 159 - protein, 10 aa, Artificial Sequence
  L-CDR3 of A56-01G11
QQLKSYPRFT

SEQ ID NO: 160 - DNA, 768 bp, Artificial Sequence
  SCFV of A56-01G11
caggtgcagctggtggagtctggaggaggcttgatccagcctggggggtccctgagactctcctgtgcagcctccggattcaactttgatgatcatgccatgcactgggtccggcaagctccagggaagggcctggagtgggtctccggtattagttggaatggacgtagcatatactatgcggactctgtgaggggccgattcaccatctccagagacaacgccaggaactccctgcatctgcaaatgaacagtctgagagccgaggacacggccgtgtattactgtgcgagagatttggcccatgcctcggggagtcttaggcgacctttttttgactactggggccagggaaccctggtcaccgtctcctcaggcctcgggggcctcggaggaggaggtagtggcggaggaggctccggtggatccagcggtgtgggttccgacatccagatgacccagtctccatccttcctgtctgcatctgtaggagacagagtcaccatcacttgccgggcaagtcaggacattagcacctatttaaattggtatcagcagaaaccagggaaagcccctaagctcctgatctattctacatccactttggaaagtggggtcccatcgcgattcagcggcagtggatctgggacaaatttcactctcacaatcaacaacctgcagcctgaagattttgcaacttattactgtcaacaacttaagagttaccctcgattcactttcggccctgggaccaaagtggatatcaaa

SEQ ID NO: 161 - protein, 125 aa, Artificial Sequence
  VH2 of A56-01G11
QVQLVESGGGLIQPGGSLRLSCAASGFNFDDHAMHWVRQAPGKGLEWVSGISWNGRSIYYADSVRGRFTISRDNARNSLHLQMNSLRAEDTAVYYCARDLAHASGSLRRPFFDYWGQGTLVTVSS

SEQ ID NO: 162 - protein, 108 aa, Artificial Sequence
  VL2 of A56-01G11
DIQMTQSPSFLSASVGDRVTITCRASQDISTYLNWYQQKPGKAPKLLIYSTSTLESGVPSRFSGSGSGTNFTLTINNLQPEDFATYYCQQLKSYPRFTFGPGTKVDIK

SEQ ID NO: 163 - protein, 25 aa, Artificial Sequence
  H-FR1 of A56-01G11
QVQLVESGGGLIQPGGSLRLSCAAS

SEQ ID NO: 164 - protein, 17 aa, Artificial Sequence
  H-FR2 of A56-01G11
MHWVRQAPGKGLEWVSG

SEQ ID NO: 165 - protein, 38 aa, Artificial Sequence
  H-FR3 of A56-01G11
YYADSVRGRFTISRDNARNSLHLQMNSLRAEDTAVYYC

SEQ ID NO: 166 - protein, 11 aa, Artificial Sequence
  H-FR4 of A56-01G11
WGQGTLVTVSS

SEQ ID NO: 167 - protein, 26 aa, Artificial Sequence
  L-FR1 of A56-01G11
DIQMTQSPSFLSASVGDRVTITCRAS

SEQ ID NO: 168 - protein, 17 aa, Artificial Sequence
  L-FR2 of A56-01G11
LNWYQQKPGKAPKLLIY

SEQ ID NO: 169 - protein, 36 aa, Artificial Sequence
  L-FR3 of A56-01G11
IYSTSTLESGVPSRFSGSGSGTNFTLTINNLQPEDF

SEQ ID NO: 170 - protein, 10 aa, Artificial Sequence
  L-FR4 of A56-01G11
FGPGTKVDIK

SEQ ID NO: 171 - protein, 8 aa, Artificial Sequence
  H-CDR1 of A56-01H01
GFKFEDHA

SEQ ID NO: 172 - protein, 8 aa, Artificial Sequence
  H-CDR2 of A56-01H01
ISGNGDDT

SEQ ID NO: 173 - protein, 7 aa, Artificial Sequence
  H-CDR3 of A56-01H01
ARDRGPG

SEQ ID NO: 174 - protein, 12 aa, Artificial Sequence
  L-CDR1 of A56-01H01
QSVLSSSNNKNY

SEQ ID NO: 175 - protein, 3 aa, Artificial Sequence
  L-CDR2 of A56-01H01
WAS

SEQ ID NO: 176 - protein, 9 aa, Artificial Sequence
  L-CDR3 of A56-01H01
QQYYSTPST

SEQ ID NO: 177 - DNA, 750 bp, Artificial Sequence
  SCFV of A56-01H01
caggtgcagctggtggagtctgggggaggcgtggtacagcctggggggtccctgagactcacctgtgtgggctctggattcaagttcgaagatcacgccatccactgggtccgtcaacgtccagggaagggtctggagtgggtctccgttataagtggcaatggcgatgacacatactatgcagattctgcgaagggccgattcaccatttccagagacaacagcaaaaactccctgtatctgcaaatgaacagtctgagagccgaggacacggccgtgtattactgtgcgagagataggggccctggcctgggccagggaaccctggtcaccgtctcctcaggcctcgggggcctcggaggaggaggtagtggcggaggaggctccggtggatccagcggtgtgggttccgacatccagatgacccagtctccatcctccctggctgtgtctctgggcgagagggccaccatcaactgcaagtccagccagagtgttttatccagctccaacaataagaactacttagcttggtaccagcagagaccaggacagtctcctaagctgctcatttactgggcatctacccgggaatccggggtccctgaccgattcagtggcagcgggtctgggacagatttcactctcaccatcaacagcctgcaggctgaagatgtggcggtttattactgtcagcaatattatagtactccctctacgttcggccaagggaccaaggtggagatcaaa

SEQ ID NO: 178 - protein, 114 aa, Artificial Sequence
  VH2 of A56-01H01
QVQLVESGGGVVQPGGSLRLTCVGSGFKFEDHAIHWVRQRPGKGLEWVSVISGNGDDTYYADSAKGRFTISRDNSKNSLYLQMNSLRAEDTAVYYCARDRGPGLGQGTLVTVSS

SEQ ID NO: 179 - protein, 113 aa, Artificial Sequence
  VL2 of A56-01H01
DIQMTQSPSSLAVSLGERATINCKSSQSVLSSSNNKNYLAWYQQRPGQSPKLLIYWASTRESGVPDRFSGSGSGTDFTLTINSLQAEDVAVYYCQQYYSTPSTFGQGTKVEIK

SEQ ID NO: 180 - protein, 25 aa, Artificial Sequence
  H-FR1 of A56-01H01
QVQLVESGGGVVQPGGSLRLTCVGS

SEQ ID NO: 181 - protein, 17 aa, Artificial Sequence
  H-FR2 of A56-01H01
IHWVRQRPGKGLEWVSV

SEQ ID NO: 182 - protein, 38 aa, Artificial Sequence
  H-FR3 of A56-01H01
YYADSAKGRFTISRDNSKNSLYLQMNSLRAEDTAVYYC

SEQ ID NO: 183 - protein, 11 aa, Artificial Sequence
  H-FR4 of A56-01H01
LGQGTLVTVSS

SEQ ID NO: 184 - protein, 26 aa, Artificial Sequence
  L-FR1 of A56-01H01
DIQMTQSPSSLAVSLGERATINCKSS

SEQ ID NO: 185 - protein, 17 aa, Artificial Sequence
  L-FR2 of A56-01H01
LAWYQQRPGQSPKLLIY

SEQ ID NO: 186 - protein, 36 aa, Artificial Sequence
  L-FR3 of A56-01H01
IYWASTRESGVPDRFSGSGSGTDFTLTINSLQAEDV

SEQ ID NO: 187 - protein, 10 aa, Artificial Sequence
  L-FR4 of A56-01H01
FGQGTKVEIK

SEQ ID NO: 188 - protein, 8 aa, Artificial Sequence
  H-CDR1 of A56-01H02
GFTFGDYA

SEQ ID NO: 189 - protein, 10 aa, Artificial Sequence
  H-CDR2 of A56-01H02
IRSKAYGGTT

SEQ ID NO: 190 - protein, 15 aa, Artificial Sequence
  H-CDR3 of A56-01H02
ARDPAKERSRNWFAP

SEQ ID NO: 191 - protein, 6 aa, Artificial Sequence
  L-CDR1 of A56-01H02
QSIGSW

SEQ ID NO: 192 - protein, 3 aa, Artificial Sequence
  L-CDR2 of A56-01H02
KAS

SEQ ID NO: 193 - protein, 9 aa, Artificial Sequence
  L-CDR3 of A56-01H02
QQYKLYPWT

SEQ ID NO: 194 - DNA, 762 bp, Artificial Sequence
  SCFV of A56-01H02
caggtgcagctggtgcagtctgggggaggcttggtaaagccagggcggtccctgagactctcctgtacagcttctggattcacctttggtgattatgctatgagctggttccgccaggctccagggaaggggctggagtgggtaggtttcattagaagcaaagcttatggtgggacaacagaatacgccgcgtctgtgaaaggcagattcaccatctcaagagatgattccaaaagcatcgcctatctgcaaatgaacagtctgagagccgaggacacggccgtgtattactgtgcgagagatcctgcgaaagagcgaagtcgcaactggttcgccccctggggccagggaaccctggtcaccgtctcctcaggcctcgggggcctcggaggaggaggtagtggcggaggaggctccggtggatccagcggtgtgggttccgacatccagatgacccagtctccttccaccctgtctgcttctgtaggcgacagagtcaccatcacttgccgggccagccagagtattggtagttggttggcctggtatcagcagaaaccagggaaagcccctaagctcctgatctacaaggcgtctagtttagagagtggggtcccatcaaggttcagcggcagtggatctgggacagaattcactctcaccatcagcagcctgcagcctgatgattttgcaacttattactgccaacagtataaactatatccgtggacgttcggccaagggaccaaggtggatatcaaa

SEQ ID NO: 195 - protein, 124 aa, Artificial Sequence
  VH2 of A56-01H02
QVQLVQSGGGLVKPGRSLRLSCTASGFTFGDYAMSWFRQAPGKGLEWVGFIRSKAYGGTTEYAASVKGRFTISRDDSKSIAYLQMNSLRAEDTAVYYCARDPAKERSRNWFAPWGQGTLVTVSS

SEQ ID NO: 196 - protein, 107 aa, Artificial Sequence
  VL2 of A56-01H02
DIQMTQSPSTLSASVGDRVTITCRASQSIGSWLAWYQQKPGKAPKLLIYKASSLESGVPSRFSGSGSGTEFTLTISSLQPDDFATYYCQQYKLYPWTFGQGTKVDIK

SEQ ID NO: 197 - protein, 25 aa, Artificial Sequence
  H-FR1 of A56-01H02
QVQLVQSGGGLVKPGRSLRLSCTAS

SEQ ID NO: 198 - protein, 17 aa, Artificial Sequence
  H-FR2 of A56-01H02
MSWFRQAPGKGLEWVGF

SEQ ID NO: 199 - protein, 38 aa, Artificial Sequence
  H-FR3 of A56-01H02
EYAASVKGRFTISRDDSKSIAYLQMNSLRAEDTAVYYC

SEQ ID NO: 200 - protein, 11 aa, Artificial Sequence
  H-FR4 of A56-01H02
WGQGTLVTVSS

SEQ ID NO: 201 - protein, 26 aa, Artificial Sequence
  L-FR1 of A56-01H02
DIQMTQSPSTLSASVGDRVTITCRAS

SEQ ID NO: 202 - protein, 17 aa, Artificial Sequence
  L-FR2 of A56-01H02
LAWYQQKPGKAPKLLIY

SEQ ID NO: 203 - protein, 36 aa, Artificial Sequence
  L-FR3 of A56-01H02
IYKASSLESGVPSRFSGSGSGTEFTLTISSLQPDDF

SEQ ID NO: 204 - protein, 10 aa, Artificial Sequence
  L-FR4 of A56-01H02
FGQGTKVDIK

SEQ ID NO: 205 - protein, 8 aa, Artificial Sequence
  H-CDR1 of A56-01H11
GYTFSRHW

SEQ ID NO: 206 - protein, 8 aa, Artificial Sequence
  H-CDR2 of A56-01H11
IHPADSDT

SEQ ID NO: 207 - protein, 9 aa, Artificial Sequence
  H-CDR3 of A56-01H11
ITEDSGRFN

SEQ ID NO: 208 - protein, 6 aa, Artificial Sequence
  L-CDR1 of A56-01H11
QSIGNY

SEQ ID NO: 209 - protein, 3 aa, Artificial Sequence
  L-CDR2 of A56-01H11
ASS

SEQ ID NO: 210 - protein, 10 aa, Artificial Sequence
  L-CDR3 of A56-01H11
QQTYNTPPIT

SEQ ID NO: 211 - DNA, 741 bp, Artificial Sequence
  SCFV of A56-01H11
caggtgcagctggtgcagtctggagcagaagtgaaaaagcccggtgactctctgaaaatctcttgtgaggcttctggctacacgtttagtaggcattggatcgtttgggtgcgccagatgcccggaaaaggcctggagtggatggggatgatccaccctgctgactctgacaccagatatagcccgtcattcggaggccaggtcaccatgtcagtcgacaagtcagccaccaccgcctacctgcagtggagcagcctgaaggcctcggacaccgccatgtattactgtattacagaagacagtggtcgcttcaactggggccagggaaccctggtcacagtctcctcaggcctcgggggcctcggaggaggaggtagtggcggaggaggctccggtggatccagcggtgtgggttccgacatccagatgacccagtctccatcctccctctctgcatctgtaggagacagagtgaccatcacttgccgggcaagtcagagcattggcaactatttaaattggtatcagcagaaacccgggaaatcccctaaactcctgatctatgcttcgtccagtttacaaagtggaattccatcaaggttcagtggcagtggatctgggacagatttcaatctcaccatcagcaatctgcaacctgaagattttggaacttattattgtcaacagacttacaatacccctccgatcaccttcggccaagggacacgactagaaatcaaa

SEQ ID NO: 212 - protein, 116 aa, Artificial Sequence
  VH2 of A56-01H11
QVQLVQSGAEVKKPGDSLKISCEASGYTFSRHWIVWVRQMPGKGLEWMGMIHPADSDTRYSPSFGGQVTMSVDKSATTAYLQWSSLKASDTAMYYCITEDSGRFNWGQGTLVTVSS

SEQ ID NO: 213 - protein, 108 aa, Artificial Sequence
  VL2 of A56-01H11
DIQMTQSPSSLSASVGDRVTITCRASQSIGNYLNWYQQKPGKSPKLLIYASSSLQSGIPSRFSGSGSGTDFNLTISNLQPEDFGTYYCQQTYNTPPITFGQGTRLEIK

SEQ ID NO: 214 - protein, 25 aa, Artificial Sequence
  H-FR1 of A56-01H11
QVQLVQSGAEVKKPGDSLKISCEAS

SEQ ID NO: 215 - protein, 17 aa, Artificial Sequence
  H-FR2 of A56-01H11
IVWVRQMPGKGLEWMGM

SEQ ID NO: 216 - protein, 38 aa, Artificial Sequence
  H-FR3 of A56-01H11
RYSPSFGGQVTMSVDKSATTAYLQWSSLKASDTAMYYC

SEQ ID NO: 217 - protein, 11 aa, Artificial Sequence
  H-FR4 of A56-01H11
WGQGTLVTVSS

SEQ ID NO: 218 - protein, 26 aa, Artificial Sequence [sequence omitted]

SEQ ID NO: 219 - protein, 17 aa, Artificial Sequence
  L-FR2 of A56-01H11
LNWYQQKPGKSPKLLIY

SEQ ID NO: 220 - protein, 36 aa, Artificial Sequence
  L-FR3 of A56-01H11
IYASSSLQSGIPSRFSGSGSGTDFNLTISNLQPEDF

SEQ ID NO: 221 - protein, 10 aa, Artificial Sequence
  L-FR4 of A56-01H11
FGQGTRLEIK

SEQ ID NO: 222 - protein, 8 aa, Artificial Sequence
  H-CDR1 of A56-02A02
GDTLTYRF

SEQ ID NO: 223 - protein, 8 aa, Artificial Sequence
  H-CDR2 of A56-02A02
ITPFNDNT

SEQ ID NO: 224 - protein, 13 aa, Artificial Sequence
  H-CDR3 of A56-02A02
ATGGGNNYYGMEV

SEQ ID NO: 225 - protein, 6 aa, Artificial Sequence
  L-CDR1 of A56-02A02
KLGDKF

SEQ ID NO: 226 - protein, 3 aa, Artificial Sequence
  L-CDR2 of A56-02A02
QDA

SEQ ID NO: 227 - protein, 9 aa, Artificial Sequence
  L-CDR3 of A56-02A02
QAWDSSSVV

SEQ ID NO: 228 - DNA, 747 bp, Artificial Sequence
  SCFV of A56-02A02
cagatgcagctggtggagtctggggctgaggtgaagaagactgggtcctcagtgaaggtttcctgcaaggcttccggagacaccctcacctaccgcttcctgcactgggtgcgacaggcccccggacaagcgcctgagtggatgggatggatcacacctttcaatgataacaccaactacgcacagaaattccaggacagagtcaccattaccagggacaggtctatgagcacagcctacatggagctgagcagcctgagatctgaggacacggccgtgtattactgtgcgactggaggtgggaacaattattacggcatggaggtctggggccaagggaccccgatcaccgtctcctcaggcctcgggggcctcggaggaggaggtagtggcggaggaggctccggtggatccagcggtgtgggttcctcctatgagctgactcagccactctcactgtccgtgtccccaggacagacagccagcatcacctgctctggagataaattgggagataaatttacttcctggtatcaacagcagccaggccagtcccctgtactggtcatctatcaagatgccaagcgaccctcagggatccctgagcgattctctggctccaactctgggagcacagccactctgaccatcagcgggacccagtctatggatgaggctgactattactgtcaggcgtgggacagcagcagtgtggtgttcggcggagggaccaagctgaccgtccta

SEQ ID NO: 229 - protein, 120 aa, Artificial Sequence
  VH2 of A56-02A02
QMQLVESGAEVKKTGSSVKVSCKASGDTLTYRFLHWVRQAPGQAPEWMGWITPFNDNTNYAQKFQDRVTITRDRSMSTAYMELSSLRSEDTAVYYCATGGGNNYYGMEVWGQGTPITVSS

SEQ ID NO: 230 - protein, 106 aa, Artificial Sequence
  VL2 of A56-02A02
SYELTQPLSLSVSPGQTASITCSGDKLGDKFTSWYQQQPGQSPVLVIYQDAKRPSGIPERFSGSNSGSTATLTISGTQSMDEADYYCQAWDSSSVVFGGGTKLTVL

SEQ ID NO: 231 - protein, 25 aa, Artificial Sequence
  H-FR1 of A56-02A02
QMQLVESGAEVKKTGSSVKVSCKAS

SEQ ID NO: 232 - protein, 17 aa, Artificial Sequence
  H-FR2 of A56-02A02
LHWVRQAPGQAPEWMGW

SEQ ID NO: 233 - protein, 38 aa, Artificial Sequence; identical to SEQ ID NO: 46
  H-FR3 of A56-02A02

SEQ ID NO: 234 - protein, 11 aa, Artificial Sequence
  H-FR4 of A56-02A02
WGQGTPITVSS

SEQ ID NO: 235 - protein, 25 aa, Artificial Sequence
  L-FR1 of A56-02A02
SYELTQPLSLSVSPGQTASITCSGD

SEQ ID NO: 236 - protein, 17 aa, Artificial Sequence
  L-FR2 of A56-02A02
TSWYQQQPGQSPVLVIY

SEQ ID NO: 237 - protein, 36 aa, Artificial Sequence
  L-FR3 of A56-02A02
IYQDAKRPSGIPERFSGSNSGSTATLTISGTQSMDE

SEQ ID NO: 238 - protein, 10 aa, Artificial Sequence
  L-FR4 of A56-02A02
FGGGTKLTVL

SEQ ID NO: 239 - protein, 8 aa, Artificial Sequence
  H-CDR1 of A56-02B01
GFTFSNYG

SEQ ID NO: 240 - protein, 8 aa, Artificial Sequence
  H-CDR2 of A56-02B01
IWFDGSNK

SEQ ID NO: 241 - protein, 12 aa, Artificial Sequence
  H-CDR3 of A56-02B01
AKAAHLWGAFDI

SEQ ID NO: 242 - protein, 6 aa, Artificial Sequence
  L-CDR1 of A56-02B01
QSVSSY

SEQ ID NO: 243 - protein, 3 aa, Artificial Sequence
  L-CDR2 of A56-02B01
GAS

SEQ ID NO: 244 - protein, 9 aa, Artificial Sequence
  L-CDR3 of A56-02B01
QQYATSPLS

SEQ ID NO: 245 - DNA, 747 bp, Artificial Sequence
  SCFV of A56-02B01
caggtgcagctggtgcagtctgggggaggtgtggtccagcctgggaggtccctgagactctcctgtgcagcgtctggattcaccttcagtaactatggcatgcactgggtccgccaggctccaggcaaggggctggaatggatggcatttatatggtttgatggaagtaataaattctatgcagactccgtgaagggccgattcaccgtctccagagacaattccaagaacaccctgtttctgcaaatgaacagtctgagagccgaggacacggccgtgtattactgtgcgaaagcggcccatttgtggggggcttttgatatctggggccaagggacaatggtcaccgtctcctcaggcctcgggggcctcggaggaggaggtagtggcggaggaggctccggtggatccagcggtgtgggttccgacatccagatgacccagtctccagacaccctgtctttgtctccaggggaaagagccaccctctcctgcagggccagtcagagtgttagcagctacttagcctggtaccaacagaaacctggccaggctcccaggctcctcatctatggtgcatccaacagggccactggcatcccagccaggttcagtggcagtgggtctgggacagacttcgctctcaccatcggcagactggagcctgaagattttgcagtttattactgtcagcagtatgctacctcaccactcagtttcggcggagggaccaaggtggaaatcaaa

SEQ ID NO: 246 - protein, 119 aa, Artificial Sequence
  VH2 of A56-02B01
QVQLVQSGGGVVQPGRSLRLSCAASGFTFSNYGMHWVRQAPGKGLEWMAFIWFDGSNKFYADSVKGRFTVSRDNSKNTLFLQMNSLRAEDTAVYYCAKAAHLWGAFDIWGQGTMVTVSS

SEQ ID NO: 247 - protein, 107 aa, Artificial Sequence
  VL2 of A56-02B01
DIQMTQSPDTLSLSPGERATLSCRASQSVSSYLAWYQQKPGQAPRLLIYGASNRATGIPARFSGSGSGTDFALTIGRLEPEDFAVYYCQQYATSPLSFGGGTKVEIK

SEQ ID NO: 248 - protein, 25 aa, Artificial Sequence
  H-FR1 of A56-02B01
QVQLVQSGGGVVQPGRSLRLSCAAS

SEQ ID NO: 249 - protein, 17 aa, Artificial Sequence
  H-FR2 of A56-02B01
MHWVRQAPGKGLEWMAF

SEQ ID NO: 250 - protein, 38 aa, Artificial Sequence
  H-FR3 of A56-02B01
FYADSVKGRFTVSRDNSKNTLFLQMNSLRAEDTAVYYC

SEQ ID NO: 251 - protein, 11 aa, Artificial Sequence
  H-FR4 of A56-02B01
WGQGTMVTVSS

SEQ ID NO: 252 - protein, 26 aa, Artificial Sequence
  L-FR1 of A56-02B01
DIQMTQSPDTLSLSPGERATLSCRAS

SEQ ID NO: 253 - protein, 17 aa, Artificial Sequence
  L-FR2 of A56-02B01
LAWYQQKPGQAPRLLIY

SEQ ID NO: 254 - protein, 36 aa, Artificial Sequence
  L-FR3 of A56-02B01
IYGASNRATGIPARFSGSGSGTDFALTIGRLEPEDF

SEQ ID NO: 255 - protein, 10 aa, Artificial Sequence
  L-FR4 of A56-02B01
FGGGTKVEIK

SEQ ID NO: 256 - protein, 8 aa, Artificial Sequence
  H-CDR1 of A56-02B02
GFTFNRHV

SEQ ID NO: 257 - protein, 8 aa, Artificial Sequence
  H-CDR2 of A56-02B02
ISNDGSKQ

SEQ ID NO: 258 - protein, 14 aa, Artificial Sequence
  H-CDR3 of A56-02B02
ASDKRGWTLNGMDV

SEQ ID NO: 259 - protein, 9 aa, Artificial Sequence
  L-CDR1 of A56-02B02
SSDVGSYNL

SEQ ID NO: 260 - protein, 3 aa, Artificial Sequence
  L-CDR2 of A56-02B02
EVT

SEQ ID NO: 261 - protein, 9 aa, Artificial Sequence
  L-CDR3 of A56-02B02
FSYAGRGVV

SEQ ID NO: 262 - DNA, 759 bp, Artificial Sequence
  SCFV of A56-02B02
caggtgcagctggtagagtctgggggaggcgtggtccagcctgggaagtccctgagactctcatgtgaagtcgctggattcaccttcaatagacatgttatgcactgggtccgccaggctccaggcaaggggctggagtggatggcttttatttcaaatgatggaagtaagcaagtctacgcagactccgtgaagggacgcttcaccatctccagagacaattccaagaacactctgtatctgcagatgaccgacctgagatctgaggacacggccgtgtattactgtgcgagtgataaaagggggtggaccctcaacggtatggacgtctggggccaagggaccacggtcaccgtctcctcaggcctcgggggcctcggaggaggaggtagtggcggaggaggctccggtggatccagcggtgtgggttcccagtctgccctgactcagcctgcctccgtgtctgggtctcctggacagtcgatcaccatctcctgcactggaaccagtagtgatgttgggagttataaccttgtctcctggtaccaacagcacccaggcaaagcccccaaactcataatttatgaggtcactaagcggccctcaggggtttctgatcgcttctctgcctccaagtctgccaacacggcctccctcacaatctctgggctccaggttgaggacgaggctgattattactgcttctcatatgcaggtcgtggcgtggtattcggcggagggaccaagctgaccgtccta

SEQ ID NO: 263 - protein, 121 aa, Artificial Sequence
  VH2 of A56-02B02
QVQLVESGGGVVQPGKSLRLSCEVAGFTFNRHVMHWVRQAPGKGLEWMAFISNDGSKQVYADSVKGRFTISRDNSKNTLYLQMTDLRSEDTAVYYCASDKRGWTLNGMDVWGQGTTVTVSS

SEQ ID NO: 264 - protein, 109 aa, Artificial Sequence
  VL2 of A56-02B02
QSALTQPASVSGSPGQSITISCTGTSSDVGSYNLVSWYQQHPGKAPKLIIYEVTKRPSGVSDRFSASKSANTASLTISGLQVEDEADYYCFSYAGRGVVFGGGTKLTVL

SEQ ID NO: 265 - protein, 25 aa, Artificial Sequence
  H-FR1 of A56-02B02
QVQLVESGGGVVQPGKSLRLSCEVA

SEQ ID NO: 266 - protein, 17 aa, Artificial Sequence
  H-FR2 of A56-02B02
MHWVRQAPGKGLEWMAF

SEQ ID NO: 267 - protein, 38 aa, Artificial Sequence
  H-FR3 of A56-02B02
VYADSVKGRFTISRDNSKNTLYLQMTDLRSEDTAVYYC

SEQ ID NO: 268 - protein, 11 aa, Artificial Sequence
  H-FR4 of A56-02B02
WGQGTTVTVSS

SEQ ID NO: 269 - protein, 25 aa, Artificial Sequence
  L-FR1 of A56-02B02
QSALTQPASVSGSPGQSITISCTGT

SEQ ID NO: 270 - protein, 17 aa, Artificial Sequence
  L-FR2 of A56-02B02
VSWYQQHPGKAPKLIIY

SEQ ID NO: 271 - protein, 36 aa, Artificial Sequence
  L-FR3 of A56-02B02
IYEVTKRPSGVSDRFSASKSANTASLTISGLQVEDE

SEQ ID NO: 272 - protein, 10 aa, Artificial Sequence
  L-FR4 of A56-02B02
FGGGTKLTVL

SEQ ID NO: 273 - protein, 8 aa, Artificial Sequence
  H-CDR1 of A56-02B06
GFTFSSYA

SEQ ID NO: 274 - protein, 8 aa, Artificial Sequence
  H-CDR2 of A56-02B06
ISYDGSNK

SEQ ID NO: 275 - protein, 11 aa, Artificial Sequence
  H-CDR3 of A56-02B06
MRDRSTGEIPH

SEQ ID NO: 276 - protein, 12 aa, Artificial Sequence
  L-CDR1 of A56-02B06
QTVLNSFNNKNY

SEQ ID NO: 277 - protein, 3 aa, Artificial Sequence
  L-CDR2 of A56-02B06
WAS

SEQ ID NO: 278 - protein, 10 aa, Artificial Sequence
  L-CDR3 of A56-02B06
QQYSSTPPIT

SEQ ID NO: 279 - DNA, 765 bp, Artificial Sequence
  SCFV of A56-02B06
caggtgcagctggtacagtctgggggaggcgtggtccagcctgggaggtccctgagactctcctgtgcagcctctggattcaccttcagtagctatgctatgcactgggtccgccaggctccaggcaaggggctggagtgggtggcagttatatcatatgatggaagcaacaaatactatgcaaactccgtgaagggccgattcatcatctccagagacaattccaacaatacggtgtatctgcaaatgaacgccctgagatctgaggacacggccgtgtattactgtatgagagatcggtcaacaggtgaaattccccactggggccagggcaccctgatcaccgtctcctcaggcctcgggggcctcggaggaggaggtagtggcggaggaggctccggtggatccagcggtgtgggttccgacatccagatgacccagtccccagactccctggctgtgtctctgggcgagagggccactatcaactgcaagtccagccagactgttttaaacagcttcaacaataagaactacttagcttggtaccagcagaaaccaggacagcctcctaaactgctcatttactgggcatctacccgggaatccggggtccctgaccgattcagtggcagcgggtctgggacagatttcactctcaccatcagcagcctgcaggctgaagatgtggcagtttattactgtcagcaatattctagtactcctccgatcaccttcggcccagggacacgactggaaatcaaa

SEQ ID NO: 280 - protein, 118 aa, Artificial Sequence
  VH2 of A56-02B06
QVQLVQSGGGVVQPGRSLRLSCAASGFTFSSYAMHWVRQAPGKGLEWVAVISYDGSNKYYANSVKGRFIISRDNSNNTVYLQMNALRSEDTAVYYCMRDRSTGEIPHWGQGTLITVSS

SEQ ID NO: 281 - protein, 114 aa, Artificial Sequence
  VL2 of A56-02B06
DIQMTQSPDSLAVSLGERATINCKSSQTVLNSFNNKNYLAWYQQKPGQPPKLLIYWASTRESGVPDRFSGSGSGTDFTLTISSLQAEDVAVYYCQQYSSTPPITFGPGTRLEIK

SEQ ID NO: 282 - protein, 25 aa, Artificial Sequence
  H-FR1 of A56-02B06
QVQLVQSGGGVVQPGRSLRLSCAAS

SEQ ID NO: 283 - protein, 17 aa, Artificial Sequence
  H-FR2 of A56-02B06
MHWVRQAPGKGLEWVAV

SEQ ID NO: 284 - protein, 38 aa, Artificial Sequence
  H-FR3 of A56-02B06
YYANSVKGRFIISRDNSNNTVYLQMNALRSEDTAVYYC

SEQ ID NO: 285 - protein, 11 aa, Artificial Sequence
  H-FR4 of A56-02B06
WGQGTLITVSS

SEQ ID NO: 286 - protein, 26 aa, Artificial Sequence
  L-FR1 of A56-02B06
DIQMTQSPDSLAVSLGERATINCKSS

SEQ ID NO: 287 - protein, 17 aa, Artificial Sequence
  L-FR2 of A56-02B06
LAWYQQKPGQPPKLLIY

SEQ ID NO: 288 - protein, 36 aa, Artificial Sequence
  L-FR3 of A56-02B06
IYWASTRESGVPDRFSGSGSGTDFTLTISSLQAEDV

SEQ ID NO: 289 - protein, 10 aa, Artificial Sequence
  L-FR4 of A56-02B06
FGPGTRLEIK

SEQ ID NO: 290 - protein, 10 aa, Artificial Sequence
  H-CDR1 of A56-02B08
GDSVSSNSAA

SEQ ID NO: 291 - protein, 9 aa, Artificial Sequence
  H-CDR2 of A56-02B08
TYYRSKWYN

SEQ ID NO: 292 - protein, 17 aa, Artificial Sequence
  H-CDR3 of A56-02B08
AKSYAGPISYYYYGLDV

SEQ ID NO: 293 - protein, 9 aa, Artificial Sequence
  L-CDR1 of A56-02B08
SSDIGRYNL

SEQ ID NO: 294 - protein, 3 aa, Artificial Sequence
  L-CDR2 of A56-02B08
GGS

SEQ ID NO: 295 - protein, 11 aa, Artificial Sequence
  L-CDR3 of A56-02B08
SSYASSSTPYV

SEQ ID NO: 296 - DNA, 784 bp, Artificial Sequence
  SCFV of A56-02B08
caggtgcagctgcagcagtcaggtccaggactggtgaagccctcgcagaccctctcactcacctgtgccatctccggggacagtgtctctagcaacagtgctgcttggaactggatcaggcagtccccatcgagaggccttgagtggctgggaaggacatactacaggtccaagtggtataatgattatgcagtatctgtgaaaagtcgaataaccatcaacccagacacatccaagaaccagttctccctgcagctgaactctgtgaccgccgtggacacggccgtgtattactgtgcgaaatcctatgcggggcctatctcttattactactacggtctggacgtctggggccaagggaccacggtcaccgtctcctcaggcctcgggggcctcggaggaggaggtagtggcggaggaggctccggtggatccagcggtgtgggttcccagtctgccctgactcagcctgcctccgtgtctgggtctcctggacagtcggtcaccatctcctgcactggaaccagcagtgacattggtcgttataaccttgtctcctggtaccaacagcacccaggcaaagcccccaaactcatgatttatgggggcagtaagcggccctcaggggtttctaatcgcttctctggctccaactctgacaacacggcctccctgacaatctctgggctccgggctgaggacgaggctgattattactgcagttcatatgcaagcagcagcaccccttatgtcttcggaactgggaccaaggtcaccgtcctaa

SEQ ID NO: 297 - protein, 127 aa, Artificial Sequence
  VH2 of A56-02B08
QVQLQQSGPGLVKPSQTLSLTCAISGDSVSSNSAAWNWIRQSPSRGLEWLGRTYYRSKWYNDYAVSVKSRITINPDTSKNQFSLQLNSVTAVDTAVYYCAKSYAGPISYYYYGLDVWGQGTTVTVSS

SEQ ID NO: 298 - protein, 111 aa, Artificial Sequence
  VL2 of A56-02B08
QSALTQPASVSGSPGQSVTISCTGTSSDIGRYNLVSWYQQHPGKAPKLMIYGGSKRPSGVSNRFSGSNSDNTASLTISGLRAEDEADYYCSSYASSSTPYVFGTGTKVTVL

SEQ ID NO: 299 - protein, 25 aa, Artificial Sequence
  H-FR1 of A56-02B08
QVQLQQSGPGLVKPSQTLSLTCAIS

SEQ ID NO: 300 - protein, 17 aa, Artificial Sequence
  H-FR2 of A56-02B08
WNWIRQSPSRGLEWLGR

SEQ ID NO: 301 - protein, 38 aa, Artificial Sequence
  H-FR3 of A56-02B08
DYAVSVKSRITINPDTSKNQFSLQLNSVTAVDTAVYYC

SEQ ID NO: 302 - protein, 11 aa, Artificial Sequence
  H-FR4 of A56-02B08
WGQGTTVTVSS

SEQ ID NO: 303 - protein, 25 aa, Artificial Sequence
  L-FR1 of A56-02B08
QSALTQPASVSGSPGQSVTISCTGT

SEQ ID NO: 304 - protein, 17 aa, Artificial Sequence
  L-FR2 of A56-02B08
VSWYQQHPGKAPKLMIY

SEQ ID NO: 305 - protein, 36 aa, Artificial Sequence
  L-FR3 of A56-02B08
IYGGSKRPSGVSNRFSGSNSDNTASLTISGLRAEDE

SEQ ID NO: 306 - protein, 10 aa, Artificial Sequence
  L-FR4 of A56-02B08
FGTGTKVTVL

SEQ ID NO: 307 - protein, 8 aa, Artificial Sequence
  H-CDR1 of A56-02B10
GGTFSRNT

SEQ ID NO: 308 - protein, 8 aa, Artificial Sequence
  H-CDR2 of A56-02B10
IIPIFHIT

SEQ ID NO: 309 - protein, 13 aa, Artificial Sequence
  H-CDR3 of A56-02B10
ARGSTTFPRYFDY

SEQ ID NO: 310 - protein, 6 aa, Artificial Sequence
  L-CDR1 of A56-02B10
QSVGSY

SEQ ID NO: 311 - protein, 3 aa, Artificial Sequence
  L-CDR2 of A56-02B10
DAS

SEQ ID NO: 312 - protein, 9 aa, Artificial Sequence
  L-CDR3 of A56-02B10
QQYGRSPFT

SEQ ID NO: 313 - DNA, 750 bp, Artificial Sequence
  SCFV of A56-02B10
caggtgcagctggtacagtctggggctgaggtgaagaagcctgggtcctcggtgaaggtctcctgcaaggcttctggaggcaccttcagcagaaatactttcagctgggtgcgacaggcccctggacaagggcttgagtggatgggagggatcatccctatctttcatataacaaattacgcacagaagatgcagggcagagtcacgatttccgcggacgagtccacgggcacagtctagatggagctgagcaggctgagatctgaggacacggccgtgtattactgtgcaagaggatcgactacttttcccagatactttgactactggggtcagggaaccctggtcaccgtctcctcaggcctcgggggcctcggaggaggaggtagtggcggaggaggctccggtggatccagcggtgtgggttccgacatccagatgacccagtctccagccaccctgtctttgtctccaggggaaagagccaccctctcctgcagggccagtcagagtgttggcagctacttagcctggtaccagcagagacctggccagcctcccaggctcctcgtctatgatgcatccaacagggccactggcatcccagccaggttcagtggcagtgggtctgggacagacttcactctcaccatcagcagactggagcctgaagattttgcagtgtatttctgtcagcagtatggtaggtcaccattcactttcggccctgggaccaaagtggatatcaaa

SEQ ID NO: 314 - protein, 120 aa, Artificial Sequence
  VH2 of A56-02B10
QVQLVQSGAEVKKPGSSVKVSCKASGGTFSRNTFSWVRQAPGQGLEWMGGIIPIFHITNYAQKMQGRVTISADESTGTVYMELSRLRSEDTAVYYCARGSTTFPRYFDYWGQGTLVTVSS

SEQ ID NO: 315 - protein, 107 aa, Artificial Sequence
  VL2 of A56-02B10
DIQMTQSPATLSLSPGERATLSCRASQSVGSYLAWYQQRPGQPPRLLVYDASNRATGIPARFSGSGSGTDFTLTISRLEPEDFAVYFCQQYGRSPFTFGPGTKVDIK

SEQ ID NO: 316 - protein, 25 aa, Artificial Sequence [sequence omitted]

SEQ ID NO: 317 - protein, 17 aa, Artificial Sequence
  H-FR2 of A56-02B10
FSWVRQAPGQGLEWMGG

SEQ ID NO: 318 - protein, 38 aa, Artificial Sequence
  H-FR3 of A56-02B10
NYAQKMQGRVTISADESTGTVYMELSRLRSEDTAVYYC

SEQ ID NO: 319 - protein, 11 aa, Artificial Sequence
  H-FR4 of A56-02B10
WGQGTLVTVSS

SEQ ID NO: 320 - protein, 26 aa, Artificial Sequence
  L-FR1 of A56-02B10
DIQMTQSPATLSLSPGERATLSCRAS

SEQ ID NO: 321 - protein, 17 aa, Artificial Sequence
  L-FR2 of A56-02B10
LAWYQQRPGQPPRLLVY

SEQ ID NO: 322 - protein, 36 aa, Artificial Sequence
  L-FR3 of A56-02B10
VYDASNRATGIPARFSGSGSGTDFTLTISRLEPEDF

SEQ ID NO: 323 - protein, 10 aa, Artificial Sequence
  L-FR4 of A56-02B10
FGPGTKVDIK

SEQ ID NO: 324 - protein, 8 aa, Artificial Sequence
  H-CDR1 of A56-02C06
GFTFSTYG

SEQ ID NO: 325 - protein, 8 aa, Artificial Sequence
  H-CDR2 of A56-02C06
ISGGGSST

SEQ ID NO: 326 - protein, 11 aa, Artificial Sequence
  H-CDR3 of A56-02C06
ARWGVMLSFDY

SEQ ID NO: 327 - protein, 6 aa, Artificial Sequence
  L-CDR1 of A56-02C06
YSVSPW

SEQ ID NO: 328 - protein, 3 aa, Artificial Sequence
  L-CDR2 of A56-02C06
KAS

SEQ ID NO: 329 - protein, 10 aa, Artificial Sequence
  L-CDR3 of A56-02C06
QQFNSYMMYT

SEQ ID NO: 330 - DNA, 747 bp, Artificial Sequence
  SCFV of A56-02C06
caggtgcagctggtggagtctgggggaggcttggtacagcctgggaaatccctgagactctcctgtgcagcctctggattcaccttcagcacctatggcatgacttgggtccgccaggctccagggaaggggctggagtgggtctcagggattagtggtgggggttctagcacaaactacgcagactccgtgaagggccgcttcatcatttctagagacaactctaacaacacgctgtatctgcaaatgaacagtctgagagccgaggacacggccgtgtattactgtgcaaggtggggagttatgctttcctttgactactggggccagggaaccccggtcaccgtctcctcaggcctcgggggcctcggaggaggaggtagtggcggaggaggctccggtggatccagcggtgtgggttccgacatccagatgacccagtctccttccaccctgcctgcatctgtaggggacagagtcaccatcacttgccgggccagttacagtgtcagtccctggttggcctggtatcagcagaaaccagggaaagcccctaaactcctgatctataaggcatctactttagaaagtggggtcccatcaaggttcagcggcagtggatctgggacagaattcactctcaccatcagcagcctgcagcctgatgattttgcaacttattactgccaacagtttaatagttatatgatgtacacttttggccaggggaccaagctggaaatcaaa

SEQ ID NO: 331 - protein, 118 aa, Artificial Sequence
  VH2 of A56-02C06
QVQLVESGGGLVQPGKSLRLSCAASGFTFSTYGMTWVRQAPGKGLEWVSGISGGGSSTNYADSVKGRFIISRDNSNNTLYLQMNSLRAEDTAVYYCARWGVMLSFDYWGQGTPVTVSS

SEQ ID NO: 332 - protein, 108 aa, Artificial Sequence
  VL2 of A56-02C06
DIQMTQSPSTLPASVGDRVTITCRASYSVSPWLAWYQQKPGKAPKLLIYKASTLESGVPSRFSGSGSGTEFTLTISSLQPDDFATYYCQQFNSYMMYTFGQGTKLEIK

SEQ ID NO: 333 - protein, 25 aa, Artificial Sequence
  H-FR1 of A56-02C06
QVQLVESGGGLVQPGKSLRLSCAAS

SEQ ID NO: 334 - protein, 17 aa, Artificial Sequence
  H-FR2 of A56-02C06
MTWVRQAPGKGLEWVSG

SEQ ID NO: 335 - protein, 38 aa, Artificial Sequence
  H-FR3 of A56-02C06
NYADSVKGRFIISRDNSNNTLYLQMNSLRAEDTAVYYC

SEQ ID NO: 336 - protein, 11 aa, Artificial Sequence
  H-FR4 of A56-02C06
WGQGTPVTVSS

SEQ ID NO: 337 - protein, 26 aa, Artificial Sequence
  L-FR1 of A56-02C06
DIQMTQSPSTLPASVGDRVTITCRAS

SEQ ID NO: 338 - protein, 17 aa, Artificial Sequence
  L-FR2 of A56-02C06
LAWYQQKPGKAPKLLIY

SEQ ID NO: 339 - protein, 36 aa, Artificial Sequence
  L-FR3 of A56-02C06
IYKASTLESGVPSRFSGSGSGTEFTLTISSLQPDDF

SEQ ID NO: 340 - protein, 10 aa, Artificial Sequence
  L-FR4 of A56-02C06
FGQGTKLEIK

SEQ ID NO: 341 - protein, 8 aa, Artificial Sequence
  H-CDR1 of A56-02C07
GVTFSGYV

SEQ ID NO: 342 - protein, 8 aa, Artificial Sequence
  H-CDR2 of A56-02C07
IIPLIDVE

SEQ ID NO: 343 - protein, 17 aa, Artificial Sequence
  H-CDR3 of A56-02C07
AKSVVRGLDYYYYGFDV

SEQ ID NO: 344 - protein, 6 aa, Artificial Sequence
  L-CDR1 of A56-02C07
NIGSKS

SEQ ID NO: 345 - protein, 3 aa, Artificial Sequence
  L-CDR2 of A56-02C07
YDG

SEQ ID NO: 346 - protein, 11 aa, Artificial Sequence
  L-CDR3 of A56-02C07
QVWDSSSDQGV

SEQ ID NO: 347 - DNA, 765 bp, Artificial Sequence
  SCFV of A56-02C07
caggtgcagctggtggagtctggggctgaggtgaggaggcctgggtcctcggtgaaggtctcctgcaagacttcgggagtcaccttcagcggctatgttctgagctgggtgcgacaggcccctggacacggccttgagtggatgggacggatcatccctttaattgacgtggaaaactatgcacgggagttccagggtagaatgaagatcaccgcagacaagtccacgaatacagtctacatggaactgaacaacctgagatctgaggacacggccgtgtattactgtgcgaaatcggtcgtacggggtcttgactactactactacggtttcgacgtctggggccaagggaccacggtcaccgtctcctcaggcctcgggggcctcggaggaggaggtagtggcggaggaggctccggtggatccagcggtgtgggttcctcctatgagctgacacaaccaccctcactgtcagtggccccaggaaagacggccaggattacctgtgggggaaacaacattggaagtaaaagtgtgcactggtaccagcagaagccaggccaggcccctagactggtcacttattatgatggcaaccggccctcagggatccctgagcgattctctggctccaactctggaaacacggccaccctaatcatcagcagggtcgaagccggggatgaggccgactattactgtcaggtgtgggatagtagtagtgatcagggggtcttcggaactgggaccaaggtcaccgtccta

SEQ ID NO: 348 - protein, 124 aa, Artificial Sequence
  VH2 of A56-02C07
QVQLVESGAEVRRPGSSVKVSCKTSGVTFSGYVLSWVRQAPGHGLEWMGRIIPLIDVENYAREFQGRMKITADKSTNTVYMELNNLRSEDTAVYYCAKSVVRGLDYYYYGFDVWGQGTTVTVSS

SEQ ID NO: 349 - protein, 108 aa, Artificial Sequence
  VL2 of A56-02C07
SYELTQPPSLSVAPGKTARITCGGNNIGSKSVHWYQQKPGQAPRLVTYYDGNRPSGIPERFSGSNSGNTATLIISRVEAGDEADYYCQVWDSSSDQGVFGTGTKVTVL

SEQ ID NO: 350 - protein, 25 aa, Artificial Sequence
  H-FR1 of A56-02C07
QVQLVESGAEVRRPGSSVKVSCKTS

SEQ ID NO: 351 - protein, 17 aa, Artificial Sequence
  H-FR2 of A56-02C07
LSWVRQAPGHGLEWMGR

SEQ ID NO: 352 - protein, 38 aa, Artificial Sequence
  H-FR3 of A56-02C07
NYAREFQGRMKITADKSTNTVYMELNNLRSEDTAVYYC

SEQ ID NO: 353 - protein, 11 aa, Artificial Sequence
  H-FR4 of A56-02C07
WGQGTTVTVSS

SEQ ID NO: 354 - protein, 25 aa, Artificial Sequence
  L-FR1 of A56-02C07
SYELTQPPSLSVAPGKTARITCGGN

SEQ ID NO: 355 - protein, 17 aa, Artificial Sequence
  L-FR2 of A56-02C07
VHWYQQKPGQAPRLVTY

SEQ ID NO: 356 - protein, 36 aa, Artificial Sequence
  L-FR3 of A56-02C07
TYYDGNRPSGIPERFSGSNSGNTATLIISRVEAGDE

SEQ ID NO: 357 - protein, 10 aa, Artificial Sequence
  L-FR4 of A56-02C07
FGTGTKVTVL

SEQ ID NO: 358 - protein, 8 aa, Artificial Sequence
  H-CDR1 of A56-02C09
GGTFSSYT

SEQ ID NO: 359 - protein, 8 aa, Artificial Sequence
  H-CDR2 of A56-02C09
IIPILGIA

SEQ ID NO: 360 - protein, 18 aa, Artificial Sequence
  H-CDR3 of A56-02C09
AKDMVRGFRHYYYYGMDV

SEQ ID NO: 361 - protein, 9 aa, Artificial Sequence
  L-CDR1 of A56-02C09
NSDVGDYNL

SEQ ID NO: 362 - protein, 3 aa, Artificial Sequence
  L-CDR2 of A56-02C09
EVT

SEQ ID NO: 363 - protein, 10 aa, Artificial Sequence
  L-CDR3 of A56-02C09
SSYTSSSTYV

SEQ ID NO: 364 - DNA, 774 bp, Artificial Sequence
  SCFV of A56-02C09
caggtgcagctggtgcagtctggggctgaggtgaagaagcctgggtcctcggtgaaggtctcctgcaaggcttctggaggcaccttcagcagctatactatcagctgggtgcgacaggcccctggacaagggcttgagtggatgggaaggatcatccctatccttggtatagcaaactacgcacagaagttccagggcagagtcacgattaccgcggacaaatccacgagcacagcctacatggagctgagcagcctgagatctgaggacacggccgtgtattactgtgcgaaagacatggttcggggatttagacactactactactacggtatggacgtctggggcccagggaccaaggtcaccgtctcctcaggcctcgggggcctcggaggaggaggtagtggcggaggaggctccggtggatccagcggtgtgggttcccagtctgccctgactcagcctgcctccgtgtctgggtctcctggacagtcgatcaccatctcctgcactggaaccaacagtgatgttggagattataaccttgtctcctggtaccaacaacacccaggcaaagcccccaaactcatgatttatgaggtcactaagcggccctcaggggtttctaatcgcttctctggctccaagtctggcaacacggcctccctgaccatctctgggctccaggctgaggacgaggctgattattactgcagctcatatacaagcagcagcacttatgtcttcggaactgggaccaaggtcaccgtccta

SEQ ID NO: 365 - protein, 125 aa, Artificial Sequence
  VH2 of A56-02C09
QVQLVQSGAEVKKPGSSVKVSCKASGGTFSSYTISWVRQAPGQGLEWMGRIIPILGIANYAQKFQGRVTITADKSTSTAYMELSSLRSEDTAVYYCAKDMVRGFRHYYYYGMDVWGPGTKVTVSS

SEQ ID NO: 366 - protein, 110 aa, Artificial Sequence
  VL2 of A56-02C09
QSALTQPASVSGSPGQSITISCTGTNSDVGDYNLVSWYQQHPGKAPKLMIYEVTKRPSGVSNRFSGSKSGNTASLTISGLQAEDEADYYCSSYTSSSTYVFGTGTKVTVL

SEQ ID NO: 367 - protein, 25 aa, Artificial Sequence [sequence omitted]

SEQ ID NO: 368 - protein, 17 aa, Artificial Sequence
  H-FR2 of A56-02C09
ISWVRQAPGQGLEWMGR

SEQ ID NO: 369 - protein, 38 aa, Artificial Sequence
  H-FR3 of A56-02C09
NYAQKFQGRVTITADKSTSTAYMELSSLRSEDTAVYYC

SEQ ID NO: 370 - protein, 11 aa, Artificial Sequence
  H-FR4 of A56-02C09
WGPGTKVTVSS

SEQ ID NO: 371 - protein, 25 aa, Artificial Sequence
  L-FR1 of A56-02C09
QSALTQPASVSGSPGQSITISCTGT

SEQ ID NO: 372 - protein, 17 aa, Artificial Sequence
  L-FR2 of A56-02C09
VSWYQQHPGKAPKLMIY

SEQ ID NO: 373 - protein, 36 aa, Artificial Sequence
  L-FR3 of A56-02C09
IYEVTKRPSGVSNRFSGSKSGNTASLTISGLQAEDE

SEQ ID NO: 374 - protein, 10 aa, Artificial Sequence
  L-FR4 of A56-02C09
FGTGTKVTVL

SEQ ID NO: 375 - protein, 8 aa, Artificial Sequence
  H-CDR1 of A56-02D04
GFTFKNFA

SEQ ID NO: 376 - protein, 8 aa, Artificial Sequence
  H-CDR2 of A56-02D04
INGDGSDT

SEQ ID NO: 377 - protein, 14 aa, Artificial Sequence
  H-CDR3 of A56-02D04
AKEIAEVGRPNFDY

SEQ ID NO: 378 - protein, 7 aa, Artificial Sequence
  L-CDR1 of A56-02D04
QSVTSTY

SEQ ID NO: 379 - protein, 3 aa, Artificial Sequence
  L-CDR2 of A56-02D04
GAS

SEQ ID NO: 380 - protein, 9 aa, Artificial Sequence
  L-CDR3 of A56-02D04
QQYGSSPYT

SEQ ID NO: 381 - DNA, 756 bp, Artificial Sequence
  SCFV of A56-02D04
caggtgcagctggtagagtccgggggaggcttagttgagcctggggggtccctgagactctcctgtgcagcctctggattcaccttcaaaaacttcgcgatgtactgggtccgccaagctccagggaaggggctggtgtgggtctcacgtattaatggtgatgggagtgacacaacgtacgcggagtccgtgaagggccgattcaccacctccagagacaacgccaagaacacagtgtatttgcaaatgaacagtctgagagccgaggacacggccgtgtattactgtgcgaaagagatagcggaagtcggtaggccgaactttgactactggggccagggaaccctggtcaccgtctcctcaggcctcgggggcctcggaggaggaggtagtggcggaggaggctccggtggatccagcggtgtgggttccgacatccagatgacccagtctccaggcaccctgtctttgtctccaggggatacagccaccctctcctgcagggccagtcagagtgttaccagcacctacttagcctggtatcagcagaaacctggccaggctcccaggctcctcatctctggtgcatccagcagggccgctggcatcccagccaggttcactggcagtgggtctgagacagacttcactctcaccatcagcagactggagcctgaagattttgcagtgtattactgtcagcagtatggtagctcaccgtacacttttggccaggggaccaagctggaaatcaaa

SEQ ID NO: 382 - protein, 121 aa, Artificial Sequence
  VH2 of A56-02D04
QVQLVESGGGLVEPGGSLRLSCAASGFTFKNFAMYWVRQAPGKGLVWVSRINGDGSDTTYAESVKGRFTTSRDNAKNTVYLQMNSLRAEDTAVYYCAKEIAEVGRPNFDYWGQGTLVTVSS

SEQ ID NO: 383 - protein, 108 aa, Artificial Sequence
  VL2 of A56-02D04
DIQMTQSPGTLSLSPGDTATLSCRASQSVTSTYLAWYQQKPGQAPRLLISGASSRAAGIPARFTGSGSETDFTLTISRLEPEDFAVYYCQQYGSSPYTFGQGTKLEIK

SEQ ID NO: 384 - protein, 25 aa, Artificial Sequence
  H-FR1 of A56-02D04
QVQLVESGGGLVEPGGSLRLSCAAS

SEQ ID NO: 385 - protein, 17 aa, Artificial Sequence
  H-FR2 of A56-02D04
MYWVRQAPGKGLVWVSR

SEQ ID NO: 386 - protein, 38 aa, Artificial Sequence
  H-FR3 of A56-02D04
TYAESVKGRFTTSRDNAKNTVYLQMNSLRAEDTAVYYC

SEQ ID NO: 387 - protein, 11 aa, Artificial Sequence
  H-FR4 of A56-02D04
WGQGTLVTVSS

SEQ ID NO: 388 - protein, 26 aa, Artificial Sequence
  L-FR1 of A56-02D04
DIQMTQSPGTLSLSPGDTATLSCRAS

SEQ ID NO: 389 - protein, 17 aa, Artificial Sequence
  L-FR2 of A56-02D04
LAWYQQKPGQAPRLLIS

SEQ ID NO: 390 - protein, 36 aa, Artificial Sequence
  L-FR3 of A56-02D04
ISGASSRAAGIPARFTGSGSETDFTLTISRLEPEDF

SEQ ID NO: 391 - protein, 10 aa, Artificial Sequence
  L-FR4 of A56-02D04
FGQGTKLEIK

SEQ ID NO: 392 - protein, 8 aa, Artificial Sequence
  H-CDR1 of A56-02E01
GGSSSNYA

SEQ ID NO: 393 - protein, 8 aa, Artificial Sequence
  H-CDR2 of A56-02E01
ITPFNGNT

SEQ ID NO: 394 - protein, 12 aa, Artificial Sequence
  H-CDR3 of A56-02E01
ASSRGRFQWFDY

SEQ ID NO: 395 - protein, 7 aa, Artificial Sequence
  L-CDR1 of A56-02E01
QSVKNND

SEQ ID NO: 396 - protein, 3 aa, Artificial Sequence
  L-CDR2 of A56-02E01
GTS

SEQ ID NO: 397 - protein, 10 aa, Artificial Sequence
  L-CDR3 of A56-02E01
QQFGGSPPWT

SEQ ID NO: 398 - DNA, 753 bp, Artificial Sequence
  SCFV of A56-02E01
caggtgcagctggtgcagtctggggctgaggtgaagaagcctgggtcctcggtgaaggtctcctgcaaggcttccggaggctcctccagcaactatgctatcagctgggtgcgacaggcccctggacaagggcttgagtggatgggatggatcacacctttcaatggtaacaccagctacgcgcagatattccaggacagagtcaccattaccagggacaggtctatgagcacagcctacatggagctgagcagcctgagatctgaggacacggccgtgtattactgtgcgagttcgagggggcggtttcaatggtttgactactggggcccgggaaccctggtcaccgtctcctcaggcctcgggggcctcggaggaggaggtagtggcggaggaggctccggtggatccagcggtgtgggttccgacatccagatgacccagtctcctgccaccctgtctgtgtctccaggggaaagagccaccctctcctgcaggaccagtcagagtgttaagaacaacgacctagcctggtaccagcagaaacctggccaggctcccaggctcctcatctatggtacgtccaccagggccactggcatccccgacaggttcagtggcagtgggtctgggacagacttcactctcaccatcagcagcctagagcctgaagattttgcagtttattactgtcaacaatttggtggttcacctccgtggacgttcggccaagggaccaaggtggatatcaaa

SEQ ID NO: 399 - protein, 119 aa, Artificial Sequence
  VH2 of A56-02E01
QVQLVQSGAEVKKPGSSVKVSCKASGGSSSNYAISWVRQAPGQGLEWMGWITPFNGNTSYAQIFQDRVTITRDRSMSTAYMELSSLRSEDTAVYYCASSRGRFQWFDYWGPGTLVTVSS

SEQ ID NO: 400 - protein, 109 aa, Artificial Sequence
  VL2 of A56-02E01
DIQMTQSPATLSVSPGERATLSCRTSQSVKNNDLAWYQQKPGQAPRLLIYGTSTRATGIPDRFSGSGSGTDFTLTISSLEPEDFAVYYCQQFGGSPPWTFGQGTKVDIK

SEQ ID NO: 401 - protein, 25 aa, Artificial Sequence [sequence omitted]

SEQ ID NO: 402 - protein, 17 aa, Artificial Sequence
  H-FR2 of A56-02E01
ISWVRQAPGQGLEWMGW

SEQ ID NO: 403 - protein, 38 aa, Artificial Sequence
  H-FR3 of A56-02E01
SYAQIFQDRVTITRDRSMSTAYMELSSLRSEDTAVYYC

SEQ ID NO: 404 - protein, 11 aa, Artificial Sequence
  H-FR4 of A56-02E01
WGPGTLVTVSS

SEQ ID NO: 405 - protein, 26 aa, Artificial Sequence
  L-FR1 of A56-02E01
DIQMTQSPATLSVSPGERATLSCRTS

SEQ ID NO: 406 - protein, 17 aa, Artificial Sequence
  L-FR2 of A56-02E01
LAWYQQKPGQAPRLLIY

SEQ ID NO: 407 - protein, 36 aa, Artificial Sequence
  L-FR3 of A56-02E01
IYGTSTRATGIPDRFSGSGSGTDFTLTISSLEPEDF

SEQ ID NO: 408 - protein, 10 aa, Artificial Sequence
  L-FR4 of A56-02E01
FGQGTKVDIK

SEQ ID NO: 409 - protein, 8 aa, Artificial Sequence
  H-CDR1 of A56-02E05
GFTSGDYA

SEQ ID NO: 410 - protein, 10 aa, Artificial Sequence
  H-CDR2 of A56-02E05
IGSSGYGGPT

SEQ ID NO: 411 - protein, 17 aa, Artificial Sequence
  H-CDR3 of A56-02E05
ARDLGFGYSGYRNAFDS

SEQ ID NO: 412 - protein, 8 aa, Artificial Sequence
  L-CDR1 of A56-02E05
GGTFASDS

SEQ ID NO: 413 - protein, 3 aa, Artificial Sequence
  L-CDR2 of A56-02E05
EGD

SEQ ID NO: 414 - protein, 9 aa, Artificial Sequence
  L-CDR3 of A56-02E05
QSYDSSNQV

SEQ ID NO: 415 - DNA, 777 bp, Artificial Sequence
  SCFV of A56-02E05
caggtgcagctggtagagtctgggggaggctgggtacagccagggcggtccctgagactctcctgtacagtctctggattcacgtctggtgattatgctgtgagttgggtccgccaggctccagggaaggggctggagtgggtaggtgtcattggaagcagcggttatggtgggccaacaaaatatgctgcgtctgtggaaggcagattcaccatctcaagagatgattccaaagacatcgcctatctgcaaatgaacagtctgagagccgaggacacggccgtgtattactgtgcgagagacttagggttcggatatagtggctacaggaatgcttttgatagttggggccaagggacaatggtcaccgtctcctcaggcctcgggggcctcggaggaggaggtagtggcggaggaggctccggtggatccagcggtgtgggttcccagctcgtgctgactcagccccactctgtgtcggagtctccggggaagacggtaaccatctcctgcaccggcagtggtggcacctttgccagcgactcggtgcagtggtaccggcagcgcccgggcagtgcccccaccactgtgatctatgagggtgaccgaagagcctctggggtccctggtcggttctctggctccatcgacagctcctccaactctgcctccctcaccatctctggactgaaggctgaagacgaggctgactactactgtcagtcttatgatagcagcaatcaggtcttcggaactgggaccaaggtcaccgtccta

SEQ ID NO: 416 - protein, 126 aa, Artificial Sequence
  VH2 of A56-02E05
QVQLVESGGGWVQPGRSLRLSCTVSGFTSGDYAVSWVRQAPGKGLEWVGVIGSSGYGGPTKYAASVEGRFTISRDDSKDIAYLQMNSLRAEDTAVYYCARDLGFGYSGYRNAFDSWGQGTMVTVSS

SEQ ID NO: 417 - protein, 110 aa, Artificial Sequence
  VL2 of A56-02E05
QLVLTQPHSVSESPGKTVTISCTGSGGTFASDSVQWYRQRPGSAPTTVIYEGDRRASGVPGRFSGSIDSSSNSASLTISGLKAEDEADYYCQSYDSSNQVFGTGTKVTVL

SEQ ID NO: 418 - protein, 25 aa, Artificial Sequence
  H-FR1 of A56-02E05
QVQLVESGGGWVQPGRSLRLSCTVS

SEQ ID NO: 419 - protein, 17 aa, Artificial Sequence
  H-FR2 of A56-02E05
VSWVRQAPGKGLEWVGV

SEQ ID NO: 420 - protein, 38 aa, Artificial Sequence
  H-FR3 of A56-02E05
KYAASVEGRFTISRDDSKDIAYLQMNSLRAEDTAVYYC

SEQ ID NO: 421 - protein, 11 aa, Artificial Sequence
  H-FR4 of A56-02E05
WGQGTMVTVSS

SEQ ID NO: 422 - protein, 25 aa, Artificial Sequence
  L-FR1 of A56-02E05
QLVLTQPHSVSESPGKTVTISCTGS

SEQ ID NO: 423 - protein, 17 aa, Artificial Sequence
  L-FR2 of A56-02E05
VQWYRQRPGSAPTTVIY

SEQ ID NO: 424 - protein, 36 aa, Artificial Sequence
  L-FR3 of A56-02E05
IYEGDRRASGVPGRFSGSIDSSSNSASLTISGLKAE

SEQ ID NO: 425 - protein, 10 aa, Artificial Sequence
  L-FR4 of A56-02E05
FGTGTKVTVL

SEQ ID NO: 426 - protein, 8 aa, Artificial Sequence
  H-CDR1 of A56-02F05
GFSFSGYA

SEQ ID NO: 427 - protein, 8 aa, Artificial Sequence
  H-CDR2 of A56-02F05
IWFDGSTK

SEQ ID NO: 428 - protein, 10 aa, Artificial Sequence
  H-CDR3 of A56-02F05
ARMFRGSFDY

SEQ ID NO: 429 - protein, 11 aa, Artificial Sequence
  L-CDR1 of A56-02F05
QSLVHRDGNTY

SEQ ID NO: 430 - protein, 3 aa, Artificial Sequence
  L-CDR2 of A56-02F05
KIS

SEQ ID NO: 431 - protein, 8 aa, Artificial Sequence
  L-CDR3 of A56-02F05
MQATRLWT

SEQ ID NO: 432 - DNA, 753 bp, Artificial Sequence
  SCFV of A56-02F05
caggtgcagctggtggagtctgggggaggtgtggtccagcctggggcgtccctgaaactctcctgtgcagcgtccggattcagcttcagtggctatgccatgcactgggtccgccaggctccaggcatggggctggagtgggtggcagttatctggtttgatggaagtactaaatactatgcagactccgtgaagggccgattcaccatctcccgagacaattccaagaatacactttttctgcaaatgaacagtctgagagccgaggacacggccgtgtattactgtgcgagaatgtttaggggttcctttgactactggggccagggagccctggtcaccgtctcctcaggcctcgggggcctcggaggaggaggtagtggcggaggaggctccggtggatccagcggtgtgggttccgatattgtgatgacccagactccactctcctcacctgtcacccttggacagccggcctccatctcctgtaggtctagtcagagcctcgtacaccgtgatggaaacacatacttgagttggtttcaacagaggccaggccagtctccaagactcctgatttctaagatttctaaccgctcctctgaagtctcagacaggttcagtggcagtggggcagggacagaattcacgctgaagatcagcagggtggaagctgaggatgtcggaatttattactgcatgcaggctacacgattgtggaccttcggccaagggaccaaggtggagatcaaa

SEQ ID NO: 433 - protein, 117 aa, Artificial Sequence
  VH2 of A56-02F05
QVQLVESGGGVVQPGASLKLSCAASGFSFSGYAMHWVRQAPGMGLEWVAVIWFDGSTKYYADSVKGRFTISRDNSKNTLFLQMNSLRAEDTAVYYCARMFRGSFDYWGQGALVTVSS

SEQ ID NO: 434 - protein, 111 aa, Artificial Sequence
  VL2 of A56-02F05
DIVMTQTPLSSPVTLGQPASISCRSSQSLVHRDGNTYLSWFQQRPGQSPRLLISKISNRSSEVSDRFSGSGAGTEFTLKISRVEAEDVGIYYCMQATRLWTFGQGTKVEIK

SEQ ID NO: 435 - protein, 25 aa, Artificial Sequence
  H-FR1 of A56-02F05
QVQLVESGGGVVQPGASLKLSCAAS

SEQ ID NO: 436 - protein, 17 aa, Artificial Sequence
  H-FR2 of A56-02F05
MHWVRQAPGMGLEWVAV

SEQ ID NO: 437 - protein, 38 aa, Artificial Sequence
  H-FR3 of A56-02F05
YYADSVKGRFTISRDNSKNTLFLQMNSLRAEDTAVYYC

SEQ ID NO: 438 - protein, 11 aa, Artificial Sequence
  H-FR4 of A56-02F05
WGQGALVTVSS

SEQ ID NO: 439 - protein, 26 aa, Artificial Sequence
  L-FR1 of A56-02F05
DIVMTQTPLSSPVTLGQPASISCRSS

SEQ ID NO: 440 - protein, 17 aa, Artificial Sequence
  L-FR2 of A56-02F05
LSWFQQRPGQSPRLLIS

SEQ ID NO: 441 - protein, 36 aa, Artificial Sequence
  L-FR3 of A56-02F05
ISKISNRSSEVSDRFSGSGAGTEFTLKISRVEAEDV

SEQ ID NO: 442 - protein, 10 aa, Artificial Sequence
  L-FR4 of A56-02F05
FGQGTKVEIK

SEQ ID NO: 443 - protein, 8 aa, Artificial Sequence
  H-CDR1 of A56-03A09
GFTFSDYA

SEQ ID NO: 444 - protein, 8 aa, Artificial Sequence
  H-CDR2 of A56-03A09
ISSSGGST

SEQ ID NO: 445 - protein, 14 aa, Artificial Sequence
  H-CDR3 of A56-03A09
ARLRPFSKADSFDY

SEQ ID NO: 446 - protein, 12 aa, Artificial Sequence
  L-CDR1 of A56-03A09
QSVLSSSSNKNF

SEQ ID NO: 447 - protein, 3 aa, Artificial Sequence
  L-CDR2 of A56-03A09
WAS

SEQ ID NO: 448 - protein, 9 aa, Artificial Sequence
  L-CDR3 of A56-03A09
QQYYSSPLT

SEQ ID NO: 449 - DNA, 771 bp, Artificial Sequence
  SCFV of A56-03A09
caggtgcagctggtggagtctgggggaggcttggtacagccgggggggtccctgagactctcctgcagtgcctctggattcacctttagtgactatgccatgagctgggtccgccaggccccagggaagcggctggagtgggtctcagcgattagtagtagtggtggtagcacacactacgcagacttcgtgaagggccggttcaccatttccagagacaaatccaagaacacactctttctgcaaatgaacagtctgagagccgaggacacggccgtgtattactgtgcgagactgagacctttttctaaggccgattcttttgactactggggccttggaaccctgatcaccgtctcctcaggcctcgggggcctcggaggaggaggtagtggcggaggaggctccggtggatccagcggtgtgggttccgacatccagatgacccagtctccagactccctggctgtgtctctgggcgagagggccaccatcaactgcaagtccagtcagagtgttttatccagctctagcaataagaacttcttagcttggtaccagcaaaaaccaggacagcctcctaagctgctcatttactgggcatctgcccgggaatccggggtccctgaccgattcagtggcagcgggtctgggacagatttcactctcaccatcagcagcctgcaggctgaagatgtggcagtttattactgtcagcaatattatagtagtccgctcactttcggcggagggaccaaggtggagatcaaa

SEQ ID NO: 450 - protein, 121 aa, Artificial Sequence
  VH2 of A56-03A09
QVQLVESGGGLVQPGGSLRLSCSASGFTFSDYAMSWVRQAPGKRLEWVSAISSSGGSTHYADFVKGRFTISRDKSKNTLFLQMNSLRAEDTAVYYCARLRPFSKADSFDYWGLGTLITVSS

SEQ ID NO: 451 - protein, 113 aa, Artificial Sequence
  VL2 of A56-03A09
DIQMTQSPDSLAVSLGERATINCKSSQSVLSSSSNKNFLAWYQQKPGQPPKLLIYWASARESGVPDRFSGSGSGTDFTLTISSLQAEDVAVYYCQQYYSSPLTFGGGTKVEIK

SEQ ID NO: 452 - protein, 25 aa, Artificial Sequence
  H-FR1 of A56-03A09
QVQLVESGGGLVQPGGSLRLSCSAS

SEQ ID NO: 453 - protein, 17 aa, Artificial Sequence
  H-FR2 of A56-03A09
MSWVRQAPGKRLEWVSA

SEQ ID NO: 454 - protein, 38 aa, Artificial Sequence
  H-FR3 of A56-03A09
HYADFVKGRFTISRDKSKNTLFLQMNSLRAEDTAVYYC

SEQ ID NO: 455 - protein, 11 aa, Artificial Sequence
  H-FR4 of A56-03A09
WGLGTLITVSS

SEQ ID NO: 456 - protein, 26 aa, Artificial Sequence
  L-FR1 of A56-03A09
DIQMTQSPDSLAVSLGERATINCKSS

SEQ ID NO: 457 - protein, 17 aa, Artificial Sequence
  L-FR2 of A56-03A09
LAWYQQKPGQPPKLLIY

SEQ ID NO: 458 - protein, 36 aa, Artificial Sequence
  L-FR3 of A56-03A09
IYWASARESGVPDRFSGSGSGTDFTLTISSLQAEDV

SEQ ID NO: 459 - protein, 10 aa, Artificial Sequence
  L-FR4 of A56-03A09
FGGGTKVEIK

SEQ ID NO: 460 - protein, 8 aa, Artificial Sequence
  H-CDR1 of A56-03B03
GGNFNSYA

SEQ ID NO: 461 - protein, 8 aa, Artificial Sequence
  H-CDR2 of A56-03B03
IIPFFTTP

SEQ ID NO: 462 - protein, 5 aa, Artificial Sequence
  H-CDR3 of A56-03B03
VTRGA

SEQ ID NO: 463 - protein, 9 aa, Artificial Sequence
  L-CDR1 of A56-03B03
SSDVGGYNY

SEQ ID NO: 464 - protein, 3 aa, Artificial Sequence
  L-CDR2 of A56-03B03
DVT

SEQ ID NO: 465 - protein, 11 aa, Artificial Sequence
  L-CDR3 of A56-03B03
QVWDSSSDHYV

SEQ ID NO: 466 - DNA, 738 bp, Artificial Sequence
  SCFV of A56-03B03
caggtgcagctggtggagtctggggctgaggtgaagaagcctgggtcctcggttaaagtctcctgcaagacttctggcggcaacttcaacagctatgctatcaactgggtgcgacaggcccctggacaagggcttgagtggatgggaagcatcatcccattctttactacaccaaactacgcacagaaattccagggcagagtcacgattaccgcggacgaatccacgaacacagccttcatggaattgagcagtctgggatctgaggacacggccgtgtattactgtgtgactagaggcgcgcagggccggggaaccctggtcaccgtctcctcaggcctcgggggcctcggaggaggaggtagtggcggaggaggctccggtggatccagcggtgtgggttccaattttatgctgactcaacccgcctccgtgtctgggtcccctggacagtcgatcaccatctcctgcactggaagcagcagcgacgttggtggttataactatgtctcctggtaccaacagcacccaggcaaagccccccaactcatcatttatgatgtcactaagcggccctcaggggtttctaatcgcttctctggctccaactctggaaacacggccaccctgaccatcagcagggtcgaagccggggatgaggccgactattactgccaggtgtgggatagtagtagtgatcactatgtcttcggaactgggaccaaggtcaccgtccta

SEQ ID NO: 467 - protein, 112 aa, Artificial Sequence
  VH2 of A56-03B03
QVQLVESGAEVKKPGSSVKVSCKTSGGNFNSYAINWVRQAPGQGLEWMGSIIPFFTTPNYAQKFQGRVTITADESTNTAFMELSSLGSEDTAVYYCVTRGAQGRGTLVTVSS

SEQ ID NO: 468 - protein, 111 aa, Artificial Sequence
  VL2 of A56-03B03
NFMLTQPASVSGSPGQSITISCTGSSSDVGGYNYVSWYQQHPGKAPQLIIYDVTKRPSGVSNRFSGSNSGNTATLTISRVEAGDEADYYCQVWDSSSDHYVFGTGTKVTVL

SEQ ID NO: 469 - protein, 25 aa, Artificial Sequence
  H-FR1 of A56-03B03
QVQLVESGAEVKKPGSSVKVSCKTS

SEQ ID NO: 470 - protein, 17 aa, Artificial Sequence
  H-FR2 of A56-03B03
INWVRQAPGQGLEWMGS

SEQ ID NO: 471 - protein, 38 aa, Artificial Sequence
  H-FR3 of A56-03B03
NYAQKFQGRVTITADESTNTAFMELSSLGSEDTAVYYC

SEQ ID NO: 472 - protein, 11 aa, Artificial Sequence
  H-FR4 of A56-03B03
QGRGTLVTVSS

SEQ ID NO: 473 - protein, 25 aa, Artificial Sequence
  L-FR1 of A56-03B03
NFMLTQPASVSGSPGQSITISCTGS

SEQ ID NO: 474 - protein, 17 aa, Artificial Sequence
  L-FR2 of A56-03B03
VSWYQQHPGKAPQLIIY

SEQ ID NO: 475 - protein, 36 aa, Artificial Sequence
  L-FR3 of A56-03B03
IYDVTKRPSGVSNRFSGSNSGNTATLTISRVEAGDE

SEQ ID NO: 476 - protein, 10 aa, Artificial Sequence
  L-FR4 of A56-03B03
FGTGTKVTVL

SEQ ID NO: 477 - protein, 8 aa, Artificial Sequence
  H-CDR1 of A56-03D02
GFTFSSYA

SEQ ID NO: 478 - protein, 8 aa, Artificial Sequence
  H-CDR2 of A56-03D02
ISYDGSNK

SEQ ID NO: 479 - protein, 15 aa, Artificial Sequence
  H-CDR3 of A56-03D02
ARDAAAMISPHGMDV

SEQ ID NO: 480 - protein, 11 aa, Artificial Sequence
  L-CDR1 of A56-03D02
QSLVHSDGNIY

SEQ ID NO: 481 - protein, 3 aa, Artificial Sequence
  L-CDR2 of A56-03D02
KVS

SEQ ID NO: 482 - protein, 9 aa, Artificial Sequence
  L-CDR3 of A56-03D02
MQGTQWPPT

SEQ ID NO: 483 - DNA, 771 bp, Artificial Sequence
  SCFV of A56-03D02
cagatgcagctggtggagtctggaggaggcgtggtccagcctgggaggtccctgagactctcctgtgcagcctctggattcaccttcagtagctatgctatgcactgggtccgccaggctccaggcaaggggctggagtgggtggcagttatatcatatgatggaagtaataaatactacgcagactccgtgaagggccgattcaccatctccagagacaattccaagaacacgctgtatctgcaaatgaacagcctgagatctgaggacacggccgtgtattactgtgcgagagatgcggctgcgatgataagtccgcacggtatggacgtctggggccaagggaccacggtcaccgtctcctcaggcctcgggggcctcggaggaggaggtagtggcggaggaggctccggtggatccagcggtgtgggttccgatattgtgatgacccagtctccactctccctgcccgtcacccttggacagccggcctccatctcctgcaggtctagtcaaagcctcgtacacagtgatggaaacatctacttgaattggtttcaacagaggccaggccagtctcccaggcgcctaatttataaggtttctaacaggggctctggggtcccagacagattcagcggcagtgggtcaggcactgatttcacactggaaatcagcagggtggaggctgaggatgtagcggtttattactgcatgcaaggtacacagtggcctccgacttttggccaggggaccaagctggaaatcaaa

SEQ ID NO: 484 - protein, 122 aa, Artificial Sequence
  VH2 of A56-03D02
QMQLVESGGGVVQPGRSLRLSCAASGFTFSSYAMHWVRQAPGKGLEWVAVISYDGSNKYYADSVKGRFTISRDNSKNTLYLQMNSLRSEDTAVYYCARDAAAMISPHGMDVWGQGTTVTVSS

SEQ ID NO: 485 - protein, 112 aa, Artificial Sequence
  VL2 of A56-03D02
DIVMTQSPLSLPVTLGQPASISCRSSQSLVHSDGNIYLNWFQQRPGQSPRRLIYKVSNRGSGVPDRFSGSGSGTDFTLEISRVEAEDVAVYYCMQGTQWPPTFGQGTKLEIK

SEQ ID NO: 486 - protein, 25 aa, Artificial Sequence
  H-FR1 of A56-03D02
QMQLVESGGGVVQPGRSLRLSCAAS

SEQ ID NO: 487 - protein, 17 aa, Artificial Sequence
  H-FR2 of A56-03D02
MHWVRQAPGKGLEWVAV

SEQ ID NO: 488 - protein, 38 aa, Artificial Sequence
  H-FR3 of A56-03D02
YYADSVKGRFTISRDNSKNTLYLQMNSLRSEDTAVYYC

SEQ ID NO: 489 - protein, 11 aa, Artificial Sequence
  H-FR4 of A56-03D02
WGQGTTVTVSS

SEQ ID NO: 490 - protein, 26 aa, Artificial Sequence
  L-FR1 of A56-03D02
DIVMTQSPLSLPVTLGQPASISCRSS

SEQ ID NO: 491 - protein, 17 aa, Artificial Sequence
  L-FR2 of A56-03D02
LNWFQQRPGQSPRRLIY

SEQ ID NO: 492 - protein, 36 aa, Artificial Sequence
  L-FR3 of A56-03D02
IYKVSNRGSGVPDRFSGSGSGTDFTLEISRVEAEDV

SEQ ID NO: 493 - protein, 10 aa, Artificial Sequence
  L-FR4 of A56-03D02
FGQGTKLEIK

SEQ ID NO: 494 - protein, 8 aa, Artificial Sequence
  H-CDR1 of A56-03H11
GFTFSSYA

SEQ ID NO: 495 - protein, 8 aa, Artificial Sequence
  H-CDR2 of A56-03H11
ISYDGSNK

SEQ ID NO: 496 - protein, 16 aa, Artificial Sequence
  H-CDR3 of A56-03H11
TPFQHDSVPRRGAFDL

SEQ ID NO: 497 - protein, 12 aa, Artificial Sequence
  L-CDR1 of A56-03H11
QSLLSSSNNKNY

SEQ ID NO: 498 - protein, 3 aa, Artificial Sequence
  L-CDR2 of A56-03H11
WAS

SEQ ID NO: 499 - protein, 9 aa, Artificial Sequence
  L-CDR3 of A56-03H11
QQYYTSPRT

SEQ ID NO: 500 - DNA, 777 bp, Artificial Sequence
  SCFV of A56-03H11
caggtgcagctggtggagtctgggggaggcgtggtccagcctgggaggtccctgagactctcctgtgcagcctctggattcaccttcagtagctatgctatgcactgggtccgccaggctccaggcaaggggctggagtgggtggcagttatatcatatgatggaagtaataaatactacgcagactccgtgaagggccgattcaccatctccagagacaattccaagaacacgctgtatctgcaaatgaacagtctgagagccgaggacacggccgtgtattactgtactccatttcaacatgatagtgttccgcgccgtggtgcttttgatctctggggccaagggacaaagatcaccgtctcctcaggcctcgggggcctcggaggaggaggtagtggcggaggaggctccggtggatccagcggtgtgggttccgacatccagatgacccagtctccatcctccctggctgtgtctctgggcgagagggccaccatcaactgcaagtccagccagagtcttttatccagctccaacaataagaactacttagcttggtaccaacacaagccaggacagcctcctaagcttctcatttactgggcatctacccgggaatccggggtccctgaccgattcagtggcagcgggtctgggacagatttcactctcaccatcagcagcctgcaggctgaagatgtggcagtttattactgtcagcaatattatacttctcctcggacgttcggccaagggaccaaggtggaaatcaaa

SEQ ID NO: 501 - protein, 123 aa, Artificial Sequence
  VH2 of A56-03H11
QVQLVESGGGVVQPGRSLRLSCAASGFTFSSYAMHWVRQAPGKGLEWVAVISYDGSNKYYADSVKGRFTISRDNSKNTLYLQMNSLRAEDTAVYYCTPFQHDSVPRRGAFDLWGQGTKITVSS

SEQ ID NO: 502 - protein, 113 aa, Artificial Sequence
  VL2 of A56-03H11
DIQMTQSPSSLAVSLGERATINCKSSQSLLSSSNNKNYLAWYQHKPGQPPKLLIYWASTRESGVPDRFSGSGSGTDFTLTISSLQAEDVAVYYCQQYYTSPRTFGQGTKVEIK

SEQ ID NO: 503 - protein, 25 aa, Artificial Sequence
  H-FR1 of A56-03H11
QVQLVESGGGVVQPGRSLRLSCAAS

SEQ ID NO: 504 - protein, 17 aa, Artificial Sequence
  H-FR2 of A56-03H11
MHWVRQAPGKGLEWVAV

SEQ ID NO: 505 - protein, 38 aa, Artificial Sequence
  H-FR3 of A56-03H11
YYADSVKGRFTISRDNSKNTLYLQMNSLRAEDTAVYYC

SEQ ID NO: 506 - protein, 11 aa, Artificial Sequence
  H-FR4 of A56-03H11
WGQGTKITVSS

SEQ ID NO: 507 - protein, 26 aa, Artificial Sequence
  L-FR1 of A56-03H11
DIQMTQSPSSLAVSLGERATINCKSS

SEQ ID NO: 508 - protein, 17 aa, Artificial Sequence
  L-FR2 of A56-03H11
LAWYQHKPGQPPKLLIY

SEQ ID NO: 509 - protein, 36 aa, Artificial Sequence; identical to SEQ ID NO: 288
  L-FR3 of A56-03H11

SEQ ID NO: 510 - protein, 10 aa, Artificial Sequence
  L-FR4 of A56-03H11
FGQGTKVEIK

SEQ ID NO: 511 - protein, 8 aa, Artificial Sequence
  H-CDR1 of A56-07A09
GGTFTRDA

SEQ ID NO: 512 - protein, 8 aa, Artificial Sequence
  H-CDR2 of A56-07A09
IIPLIDTA

SEQ ID NO: 513 - protein, 17 aa, Artificial Sequence
  H-CDR3 of A56-07A09
ARGEMYSRSWYWGAFDL

SEQ ID NO: 514 - protein, 9 aa, Artificial Sequence
  L-CDR1 of A56-07A09
SSDVGGYNY

SEQ ID NO: 515 - protein, 3 aa, Artificial Sequence
  L-CDR2 of A56-07A09
DVT

SEQ ID NO: 516 - protein, 10 aa, Artificial Sequence
  L-CDR3 of A56-07A09
SSYSSSTFYV

SEQ ID NO: 517 - DNA, 771 bp, Artificial Sequence
  SCFV of A56-07A09
caggtgcagctggtagagtctggggctgaggtgaagaagcctgggtcttcggtgaaggtctcctgcaaggtttctggaggcaccttcaccagggatgctatcagttgggtgcgacaggcccctggacaagggcttgagtggatgggaaggatcatccctctcattgatacagcaaattacgcacagaagttccagggcagagtcacgattaccgcggacaaatccacgagcacagcctacatgagtctaagcagcctgggatctgaggacacggccgtgtattactgtgcgagaggcgagatgtatagcaggagctggtactggggggcttttgatctctggggccaagggacaatggtcaccgtctcctcaggcctcgggggcctcggaggaggaggtagtggcggaggaggctccggtggatccagcggtgtgggttccaattttatgctgactcagcccgcctccgtgtctgggtcccctggacagtcgatcaccatctcctgcactggaagcagcagcgacgttggtggttataactatgtctcctggtaccaacagcacccaggcaaagccccccaactcatcatttatgatgtcactaagcggccctcaggggtttctaatcgcttctccggctccaagtctggcaactcggcctccctgactatctctggactccaggctgaggacgaggctgattattactgcagctcatacagcagcagcactttttacgtcttcggaactgggaccaaggtcaccgtccta

SEQ ID NO: 518 - protein, 124 aa, Artificial Sequence
  VH2 of A56-07A09
QVQLVESGAEVKKPGSSVKVSCKVSGGTFTRDAISWVRQAPGQGLEWMGRIIPLIDTANYAQKFQGRVTITADKSTSTAYMSLSSLGSEDTAVYYCARGEMYSRSWYWGAFDLWGQGTMVTVSS

SEQ ID NO: 519 - protein, 110 aa, Artificial Sequence
  VL2 of A56-07A09
NFMLTQPASVSGSPGQSITISCTGSSSDVGGYNYVSWYQQHPGKAPQLIIYDVTKRPSGVSNRFSGSKSGNSASLTISGLQAEDEADYYCSSYSSSTFYVFGTGTKVTVL

SEQ ID NO: 520 - protein, 25 aa, Artificial Sequence
  H-FR1 of A56-07A09
QVQLVESGAEVKKPGSSVKVSCKVS

SEQ ID NO: 521 - protein, 17 aa, Artificial Sequence
  H-FR2 of A56-07A09
ISWVRQAPGQGLEWMGR

SEQ ID NO: 522 - protein, 38 aa, Artificial Sequence
  H-FR3 of A56-07A09
NYAQKFQGRVTITADKSTSTAYMSLSSLGSEDTAVYYC

SEQ ID NO: 523 - protein, 11 aa, Artificial Sequence
  H-FR4 of A56-07A09
WGQGTMVTVSS

SEQ ID NO: 524 - protein, 25 aa, Artificial Sequence
  L-FR1 of A56-07A09
NFMLTQPASVSGSPGQSITISCTGS

SEQ ID NO: 525 - protein, 17 aa, Artificial Sequence
  L-FR2 of A56-07A09
VSWYQQHPGKAPQLIIY

SEQ ID NO: 526 - protein, 36 aa, Artificial Sequence; identical to SEQ ID NO: 152
  L-FR3 of A56-07A09

SEQ ID NO: 527 - protein, 10 aa, Artificial Sequence
  L-FR4 of A56-07A09
FGTGTKVTVL

SEQ ID NO: 528 - protein, 8 aa, Artificial Sequence
  H-CDR1 of A56-08A01
GFSFSNYG

SEQ ID NO: 529 - protein, 8 aa, Artificial Sequence
  H-CDR2 of A56-08A01
VSFDGIKK

SEQ ID NO: 530 - protein, 17 aa, Artificial Sequence
  H-CDR3 of A56-08A01
AKAPVYCSGDCRFAFDF

SEQ ID NO: 531 - protein, 11 aa, Artificial Sequence
  L-CDR1 of A56-08A01
QSLLHSDGKTY

SEQ ID NO: 532 - protein, 3 aa, Artificial Sequence
  L-CDR2 of A56-08A01
EVS

SEQ ID NO: 533 - protein, 6 aa, Artificial Sequence
  L-CDR3 of A56-08A01
MQGSYT

SEQ ID NO: 534 - DNA, 768 bp, Artificial Sequence
  SCFV of A56-08A01
caggtgcagctggtggagtcagggggaggcgtggtccagcctgggaggtccctgagactctcctgtgcagcctctggattcagtttcagtaattatggcatgcactgggtccgccaggctccaggcaaggggctgcagtgggtggcaaccgtctcttttgatggaataaaaaaacattattcagactccgtgaagggccgtttcaccatctccagagacaattccaagaacacgctgtatctccaaatgaacagtctgagagccgaggacacggccgtgtattactgtgcgaaagctcccgtctattgtagtggtgactgccgttttgcatttgatttctggggcctagggacaacggtcaccgtctcctcaggcctcgggggcctcggaggaggaggtagtggcggaggaggctccggtggatccagcggtgtgggttccgatattgtgatgacccagactccactctctctgtccgtcacccctggacagtcggcctccatctcctgcaagtctagtcagagcctcctgcatagtgatggaaagacctatttgtattggtacttgcagaggccaggccagtctccacaactcctgatctatgaagtttccaaccggttctctggagtgccagataggttcagtggcagcgggtcagggacagatttcacactgaatatcagccgggtggaggctgaggatgttgggatttattactgcatgcaaggttcgtacacttttggccaggggaccaaggtagatatcaaa

SEQ ID NO: 535 - protein, 124 aa, Artificial Sequence
  VH2 of A56-08A01
QVQLVESGGGVVQPGRSLRLSCAASGFSFSNYGMHWVRQAPGKGLQWVATVSFDGIKKHYSDSVKGRFTISRDNSKNTLYLQMNSLRAEDTAVYYCAKAPVYCSGDCRFAFDFWGLGTTVTVSS

SEQ ID NO: 536 - protein, 109 aa, Artificial Sequence
  VL2 of A56-08A01
DIVMTQTPLSLSVTPGQSASISCKSSQSLLHSDGKTYLYWYLQRPGQSPQLLIYEVSNRFSGVPDRFSGSGSGTDFTLNISRVEAEDVGIYYCMQGSYTFGQGTKVDIK

SEQ ID NO: 537 - protein, 25 aa, Artificial Sequence
  H-FR1 of A56-08A01
QVQLVESGGGVVQPGRSLRLSCAAS

SEQ ID NO: 538 - protein, 17 aa, Artificial Sequence
  H-FR2 of A56-08A01
MHWVRQAPGKGLQWVAT

SEQ ID NO: 539 - protein, 38 aa, Artificial Sequence
  H-FR3 of A56-08A01
HYSDSVKGRFTISRDNSKNTLYLQMNSLRAEDTAVYYC

SEQ ID NO: 540 - protein, 11 aa, Artificial Sequence
  H-FR4 of A56-08A01
WGLGTTVTVSS

SEQ ID NO: 541 - protein, 26 aa, Artificial Sequence
  L-FR1 of A56-08A01
DIVMTQTPLSLSVTPGQSASISCKSS

SEQ ID NO: 542 - protein, 17 aa, Artificial Sequence
  L-FR2 of A56-08A01
LYWYLQRPGQSPQLLIY

SEQ ID NO: 543 - protein, 36 aa, Artificial Sequence
  L-FR3 of A56-08A01
IYEVSNRFSGVPDRFSGSGSGTDFTLNISRVEAEDV

SEQ ID NO: 544 - protein, 10 aa, Artificial Sequence
  L-FR4 of A56-08A01
FGQGTKVDIK

SEQ ID NO: 545 - protein, 8 aa, Artificial Sequence
  H-CDR1 of A56-10A01
GYTFTHYD

SEQ ID NO: 546 - protein, 8 aa, Artificial Sequence
  H-CDR2 of A56-10A01
MNPNKGNT

SEQ ID NO: 547 - protein, 20 aa, Artificial Sequence
  H-CDR3 of A56-10A01
ARERVPNAMVGYFSFYGMDV

SEQ ID NO: 548 - protein, 6 aa, Artificial Sequence
  L-CDR1 of A56-10A01
DITRKS

SEQ ID NO: 549 - protein, 3 aa, Artificial Sequence
  L-CDR2 of A56-10A01
YDR

SEQ ID NO: 550 - protein, 9 aa, Artificial Sequence
  L-CDR3 of A56-10A01
QVWDTNSVV

SEQ ID NO: 551 - DNA, 768 bp, Artificial Sequence
  SCFV of A56-10A01
caggtgcagctggtgcagtctggggctgaggtgaagaagcctggggcctcagtgaaggtctcctgcaagacctctggatacaccttcacccattatgatatcaactgggtgcgacaggcctctggacaagggcttgagtggatgggacggatgaacccgaataagggaaacacaggctatgctcagaagttccagggcagagtcaccatgaccagggacgcctcgacagacacagcctacatggagctgagcagcctgagatctgaggacacggccgtgtattactgtgcgcgagaaagagtaccgaatgctatggtgggttacttctccttctacgggatggacgtctggggccaagggaccacggtcaccgtctcctcaggcctcgggggcctcggaggaggaggtagtggcggaggaggctccggtggatccagcggtgtgggttcctcctatgagctgactcaggcaccctcattgtcagtggccccaggagagacggccactattacctgtgggggaaacgacattacaagaaagagtgtgcactggtaccagcagaggccaggccaggcccctgtgctggtcatctattatgatagagcccggccctcagggatccctgagcgattctctggctccaactctgagaacacggccagcctgaccatcagcagggtcgaggccggggatgaggccgactattactgtcaggtgtgggatactaatagtgtggtttttggcggagggaccaagctgaccgtccta

SEQ ID NO: 552 - protein, 127 aa, Artificial Sequence
  VH2 of A56-10A01
QVQLVQSGAEVKKPGASVKVSCKTSGYTFTHYDINWVRQASGQGLEWMGRMNPNKGNTGYAQKFQGRVTMTRDASTDTAYMELSSLRSEDTAVYYCARERVPNAMVGYFSFYGMDVWGQGTTVTVSS

SEQ ID NO: 553 - protein, 106 aa, Artificial Sequence
  VL2 of A56-10A01
SYELTQAPSLSVAPGETATITCGGNDITRKSVHWYQQRPGQAPVLVIYYDRARPSGIPERFSGSNSENTASLTISRVEAGDEADYYCQVWDTNSVVFGGGTKLTVL

SEQ ID NO: 554 - protein, 25 aa, Artificial Sequence
  H-FR1 of A56-10A01
QVQLVQSGAEVKKPGASVKVSCKTS

SEQ ID NO: 555 - protein, 17 aa, Artificial Sequence
  H-FR2 of A56-10A01
INWVRQASGQGLEWMGR

SEQ ID NO: 556 - protein, 38 aa, Artificial Sequence
  H-FR3 of A56-10A01
GYAQKFQGRVTMTRDASTDTAYMELSSLRSEDTAVYYC

SEQ ID NO: 557 - protein, 11 aa, Artificial Sequence
  H-FR4 of A56-10A01
WGQGTTVTVSS

SEQ ID NO: 558 - protein, 25 aa, Artificial Sequence
  L-FR1 of A56-10A01
SYELTQAPSLSVAPGETATITCGGN

SEQ ID NO: 559 - protein, 17 aa, Artificial Sequence
  L-FR2 of A56-10A01
VHWYQQRPGQAPVLVIY

SEQ ID NO: 560 - protein, 36 aa, Artificial Sequence
  L-FR3 of A56-10A01
IYYDRARPSGIPERFSGSNSENTASLTISRVEAGDE

SEQ ID NO: 561 - protein, 10 aa, Artificial Sequence
  L-FR4 of A56-10A01
FGGGTKLTVL

SEQ ID NO: 562 - protein, 8 aa, Artificial Sequence
  H-CDR1 of A56-11B10
GFTFANAW

SEQ ID NO: 563 - protein, 10 aa, Artificial Sequence
  H-CDR2 of A56-11B10
IYSTSDGGAT

SEQ ID NO: 564 - protein, 24 aa, Artificial Sequence
  H-CDR3 of A56-11B10
AKDRGMDNIHTGQNSGWSFGWFDP

SEQ ID NO: 565 - protein, 9 aa, Artificial Sequence
  L-CDR1 of A56-11B10
SSDVGGYNY

SEQ ID NO: 566 - protein, 3 aa, Artificial Sequence
  L-CDR2 of A56-11B10
DVT

SEQ ID NO: 567 - protein, 10 aa, Artificial Sequence
  L-CDR3 of A56-11B10
SSYAGSYTSV

SEQ ID NO: 568 - DNA, 798 bp, Artificial Sequence
  SCFV of A56-11B10
caggtgcagctggtggagtctgggggaggcttggtaaagcctggggagtctcttagactctcctgtgaagcctctggtttcactttcgctaacgcctggatgagttggttccgccaggcgccagggaaggggctggagtgggttggccgtatttatagcacatctgatggtggagccacagactacgctgctcccgttgagggccgatttaccatctccagagatgactcaaaaaacacgctgtttctgcaaatgaacagtctgagagccgaggacacggccgtgtattactgtgcgaaagatcggggcatggataacattcacacgggtcagaacagtggctggtcgtttggttggttcgacccctggggccagggaaccctggtcaccgtctcctcaggcctcgggggcctcggaggaggaggtagtggcggaggaggctccggtggatccagcggtgtgggttcccagtctgccctgactcagcctcgctcagtgtccgggtctcctggacagtcagtcaccatctcctgcactggaaccagcagtgatgttggtggttataactatgtctcctggtaccaacagcacccaggcaaagcccccaaactcatgatttatgatgtcactaagcggccctcaggggtccctgatcgcttctctggctccaagtctggcaacacggcctccctgaccatctctgggctccaggctgaggatgaggctgattattactgcagctcatatgcaggcagctacacttctgtcttcggaactgggaccaaggtcaccgtccta

SEQ ID NO: 569 - protein, 133 aa, Artificial Sequence
  VH2 of A56-11B10
QVQLVESGGGLVKPGESLRLSCEASGFTFANAWMSWFRQAPGKGLEWVGRIYSTSDGGATDYAAPVEGRFTISRDDSKNTLFLQMNSLRAEDTAVYYCAKDRGMDNIHTGQNSGWSFGWFDPWGQGTLVTVSS

SEQ ID NO: 570 - protein, 110 aa, Artificial Sequence
  VL2 of A56-11B10
QSALTQPRSVSGSPGQSVTISCTGTSSDVGGYNYVSWYQQHPGKAPKLMIYDVTKRPSGVPDRFSGSKSGNTASLTISGLQAEDEADYYCSSYAGSYTSVFGTGTKVTVL

SEQ ID NO: 571 - protein, 25 aa, Artificial Sequence
  H-FR1 of A56-11B10
QVQLVESGGGLVKPGESLRLSCEAS

SEQ ID NO: 572 - protein, 17 aa, Artificial Sequence
  H-FR2 of A56-11B10
MSWFRQAPGKGLEWVGR

SEQ ID NO: 573 - protein, 38 aa, Artificial Sequence
  H-FR3 of A56-11B10
DYAAPVEGRFTISRDDSKNTLFLQMNSLRAEDTAVYYC

SEQ ID NO: 574 - protein, 11 aa, Artificial Sequence
  H-FR4 of A56-11B10
WGQGTLVTVSS

SEQ ID NO: 575 - protein, 25 aa, Artificial Sequence
  L-FR1 of A56-11B10
QSALTQPRSVSGSPGQSVTISCTGT

SEQ ID NO: 576 - protein, 17 aa, Artificial Sequence
  L-FR2 of A56-11B10
VSWYQQHPGKAPKLMIY

SEQ ID NO: 577 - protein, 36 aa, Artificial Sequence
  L-FR3 of A56-11B10
IYDVTKRPSGVPDRFSGSKSGNTASLTISGLQAEDE

SEQ ID NO: 578 - protein, 10 aa, Artificial Sequence
  L-FR4 of A56-11B10
FGTGTKVTVL

SEQ ID NO: 579 - protein, 8 aa, Artificial Sequence
  H-CDR1 of A56-11C04
GFTVSNAW

SEQ ID NO: 580 - protein, 10 aa, Artificial Sequence
  H-CDR2 of A56-11C04
IKSKTDGGTT

SEQ ID NO: 581 - protein, 11 aa, Artificial Sequence
  H-CDR3 of A56-11C04
AKDPDAENTGA

SEQ ID NO: 582 - protein, 6 aa, Artificial Sequence
  L-CDR1 of A56-11C04
DIGSKS

SEQ ID NO: 583 - protein, 3 aa, Artificial Sequence
  L-CDR2 of A56-11C04
SDS

SEQ ID NO: 584 - protein, 12 aa, Artificial Sequence
  L-CDR3 of A56-11C04
QVWDNGSDHPGV

SEQ ID NO: 585 - DNA, 756 bp, Artificial Sequence
  SCFV of A56-11C04
caggtgcagctggtacagtcggggggaggcttggtaaagcctggggggtcccttagactctcctgtgcagtcagtggattcactgtcagtaatgcctggatgatgtggttccgccaggtaccagggaaggggctggagtgggttggccgtattaaaagcaaaactgatggtgggacaacagagtacgctgcacccgtgaaaggcagattcagcatctcaggagacgactcaaaaaacacactgtatctccaaatgaacagtctgagagccgaggacacggccgtgtattactgtgcaaaagatccagacgccgagaatacaggggcactgggccagggaaccctggtcaccgtctcctcaggcctcgggggcctcggaggaggaggtagtggcggaggaggctccggtggatccagcggtgtgggttccaattttatgctgactcagcccccctcagtgtcagtggccccaggaaagacggccgggattacctgtgggggagacgacattggaagtaaaagtgtgcattggtaccagcagaggccaggccaggcccctgtcctggtcatctcttccgatagcgaccggccctcagggatccctgagcgattctctggctccaattctgggaacacggccaccctgaccatcaccagagtcgaagacggggatgaggccgactattactgtcaggtgtgggataatggtagtgatcatcccggggtcttcggaactgggaccaaggtcaccgtccta

SEQ ID NO: 586 - protein, 120 aa, Artificial Sequence
  VH2 of A56-11C04
QVQLVQSGGGLVKPGGSLRLSCAVSGFTVSNAWMMWFRQVPGKGLEWVGRIKSKTDGGTTEYAAPVKGRFSISGDDSKNTLYLQMNSLRAEDTAVYYCAKDPDAENTGALGQGTLVTVSS

SEQ ID NO: 587 - protein, 109 aa, Artificial Sequence
  VL2 of A56-11C04
NFMLTQPPSVSVAPGKTAGITCGGDDIGSKSVHWYQQRPGQAPVLVISSDSDRPSGIPERFSGSNSGNTATLTITRVEDGDEADYYCQVWDNGSDHPGVFGTGTKVTVL

SEQ ID NO: 588 - protein, 25 aa, Artificial Sequence
  H-FR1 of A56-11C04
QVQLVQSGGGLVKPGGSLRLSCAVS

SEQ ID NO: 589 - protein, 17 aa, Artificial Sequence
  H-FR2 of A56-11C04
MMWFRQVPGKGLEWVGR

SEQ ID NO: 590 - protein, 38 aa, Artificial Sequence
  H-FR3 of A56-11C04
EYAAPVKGRFSISGDDSKNTLYLQMNSLRAEDTAVYYC

SEQ ID NO: 591 - protein, 11 aa, Artificial Sequence
  H-FR4 of A56-11C04
LGQGTLVTVSS

SEQ ID NO: 592 - protein, 25 aa, Artificial Sequence
  L-FR1 of A56-11C04
NFMLTQPPSVSVAPGKTAGITCGGD

SEQ ID NO: 593 - protein, 17 aa, Artificial Sequence
  L-FR2 of A56-11C04
VHWYQQRPGQAPVLVIS

SEQ ID NO: 594 - protein, 36 aa, Artificial Sequence
  L-FR3 of A56-11C04
ISSDSDRPSGIPERFSGSNSGNTATLTITRVEDGDE

SEQ ID NO: 595 - protein, 10 aa, Artificial Sequence
  L-FR4 of A56-11C04
FGTGTKVTVL

SEQ ID NO: 596 - protein, 8 aa, Artificial Sequence
  H-CDR1 of A56-15A01
GFTFTKYT

SEQ ID NO: 597 - protein, 8 aa, Artificial Sequence
  H-CDR2 of A56-15A01
ISYDGSNK

SEQ ID NO: 598 - protein, 16 aa, Artificial Sequence
  H-CDR3 of A56-15A01
TPFQHDSVPRRGAFDL

SEQ ID NO: 599 - protein, 9 aa, Artificial Sequence
  L-CDR1 of A56-15A01
SSDVGGYNY

SEQ ID NO: 600 - protein, 3 aa, Artificial Sequence
  L-CDR2 of A56-15A01
DVD

SEQ ID NO: 601 - protein, 11 aa, Artificial Sequence
  L-CDR3 of A56-15A01
SSSRPSSTPRV

SEQ ID NO: 602 - DNA, 771 bp, Artificial Sequence
  SCFV of A56-15A01
cagatgcagctggtggagtctgggggaggcgtggtccagcctggggggtccctgagactctcctgtgcagcctctggattcaccttcactaaatatactatgctctgggtccgccaggctccaggcaaggggctggagtgggtggcacttatatcatatgatggaagcaacaaaaattacgcagattccgtgaagggccgattcaccatttcccgagacgattccaagagcacgctatttctgcaaatgagcagcctgagatctgaggacacggccgtgtattactgtactccatttcaacatgatagtgttccgcgccgtggtgcttttgatctctggggccaagggacaatggtcaccgtctcctcaggcctcgggggcctcggaggaggaggtagtggcggaggaggctccggtggatccagcggtgtgggttcccagtctgccctgactcagcctgcctccgtgtctgggtctcctggacagtcgatcgccatctcctgcactgggactagcagtgacgttggtggttataactatgtctcctggtaccaacaacacccaggcaaagcccccaaactcgtgatttatgatgttgataagcggccctcaggggtttctaatcgcttctctggctccaagtctgccaacacggcctccctgaccatctctgggctccaggctgacgacgaggctgattattactgcagctcatctagacccagcagcactcctcgggtcttcggaactgggaccaaggtcaccgtccta

SEQ ID NO: 603 - protein, 123 aa, Artificial Sequence
  VH2 of A56-15A01
QMQLVESGGGVVQPGGSLRLSCAASGFTFTKYTMLWVRQAPGKGLEWVALISYDGSNKNYADSVKGRFTISRDDSKSTLFLQMSSLRSEDTAVYYCTPFQHDSVPRRGAFDLWGQGTMVTVSS

SEQ ID NO: 604 - protein, 111 aa, Artificial Sequence
  VL2 of A56-15A01
QSALTQPASVSGSPGQSIAISCTGTSSDVGGYNYVSWYQQHPGKAPKLVIYDVDKRPSGVSNRFSGSKSANTASLTISGLQADDEADYYCSSSRPSSTPRVFGTGTKVTVL

SEQ ID NO: 605 - protein, 25 aa, Artificial Sequence
  H-FR1 of A56-15A01
QMQLVESGGGVVQPGGSLRLSCAAS

SEQ ID NO: 606 - protein, 17 aa, Artificial Sequence
  H-FR2 of A56-15A01
MLWVRQAPGKGLEWVAL

SEQ ID NO: 607 - protein, 38 aa, Artificial Sequence
  H-FR3 of A56-15A01
NYADSVKGRFTISRDDSKSTLFLQMSSLRSEDTAVYYC

SEQ ID NO: 608 - protein, 11 aa, Artificial Sequence
  H-FR4 of A56-15A01
WGQGTMVTVSS

SEQ ID NO: 609 - protein, 25 aa, Artificial Sequence
  L-FR1 of A56-15A01
QSALTQPASVSGSPGQSIAISCTGT

SEQ ID NO: 610 - protein, 17 aa, Artificial Sequence
  L-FR2 of A56-15A01
VSWYQQHPGKAPKLVIY

SEQ ID NO: 611 - protein, 36 aa, Artificial Sequence
  L-FR3 of A56-15A01
IYDVDKRPSGVSNRFSGSKSANTASLTISGLQADDE

SEQ ID NO: 612 - protein, 10 aa, Artificial Sequence
  L-FR4 of A56-15A01
FGTGTKVTVL

SEQ ID NO: 613 - protein, 8 aa, Artificial Sequence
  H-CDR1 of A56-16E02
GIAFSRYA

SEQ ID NO: 614 - protein, 7 aa, Artificial Sequence
  H-CDR2 of A56-16E02
IGSTGTT

SEQ ID NO: 615 - protein, 9 aa, Artificial Sequence
  H-CDR3 of A56-16E02
ATHFGFFSK

SEQ ID NO: 616 - protein, 11 aa, Artificial Sequence
  L-CDR1 of A56-16E02
QSLLHRNGYNY

SEQ ID NO: 617 - protein, 3 aa, Artificial Sequence
  L-CDR2 of A56-16E02
LGS

SEQ ID NO: 618 - protein, 9 aa, Artificial Sequence
  L-CDR3 of A56-16E02
MQALETRWT

SEQ ID NO: 619 - DNA, 750 bp, Artificial Sequence
  SCFV of A56-16E02
caggtgcagctggtggagtctgggggagacttggtacagcctggggggtccctgagactctcctgtgtagactctggaatcgcctttagcagatatgccatgaactgggtccgccaggctccagggaaggggctggagtgggtctcaagtattggtagtactggtaccacatactacgcagactccgtgaagggccggttcaccatctccagagacagatccaagaacacgctgtatctgcaaatgaacagtctgagagccgaggacacggccgtgtattactgtgccacacactttggattctttagcaagtggggccagggaaccctggtcaccgtctcctcaggcctcgggggcctcggaggaggaggtagtggcggaggaggctccggtggatccagcggtgtgggttccgatattgtgatgacccagactccactctccctgcccgtcacccctggagagccggcctccatctcctgcaggtctagtcagagcctcctgcatagaaatggatacaattatttggattggtacctgcagaagccagggcagtctccacagctcctgatctatctgggttctaatcgggcctccggggtccctgacaggttcagtggcagtggatcaggcacagatttcacactgaatatcagcagagtggaggctgaggatgttggggtttattattgcatgcaagcccttgaaactcggtggacgttcggccaagggaccaaggtggatatcaaa

SEQ ID NO: 620 - protein, 115 aa, Artificial Sequence
  VH2 of A56-16E02
QVQLVESGGDLVQPGGSLRLSCVDSGIAFSRYAMNWVRQAPGKGLEWVSSIGSTGTTYYADSVKGRFTISRDRSKNTLYLQMNSLRAEDTAVYYCATHFGFFSKWGQGTLVTVSS

SEQ ID NO: 621 - protein, 112 aa, Artificial Sequence
  VL2 of A56-16E02
DIVMTQTPLSLPVTPGEPASISCRSSQSLLHRNGYNYLDWYLQKPGQSPQLLIYLGSNRASGVPDRFSGSGSGTDFTLNISRVEAEDVGVYYCMQALETRWTFGQGTKVDIK

SEQ ID NO: 622 - protein, 25 aa, Artificial Sequence
  H-FR1 of A56-16E02
QVQLVESGGDLVQPGGSLRLSCVDS

SEQ ID NO: 623 - protein, 17 aa, Artificial Sequence
  H-FR2 of A56-16E02
MNWVRQAPGKGLEWVSS

SEQ ID NO: 624 - protein, 38 aa, Artificial Sequence
  H-FR3 of A56-16E02
YYADSVKGRFTISRDRSKNTLYLQMNSLRAEDTAVYYC

SEQ ID NO: 625 - protein, 11 aa, Artificial Sequence
  H-FR4 of A56-16E02
WGQGTLVTVSS

SEQ ID NO: 626 - protein, 26 aa, Artificial Sequence
  L-FR1 of A56-16E02
DIVMTQTPLSLPVTPGEPASISCRSS

SEQ ID NO: 627 - protein, 17 aa, Artificial Sequence
  L-FR2 of A56-16E02
LDWYLQKPGQSPQLLIY

SEQ ID NO: 628 - protein, 36 aa, Artificial Sequence
  L-FR3 of A56-16E02
IYLGSNRASGVPDRFSGSGSGTDFTLNISRVEAEDV

SEQ ID NO: 629 - protein, 10 aa, Artificial Sequence
  L-FR4 of A56-16E02
FGQGTKVDIK

SEQ ID NO: 630 - protein, 8 aa, Artificial Sequence
  H-CDR1 of A56-18C03
GGTLSSYP

SEQ ID NO: 631 - protein, 8 aa, Artificial Sequence
  H-CDR2 of A56-18C03
INPNGGAT

SEQ ID NO: 632 - protein, 9 aa, Artificial Sequence
  H-CDR3 of A56-18C03
AQLGSSGGG

SEQ ID NO: 633 - protein, 6 aa, Artificial Sequence
  L-CDR1 of A56-18C03
SLRKYH

SEQ ID NO: 634 - protein, 3 aa, Artificial Sequence
  L-CDR2 of A56-18C03
GKN

SEQ ID NO: 635 - protein, 12 aa, Artificial Sequence
  L-CDR3 of A56-18C03
NSRDSSGNDLRV

SEQ ID NO: 636 - DNA, 744 bp, Artificial Sequence
  SCFV of A56-18C03
caggtgcagctggtggagtctggggctgaggtgaagaagcctgggtcctcggtgaaggtctcctgcaagacttctggaggcactttaagcagttatcccatcacctgggtgcgacaggcccctggacaagggcctgagtggatgggaattatcaaccccaatggtggcgccacaaactacgcacagaagttccagggcagagtcaccatgaccagggacacgtccacgggcacagtctacatggaactgagcagcctgagatctgaggacacggccgtgtattactgtgcgcagttgggtagcagtggagggggtttgggccagggaaccctggtcaccgtctcctcaggcctcgggggcctcggaggaggaggtagtggcggaggaggctccggtggatccagcggtgtgggttcctcctatgagctgacacaggaccctgctgtgtctgtggccttgggacagacagtcaggatcacatgccaaggagacagcctcagaaaatatcatgcaagctggtaccagcagaagccaggacaggcccctgtacttgtcatctatggtaaaaacaaccggccctcagggatcccaggccgattctctggctccagctcaggaaacacagcttccttgaccatcactggggctcaggcggaagatgaggctgactattactgtaactcccgggacagcagtggtaacgatctcagggtgttcggcggagggaccaagctgaccgtccta

SEQ ID NO: 637 - protein, 116 aa, Artificial Sequence
  VH2 of A56-18C03
QVQLVESGAEVKKPGSSVKVSCKTSGGTLSSYPITWVRQAPGQGPEWMGIINPNGGATNYAQKFQGRVTMTRDTSTGTVYMELSSLRSEDTAVYYCAQLGSSGGGLGQGTLVTVSS

SEQ ID NO: 638 - protein, 109 aa, Artificial Sequence
  VL2 of A56-18C03
SYELTQDPAVSVALGQTVRITCQGDSLRKYHASWYQQKPGQAPVLVIYGKNNRPSGIPGRFSGSSSGNTASLTITGAQAEDEADYYCNSRDSSGNDLRVFGGGTKLTVL

SEQ ID NO: 639 - protein, 25 aa, Artificial Sequence
  H-FR1 of A56-18C03
QVQLVESGAEVKKPGSSVKVSCKTS

SEQ ID NO: 640 - protein, 17 aa, Artificial Sequence
  H-FR2 of A56-18C03
ITWVRQAPGQGPEWMGI

SEQ ID NO: 641 - protein, 38 aa, Artificial Sequence
  H-FR3 of A56-18C03
NYAQKFQGRVTMTRDTSTGTVYMELSSLRSEDTAVYYC

SEQ ID NO: 642 - protein, 11 aa, Artificial Sequence
  H-FR4 of A56-18C03
LGQGTLVTVSS

SEQ ID NO: 643 - protein, 25 aa, Artificial Sequence
  L-FR1 of A56-18C03
SYELTQDPAVSVALGQTVRITCQGD

SEQ ID NO: 644 - protein, 17 aa, Artificial Sequence
  L-FR2 of A56-18C03
ASWYQQKPGQAPVLVIY

SEQ ID NO: 645 - protein, 36 aa, Artificial Sequence
  L-FR3 of A56-18C03
IYGKNNRPSGIPGRFSGSSSGNTASLTITGAQAEDE

SEQ ID NO: 646 - protein, 10 aa, Artificial Sequence
  L-FR4 of A56-18C03
FGGGTKLTVL

SEQ ID NO: 647 - protein, 8 aa, Artificial Sequence
  H-CDR1 of A56-18G02
GFTFSSYG

SEQ ID NO: 648 - protein, 8 aa, Artificial Sequence
  H-CDR2 of A56-18G02
ISYDGSNK

SEQ ID NO: 649 - protein, 15 aa, Artificial Sequence
  H-CDR3 of A56-18G02
ARMRWAVAGMGAFEI

SEQ ID NO: 650 - protein, 7 aa, Artificial Sequence
  L-CDR1 of A56-18G02
QSVTSSY

SEQ ID NO: 651 - protein, 3 aa, Artificial Sequence
  L-CDR2 of A56-18G02
GAS

SEQ ID NO: 652 - protein, 10 aa, Artificial Sequence
  L-CDR3 of A56-18G02
QQRSSWPPLT

SEQ ID NO: 653 - DNA, 762 bp, Artificial Sequence
  SCFV of A56-18G02
cagatgcagctggtgcagtctgggggaggcgtggtccagcctgggaggtccctgagactctcctgtgcagcctctggattcaccttcagtagctatggcatgcactgggtccgccaggctccaggcaaggggctggagtgggtggcagttatatcatatgatggaagtaataaatactatgcagactccgtgaagggccgattcaccatctccagagacaattccaagaacacgctgtatctgcaaatgaacagcctgagatctgaggacacggccgtgtattactgtgcgaggatgcgatgggccgtggctgggatgggggcttttgaaatctggggccaagggaccacggtcaccgtctcctcaggcctcgggggcctcggaggaggaggtagtggcggaggaggctccggtggatccagcggtgtgggttccgacatccagatgacccagtctccaggcaccctgtctttgtctccaggggaaagcgccaccctctcctgcagggccagtcagagtgttaccagtagttacttagcctggtatcagcagaaacctggccaggctcccaaagtcctcatctatggtgcatccggcagggccactggcaccccagccaggttcagtggcggtgggtctgggacagacttcactctcaccatcagcagcctagagcctgaagattttgcagtttattactgtcagcagcgtagcagctggcctccgctcactttcggccctgggtccaaagtggagatcaaa

SEQ ID NO: 654 - protein, 122 aa, Artificial Sequence
  VH2 of A56-18G02
QMQLVQSGGGVVQPGRSLRLSCAASGFTFSSYGMHWVRQAPGKGLEWVAVISYDGSNKYYADSVKGRFTISRDNSKNTLYLQMNSLRSEDTAVYYCARMRWAVAGMGAFEIWGQGTTVTVSS

SEQ ID NO: 655 - protein, 109 aa, Artificial Sequence
  VL2 of A56-18G02
DIQMTQSPGTLSLSPGESATLSCRASQSVTSSYLAWYQQKPGQAPKVLIYGASGRATGTPARFSGGGSGTDFTLTISSLEPEDFAVYYCQQRSSWPPLTFGPGSKVEIK

SEQ ID NO: 656 - protein, 25 aa, Artificial Sequence
  H-FR1 of A56-18G02
QMQLVQSGGGVVQPGRSLRLSCAAS

SEQ ID NO: 657 - protein, 17 aa, Artificial Sequence
  H-FR2 of A56-18G02
MHWVRQAPGKGLEWVAV

SEQ ID NO: 658 - protein, 38 aa, Artificial Sequence; identical to SEQ ID NO: 488
  H-FR3 of A56-18G02

SEQ ID NO: 659 - protein, 11 aa, Artificial Sequence
  H-FR4 of A56-18G02
WGQGTTVTVSS

SEQ ID NO: 660 - protein, 26 aa, Artificial Sequence
  L-FR1 of A56-18G02
DIQMTQSPGTLSLSPGESATLSCRAS

SEQ ID NO: 661 - protein, 17 aa, Artificial Sequence
  L-FR2 of A56-18G02
LAWYQQKPGQAPKVLIY

SEQ ID NO: 662 - protein, 36 aa, Artificial Sequence
  L-FR3 of A56-18G02
IYGASGRATGTPARFSGGGSGTDFTLTISSLEPEDF

SEQ ID NO: 663 - protein, 10 aa, Artificial Sequence
  L-FR4 of A56-18G02
FGPGSKVEIK

SEQ ID NO: 664 - protein, 8 aa, Artificial Sequence
  H-CDR1 of A56-20A05
GGSFRSNA

SEQ ID NO: 665 - protein, 8 aa, Artificial Sequence
  H-CDR2 of A56-20A05
IIPLANRS

SEQ ID NO: 666 - protein, 13 aa, Artificial Sequence
  H-CDR3 of A56-20A05
ARLDDNVSWGLDP

SEQ ID NO: 667 - protein, 6 aa, Artificial Sequence
  L-CDR1 of A56-20A05
QDISRR

SEQ ID NO: 668 - protein, 3 aa, Artificial Sequence
  L-CDR2 of A56-20A05
AAS

SEQ ID NO: 669 - protein, 9 aa, Artificial Sequence
  L-CDR3 of A56-20A05
QQSSNVPLT

SEQ ID NO: 670 - DNA, 750 bp, Artificial Sequence
  SCFV of A56-20A05
caggtgcagctggtgcagtctggggctgaggtggtgaagcccgggtcctcggtgaaggtctcctgtaaggcttctggaggcagcttcagaagcaatgctgtcagctgggtgcgacaggcccctggacaaggtcttgagtggataggaggcatcatccctctggctaataggtcagtctacgcacagaagttccagggcagactcaccattaccgcggacaaatccacgggtacagcctacatggagttgagcagcctgagatctgaggacacggccgtgtattactgtgccagattggatgacaatgtctcttggggactcgacccctggggccagggaaccctggtcaccgtctcctcaggcctcgggggcctcggaggaggaggtagtggcggaggaggctccggtggatccagcggtgtgggttccgacatccagatgacccagtctccatccttcctgtctgcttctgtgggagacagagtcaacatcacttgccgggccagtcaggacattagcagacgtttagcctggtatcagcagaaaccagggaaagcccctaagctcctgatctctgctgcatccagtttgcaaagtggggtcccatcaaggttcagcggcagtggatctgggacagatttcaccctcaccatcagcagtctgcaacctgaagattttgcaacttactactgtcaacagagttccaatgtccccctcactttcggcggagggaccaaggtggaaatcaaa

SEQ ID NO: 671 - protein, 120 aa, Artificial Sequence
  VH2 of A56-20A05
QVQLVQSGAEVVKPGSSVKVSCKASGGSFRSNAVSWVRQAPGQGLEWIGGIIPLANRSVYAQKFQGRLTITADKSTGTAYMELSSLRSEDTAVYYCARLDDNVSWGLDPWGQGTLVTVSS

SEQ ID NO: 672 - protein, 107 aa, Artificial Sequence
  VL2 of A56-20A05
DIQMTQSPSFLSASVGDRVNITCRASQDISRRLAWYQQKPGKAPKLLISAASSLQSGVPSRFSGSGSGTDFTLTISSLQPEDFATYYCQQSSNVPLTFGGGTKVEIK

SEQ ID NO: 673 - protein, 25 aa, Artificial Sequence
  H-FR1 of A56-20A05
QVQLVQSGAEVVKPGSSVKVSCKAS

SEQ ID NO: 674 - protein, 17 aa, Artificial Sequence
  H-FR2 of A56-20A05
VSWVRQAPGQGLEWIGG

SEQ ID NO: 675 - protein, 38 aa, Artificial Sequence
  H-FR3 of A56-20A05
VYAQKFQGRLTITADKSTGTAYMELSSLRSEDTAVYYC

SEQ ID NO: 676 - protein, 11 aa, Artificial Sequence
  H-FR4 of A56-20A05
WGQGTLVTVSS

SEQ ID NO: 677 - protein, 26 aa, Artificial Sequence
  L-FR1 of A56-20A05
DIQMTQSPSFLSASVGDRVNITCRAS

SEQ ID NO: 678 - protein, 17 aa, Artificial Sequence
  L-FR2 of A56-20A05
LAWYQQKPGKAPKLLIS

SEQ ID NO: 679 - protein, 36 aa, Artificial Sequence
  L-FR3 of A56-20A05
ISAASSLQSGVPSRFSGSGSGTDFTLTISSLQPEDF

SEQ ID NO: 680 - protein, 10 aa, Artificial Sequence
  L-FR4 of A56-20A05
FGGGTKVEIK

SEQ ID NO: 681 - protein, 8 aa, Artificial Sequence
  H-CDR1 of A56-20G03
GGTFSSYA

SEQ ID NO: 682 - protein, 8 aa, Artificial Sequence
  H-CDR2 of A56-20G03
IIPIFGTA

SEQ ID NO: 683 - protein, 20 aa, Artificial Sequence
  H-CDR3 of A56-20G03
ATKGGGNSRSFLRYFYGLDV

SEQ ID NO: 684 - protein, 11 aa, Artificial Sequence
  L-CDR1 of A56-20G03
QSLVHSDGNTY

SEQ ID NO: 685 - protein, 3 aa, Artificial Sequence
  L-CDR2 of A56-20G03
KVS

SEQ ID NO: 686 - protein, 9 aa, Artificial Sequence
  L-CDR3 of A56-20G03
MQGTHWPWT

SEQ ID NO: 687 - DNA, 786 bp, Artificial Sequence
  SCFV of A56-20G03
caggtgcagctggtgcagtctggggctgaggtgaagaagcctgggtcctcggtgaaggtctcctgcaaggcttctggaggcaccttcagcagctatgctatcagctgggtgcgacaggcccctggacaagggcttgagtggatgggagggatcatccctatctttggtacagcaaactacgcacagaagttccagggcagagtcacgattaccgcggacgaatccacgaacacagcctacatggagctgagcagcctgagatctgaggacacggccgtgtattactgtgcaacaaaagggggcggcaacagccggagttttcttcggtacttttacggtttggacgtctggggccaagggaccacggtcaccgtctcctcaggcctcgggggcctcggaggaggaggtagtggcggaggaggctccggtggatccagcggtgtgggttccgatattgtgatgacccagactccactctccctgcccgtcgcccttggacagccggcctccatctcctgcaggtctagtcaaagcctcgtacacagtgatggaaacacctacttgaattggtttcagcagaggccaggccaatctccaaggcgcctgatttataaggtttctaaccgggactctggggtcccagacagattcagcggcagtgggtcaggcactgatttcacactgaaaatcagcagggtggaggctgaggatgttggggtttattactgcatgcaaggtacacactggccgtggacgttcggccaagggaccaaggtagaaatcaaa

SEQ ID NO: 688 - protein, 127 aa, Artificial Sequence
  VH2 of A56-20G03
QVQLVQSGAEVKKPGSSVKVSCKASGGTFSSYAISWVRQAPGQGLEWMGGIIPIFGTANYAQKFQGRVTITADESTNTAYMELSSLRSEDTAVYYCATKGGGNSRSFLRYFYGLDVWGQGTTVTVSS

SEQ ID NO: 689 - protein, 112 aa, Artificial Sequence
  VL2 of A56-20G03
DIVMTQTPLSLPVALGQPASISCRSSQSLVHSDGNTYLNWFQQRPGQSPRRLIYKVSNRDSGVPDRFSGSGSGTDFTLKISRVEAEDVGVYYCMQGTHWPWTFGQGTKVEIK

SEQ ID NO: 690 - protein, 25 aa, Artificial Sequence [sequence omitted]

SEQ ID NO: 691 - protein, 17 aa, Artificial Sequence
  H-FR2 of A56-20G03
ISWVRQAPGQGLEWMGG

SEQ ID NO: 692 - protein, 38 aa, Artificial Sequence
  H-FR3 of A56-20G03
NYAQKFQGRVTITADESTNTAYMELSSLRSEDTAVYYC

SEQ ID NO: 693 - protein, 11 aa, Artificial Sequence
  H-FR4 of A56-20G03
WGQGTTVTVSS

SEQ ID NO: 694 - protein, 26 aa, Artificial Sequence
  L-FR1 of A56-20G03
DIVMTQTPLSLPVALGQPASISCRSS

SEQ ID NO: 695 - protein, 17 aa, Artificial Sequence
  L-FR2 of A56-20G03
LNWFQQRPGQSPRRLIY

SEQ ID NO: 696 - protein, 36 aa, Artificial Sequence
  L-FR3 of A56-20G03
IYKVSNRDSGVPDRFSGSGSGTDFTLKISRVEAEDV

SEQ ID NO: 697 - protein, 10 aa, Artificial Sequence
  L-FR4 of A56-20G03
FGQGTKVEIK

SEQ ID NO: 698 - protein, 8 aa, Artificial Sequence
  H-CDR1 of A56-20G12
GFNFNTYA

SEQ ID NO: 699 - protein, 8 aa, Artificial Sequence
  H-CDR2 of A56-20G12
IGGGGGNT

SEQ ID NO: 700 - protein, 10 aa, Artificial Sequence
  H-CDR3 of A56-20G12
ATRGGWYVND

SEQ ID NO: 701 - protein, 9 aa, Artificial Sequence
  L-CDR1 of A56-20G12
SSNIGAGYA

SEQ ID NO: 702 - protein, 3 aa, Artificial Sequence
  L-CDR2 of A56-20G12
SNT

SEQ ID NO: 703 - protein, 12 aa, Artificial Sequence
  L-CDR3 of A56-20G12
QSYDNSLSDSVV

SEQ ID NO: 704 - DNA, 756 bp, Artificial Sequence
  SCFV of A56-20G12
caggtgcagctggtggagtctgggggagggttggtacagccgggggggtccctgagactctcctgtacagcctctggattcaactttaatacctatgccatgagctgggtccgccagcctccagggaaggggctggagtgggtctcaactattgggggtggtggtgggaacacattttacgcagattccgtgaggggccggttcaccatctccagagacaattccgagaacacgctgtatctgcaaatgaacagtctgagagccgaggacacggccgtgtattactgtgcgactcgaggtggctggtacgtcaatgactggggccgcggaaccctggtcaccgtctcctcaggcctcgggggcctcggaggaggaggtagtggcggaggaggctccggtggatccagcggtgtgggttcccagctcgtgctgactcagccgccctcagtgtctggggccccaggacagagggtcaccatctcctgcactgggagtagctccaacatcggggcaggttatgctgtacactggtaccagcagattccaggaacagcccccaaactcctcatctatagtaacaccaataggccctcaggggtccctgaccgattctctggctccaagtctggcacctcagcctccctggccatcactgggctccaggctgaggatgaggctgattattactgccagtcctatgacaacagcctgagtgattctgtggtattcggcggagggaccaagctgaccgtccta

SEQ ID NO: 705 - protein, 117 aa, Artificial Sequence
  VH2 of A56-20G12
QVQLVESGGGLVQPGGSLRLSCTASGFNFNTYAMSWVRQPPGKGLEWVSTIGGGGGNTFYADSVRGRFTISRDNSENTLYLQMNSLRAEDTAVYYCATRGGWYVNDWGRGTLVTVSS

SEQ ID NO: 706 - protein, 112 aa, Artificial Sequence
  VL2 of A56-20G12
QLVLTQPPSVSGAPGQRVTISCTGSSSNIGAGYAVHWYQQIPGTAPKLLIYSNTNRPSGVPDRFSGSKSGTSASLAITGLQAEDEADYYCQSYDNSLSDSVVFGGGTKLTVL

SEQ ID NO: 707 - protein, 25 aa, Artificial Sequence
  H-FR1 of A56-20G12
QVQLVESGGGLVQPGGSLRLSCTAS

SEQ ID NO: 708 - protein, 17 aa, Artificial Sequence
  H-FR2 of A56-20G12
MSWVRQPPGKGLEWVST

SEQ ID NO: 709 - protein, 38 aa, Artificial Sequence
  H-FR3 of A56-20G12
FYADSVRGRFTISRDNSENTLYLQMNSLRAEDTAVYYC

SEQ ID NO: 710 - protein, 11 aa, Artificial Sequence
  H-FR4 of A56-20G12
WGRGTLVTVSS

SEQ ID NO: 711 - protein, 25 aa, Artificial Sequence
  L-FR1 of A56-20G12
QLVLTQPPSVSGAPGQRVTISCTGS

SEQ ID NO: 712 - protein, 17 aa, Artificial Sequence
  L-FR2 of A56-20G12
VHWYQQIPGTAPKLLIY

SEQ ID NO: 713 - protein, 36 aa, Artificial Sequence
  L-FR3 of A56-20G12
IYSNTNRPSGVPDRFSGSKSGTSASLAITGLQAEDE

SEQ ID NO: 714 - protein, 10 aa, Artificial Sequence
  L-FR4 of A56-20G12
FGGGTKLTVL

SEQ ID NO: 715 - protein, 8 aa, Artificial Sequence
  H-CDR1 of A56-21B10
GDTFSTYA

SEQ ID NO: 716 - protein, 8 aa, Artificial Sequence
  H-CDR2 of A56-21B10
IIPRLGIA

SEQ ID NO: 717 - protein, 19 aa, Artificial Sequence
  H-CDR3 of A56-21B10
AADPLWFGDFIRGGRAFNI

SEQ ID NO: 718 - protein, 6 aa, Artificial Sequence
  L-CDR1 of A56-21B10
QSISTW

SEQ ID NO: 719 - protein, 3 aa, Artificial Sequence
  L-CDR2 of A56-21B10
KAS

SEQ ID NO: 720 - protein, 9 aa, Artificial Sequence
  L-CDR3 of A56-21B10
QQYYNYPYT

SEQ ID NO: 721 - DNA, 768 bp, Artificial Sequence
  SCFV of A56-21B10
cagatgcagctggtgcagtctggggctgaggtgagaaagcctgggtcttcggtgacggtctcctgcaaggctcctggagacaccttcagtacttatgctatcagttgggtgcgacaggcccctggacaagggcttgactggatggggaggatcatccctcgccttggtattgcaaaaaatgcaccggagttccaggacagagtctcgatcaccgcggacaaatccacgaatacagtgcatatggagttgagaaacctcagatctgaggacacggccgtgtattactgtgcagcagaccccctatggttcggggactttattcgagggggacgtgctttcaatatctggggccaagggacaatgatcaccgtctcctcaggcctcgggggcctcggaggaggaggtagtggcggaggaggctccggtggatccagcggtgtgggttccgacatccagatgacccagtctccttccaccctgtctgcatctataggagacagagtcaccatcacttgccgggccagtcagagtattagtacctggttggcctggtatcagcagaaaccagggaaagccccaaagctcctgatctataaggcgtctactatagaaagtggggtcccatcaaggttcagcggcagcggatctgacacagaattcactctcaccatcaccaacctgcagcctgatgactctgcaacttattactgccaacaatattataattatccgtacacttttggccaggggaccaagctggagatcaaa

SEQ ID NO: 722 - protein, 126 aa, Artificial Sequence
  VH2 of A56-21B10
QMQLVQSGAEVRKPGSSVTVSCKAPGDTFSTYAISWVRQAPGQGLDWMGRIIPRLGIAKNAPEFQDRVSITADKSTNTVHMELRNLRSEDTAVYYCAADPLWFGDFIRGGRAFNIWGQGTMITVSS

SEQ ID NO: 723 - protein, 107 aa, Artificial Sequence
  VL2 of A56-21B10
DIQMTQSPSTLSASIGDRVTITCRASQSISTWLAWYQQKPGKAPKLLIYKASTIESGVPSRFSGSGSDTEFTLTITNLQPDDSATYYCQQYYNYPYTFGQGTKLEIK

SEQ ID NO: 724 - protein, 25 aa, Artificial Sequence
  H-FR1 of A56-21B10
QMQLVQSGAEVRKPGSSVTVSCKAP

SEQ ID NO: 725 - protein, 17 aa, Artificial Sequence
  H-FR2 of A56-21B10
ISWVRQAPGQGLDWMGR

SEQ ID NO: 726 - protein, 38 aa, Artificial Sequence
  H-FR3 of A56-21B10
KNAPEFQDRVSITADKSTNTVHMELRNLRSEDTAVYYC

SEQ ID NO: 727 - protein, 11 aa, Artificial Sequence
  H-FR4 of A56-21B10
WGQGTMITVSS

SEQ ID NO: 728 - protein, 26 aa, Artificial Sequence
  L-FR1 of A56-21B10
DIQMTQSPSTLSASIGDRVTITCRAS

SEQ ID NO: 729 - protein, 17 aa, Artificial Sequence
  L-FR2 of A56-21B10
LAWYQQKPGKAPKLLIY

SEQ ID NO: 730 - protein, 36 aa, Artificial Sequence
  L-FR3 of A56-21B10
IYKASTIESGVPSRFSGSGSDTEFTLTITNLQPDDS

SEQ ID NO: 731 - protein, 10 aa, Artificial Sequence
  L-FR4 of A56-21B10
FGQGTKLEIK

SEQ ID NO: 732 - protein, 8 aa, Artificial Sequence
  H-CDR1 of A56-21F02
GFTFDYSA

SEQ ID NO: 733 - protein, 8 aa, Artificial Sequence
  H-CDR2 of A56-21F02
ISGDGGTA

SEQ ID NO: 734 - protein, 16 aa, Artificial Sequence
  H-CDR3 of A56-21F02
ARDRWRWMDDYYGMDV

SEQ ID NO: 735 - protein, 6 aa, Artificial Sequence
  L-CDR1 of A56-21F02
QGITGY

SEQ ID NO: 736 - protein, 3 aa, Artificial Sequence
  L-CDR2 of A56-21F02
KSS

SEQ ID NO: 737 - protein, 9 aa, Artificial Sequence
  L-CDR3 of A56-21F02
QQYDSYPWT

SEQ ID NO: 738 - DNA, 759 bp, Artificial Sequence
  SCFV of A56-21F02
cagatgcagctggtgcagtcggggggaaccgtggtacagcctggggagtccctgagactctcctgtgcaacctctggattcacctttgattattctgccatgcactgggtccgtcaagctccagggaagggtctggagtgggtctctctcatcagtggggatggtggtaccgcatattatgcagactctgtgaagggccgattcaccgtctccagagacaacagcaaaaactccctgtatctgcaaatgaacagtctgagagccgaggacacggccgtgtattactgtgcgagagacaggtggcgctggatggacgactactacggtatggacgtctggggccaagggaccacggtcaccgtctcctcaggcctcgggggcctcggaggaggaggtagtggcggaggaggctccggtggatccagcggtgtgggttccgacatccagatgacccagtctccatcctccctgtctacttctgtaggagacagagtcaccatcacttgccgggccagtcagggcattaccggttattttgcctggtatcagcagaaaccagggaaagcccctaacctcctcctctataagtcatctatcttacaaagtggagtcccatctagattcagcggcagtggatctgggacagaattcactctcaccatcaacagcctgcaggctgatgattttgcaacttattactgccaacagtatgatagttatccgtggacgttcggccaagggaccaaggtggatatcaaa

SEQ ID NO: 739 - protein, 123 aa, Artificial Sequence
  VH2 of A56-21F02
QMQLVQSGGTVVQPGESLRLSCATSGFTFDYSAMHWVRQAPGKGLEWVSLISGDGGTAYYADSVKGRFTVSRDNSKNSLYLQMNSLRAEDTAVYYCARDRWRWMDDYYGMDVWGQGTTVTVSS

SEQ ID NO: 740 - protein, 107 aa, Artificial Sequence
  VL2 of A56-21F02
DIQMTQSPSSLSTSVGDRVTITCRASQGITGYFAWYQQKPGKAPNLLLYKSSILQSGVPSRFSGSGSGTEFTLTINSLQADDFATYYCQQYDSYPWTFGQGTKVDIK

SEQ ID NO: 741 - protein, 25 aa, Artificial Sequence
  H-FR1 of A56-21F02
QMQLVQSGGTVVQPGESLRLSCATS

SEQ ID NO: 742 - protein, 17 aa, Artificial Sequence
  H-FR2 of A56-21F02
MHWVRQAPGKGLEWVSL

SEQ ID NO: 743 - protein, 38 aa, Artificial Sequence
  H-FR3 of A56-21F02
YYADSVKGRFTVSRDNSKNSLYLQMNSLRAEDTAVYYC

SEQ ID NO: 744 - protein, 11 aa, Artificial Sequence
  H-FR4 of A56-21F02
WGQGTTVTVSS

SEQ ID NO: 745 - protein, 26 aa, Artificial Sequence
  L-FR1 of A56-21F02
DIQMTQSPSSLSTSVGDRVTITCRAS

SEQ ID NO: 746 - protein, 17 aa, Artificial Sequence
  L-FR2 of A56-21F02
FAWYQQKPGKAPNLLLY

SEQ ID NO: 747 - protein, 36 aa, Artificial Sequence
  L-FR3 of A56-21F02
LYKSSILQSGVPSRFSGSGSGTEFTLTINSLQADDF

SEQ ID NO: 748 - protein, 10 aa, Artificial Sequence
  L-FR4 of A56-21F02
FGQGTKVDIK

SEQ ID NO: 749 - protein, 8 aa, Artificial Sequence
  H-CDR1 of A56-21H04
GFTFNFYG

SEQ ID NO: 750 - protein, 8 aa, Artificial Sequence
  H-CDR2 of A56-21H04
ISYEGSKK

SEQ ID NO: 751 - protein, 20 aa, Artificial Sequence
  H-CDR3 of A56-21H04
ARGFDPDYLRGNNRYFGLDV

SEQ ID NO: 752 - protein, 6 aa, Artificial Sequence
  L-CDR1 of A56-21H04
EDISRQ

SEQ ID NO: 753 - protein, 3 aa, Artificial Sequence
  L-CDR2 of A56-21H04
GAS

SEQ ID NO: 754 - protein, 9 aa, Artificial Sequence
  L-CDR3 of A56-21H04
QKANNFPYT

SEQ ID NO: 755 - DNA, 771 bp, Artificial Sequence
  SCFV of A56-21H04
caggtgcagctggtggagtctgggggaggtgtggtccagcctgggaggtccctgagactctcctgtgcagcctctggattcaccttcaatttctatggtatgcactgggtccgccaggctccaggtaaggggctagagtggctggcagctatatcatatgaaggaagtaagaagtactacgcagactccgtgaagggccgattcaccatctccagagacaattccaagaacacgccggatctgcaaatgaacagtctgagagccgaggacacggccgtgtattactgtgcgagaggcttcgatcccgattaccttcggggtaataatcgttacttcggtctggacgtctggggccaagggaccacggtcaccgtctcctcaggcctcgggggcctcggaggaggaggtagtggcggaggaggctccggtggatccagcggtgtgggttccgacatccagatgacccagtctccatcttccgtgtctgcatctgtaggagacagagtcaccatcacttgtcgggcgagtgaggacattagtaggcagttagcctggtatcagcagaaaccagggaaagcccctaaactcctgatctatggtgcttctagtttgcaaagtggagtcccatcaaggttcagcggcagtggatttgggacagaattcactcttaccatcaacagcctgcagcctgaagattttgcaacttactattgtcaaaaggctaataatttcccgtacacttttggccaagggaccaaggtggatatcaaa

SEQ ID NO: 756 - protein, 127 aa, Artificial Sequence
  VH2 of A56-21H04
QVQLVESGGGVVQPGRSLRLSCAASGFTFNFYGMHWVRQAPGKGLEWLAAISYEGSKKYYADSVKGRFTISRDNSKNTPDLQMNSLRAEDTAVYYCARGFDPDYLRGNNRYFGLDVWGQGTTVTVSS

SEQ ID NO: 757 - protein, 107 aa, Artificial Sequence
  VL2 of A56-21H04
DIQMTQSPSSVSASVGDRVTITCRASEDISRQLAWYQQKPGKAPKLLIYGASSLQSGVPSRFSGSGFGTEFTLTINSLQPEDFATYYCQKANNFPYTFGQGTKVDIK

SEQ ID NO: 758 - protein, 25 aa, Artificial Sequence
  H-FR1 of A56-21H04
QVQLVESGGGVVQPGRSLRLSCAAS

SEQ ID NO: 759 - protein, 17 aa, Artificial Sequence
  H-FR2 of A56-21H04
MHWVRQAPGKGLEWLAA

SEQ ID NO: 760 - protein, 38 aa, Artificial Sequence
  H-FR3 of A56-21H04
YYADSVKGRFTISRDNSKNTPDLQMNSLRAEDTAVYYC

SEQ ID NO: 761 - protein, 11 aa, Artificial Sequence
  H-FR4 of A56-21H04
WGQGTTVTVSS

SEQ ID NO: 762 - protein, 26 aa, Artificial Sequence [sequence omitted]

SEQ ID NO: 763 - protein, 17 aa, Artificial Sequence
  L-FR2 of A56-21H04
LAWYQQKPGKAPKLLIY

SEQ ID NO: 764 - protein, 36 aa, Artificial Sequence
  L-FR3 of A56-21H04
IYGASSLQSGVPSRFSGSGFGTEFTLTINSLQPEDF

SEQ ID NO: 765 - protein, 10 aa, Artificial Sequence
  L-FR4 of A56-21H04
FGQGTKVDIK

SEQ ID NO: 766 - protein, 8 aa, Artificial Sequence
  H-CDR1 of A56-22G10
GFMFKNYA

SEQ ID NO: 767 - protein, 8 aa, Artificial Sequence
  H-CDR2 of A56-22G10
VSGSGDTT

SEQ ID NO: 768 - protein, 12 aa, Artificial Sequence
  H-CDR3 of A56-22G10
AKVGVAVAQGDY

SEQ ID NO: 769 - protein, 12 aa, Artificial Sequence
  L-CDR1 of A56-22G10
QSVLSSSNNKNY

SEQ ID NO: 770 - protein, 3 aa, Artificial Sequence
  L-CDR2 of A56-22G10
WAS

SEQ ID NO: 771 - protein, 9 aa, Artificial Sequence
  L-CDR3 of A56-22G10
QQYYGTPLT

SEQ ID NO: 772 - DNA, 765 bp, Artificial Sequence
  SCFV of A56-22G10
cagatgcagctggtggagtcggggggaggcttcgtacagcctggggggtcccggagactctcctgtgcaggctctggattcatgtttaagaattatgccatgacttggtttcgccaggctccagggaaggggctggagtgggtctcagctgtcagtggttctggtgacaccacatactacacagactccgtgaagggccggttcatcatctccagagacaattccaacaacaccgtctatctgcaaatgaacagtctgagagccgaggacacggccgtgtattactgtgcgaaagtgggtgtagcagtggcccaaggggactactggggccagggaaccctggtcaccgtctcctcaggcctcgggggcctcggaggaggaggtagtggcggaggaggctccggtggatccagcggtgtgggttccgacatccagatgacccagtctccagactccctggctgtgtctctgggcgagagggccaccatcaactgcaagtccagccagagtgttttatccagctccaacaataagaactacttagcttggtaccagcagaaaccgggacagcctcctaaactgctcatttactgggcatctacccgggaatccggggtccctgaccgattcagtggcagcgggtctgggacagatttcactctcaccatcagcagcctgcaggctgaagatgtggcagtttattactgtcagcaatattatggtactcccctcactttcggcggagggaccaaggtggaaatcaaa

SEQ ID NO: 773 - protein, 119 aa, Artificial Sequence
  VH2 of A56-22G10
QMQLVESGGGFVQPGGSRRLSCAGSGFMFKNYAMTWFRQAPGKGLEWVSAVSGSGDTTYYTDSVKGRFIISRDNSNNTVYLQMNSLRAEDTAVYYCAKVGVAVAQGDYWGQGTLVTVSS

SEQ ID NO: 774 - protein, 113 aa, Artificial Sequence
  VL2 of A56-22G10
DIQMTQSPDSLAVSLGERATINCKSSQSVLSSSNNKNYLAWYQQKPGQPPKLLIYWASTRESGVPDRFSGSGSGTDFTLTISSLQAEDVAVYYCQQYYGTPLTFGGGTKVEIK

SEQ ID NO: 775 - protein, 25 aa, Artificial Sequence
  H-FR1 of A56-22G10
QMQLVESGGGFVQPGGSRRLSCAGS

SEQ ID NO: 776 - protein, 17 aa, Artificial Sequence
  H-FR2 of A56-22G10
MTWFRQAPGKGLEWVSA

SEQ ID NO: 777 - protein, 38 aa, Artificial Sequence
  H-FR3 of A56-22G10
YYTDSVKGRFIISRDNSNNTVYLQMNSLRAEDTAVYYC

SEQ ID NO: 778 - protein, 11 aa, Artificial Sequence
  H-FR4 of A56-22G10
WGQGTLVTVSS

SEQ ID NO: 779 - protein, 26 aa, Artificial Sequence
  L-FR1 of A56-22G10
DIQMTQSPDSLAVSLGERATINCKSS

SEQ ID NO: 780 - protein, 17 aa, Artificial Sequence
  L-FR2 of A56-22G10
LAWYQQKPGQPPKLLIY

SEQ ID NO: 781 - protein, 36 aa, Artificial Sequence; identical to SEQ ID NO: 288
  L-FR3 of A56-22G10

SEQ ID NO: 782 - protein, 10 aa, Artificial Sequence
  L-FR4 of A56-22G10
FGGGTKVEIK

SEQ ID NO: 783 - protein, 8 aa, Artificial Sequence
  H-CDR1 of A56-24A05
RYTFTYRY

SEQ ID NO: 784 - protein, 8 aa, Artificial Sequence
  H-CDR2 of A56-24A05
IQPFNGNT

SEQ ID NO: 785 - protein, 16 aa, Artificial Sequence
  H-CDR3 of A56-24A05
AKDIRIEDIVVVPAAI

SEQ ID NO: 786 - protein, 9 aa, Artificial Sequence
  L-CDR1 of A56-24A05
SSDVGGYNY

SEQ ID NO: 787 - protein, 3 aa, Artificial Sequence
  L-CDR2 of A56-24A05
EVN

SEQ ID NO: 788 - protein, 10 aa, Artificial Sequence
  L-CDR3 of A56-24A05
SSYTSSSTFD

SEQ ID NO: 789 - DNA, 768 bp, Artificial Sequence
  SCFV of A56-24A05
caggtgcagctggtgcagtctggggctgaggtgaagaagactgggtcctcagtgaaagtttcctgcaagacttccagatacaccttcacctaccgttatctgcactgggtgcgacaggcccccggacaagcgcttgagtggttggggtggatccaacctttcaatggtaataccaactacgcacagaaattccaagacagagtcaccattacccgggacaggtctatgagcacagcctacatggagctgagcagcctgagatctgaggacacggccgtgtattactgtgcaaaagatatccgaatcgaggatattgtagtagtaccagctgctatttggggccagggaaccctggtcaccgtctcctcaggcctcgggggcctcggaggaggaggtagtggcggaggaggctccggtggatccagcggtgtgggttcccagtctgccctgactcagcctgcctccgtgtctgggtctcctggacagtcgatcaccatctcctgcactggaaccagcagtgacgttggtggttataactatgtctcctggtaccaacagcacccaggcaaagcccccaaactcatgatttatgaggtcaataagcggccctcaggggtttctaatcgcttctctggctccaagtctggcaacacggccttcctgaccatctctgggctccagtctgaggacgaggctgattattactgcagctcatatacaagcagcagtactttcgacttcggaactgggaccaaggtcaccgtccta

SEQ ID NO: 790 - protein, 123 aa, Artificial Sequence
  VH2 of A56-24A05
QVQLVQSGAEVKKTGSSVKVSCKTSRYTFTYRYLHWVRQAPGQALEWLGWIQPFNGNTNYAQKFQDRVTITRDRSMSTAYMELSSLRSEDTAVYYCAKDIRIEDIVVVPAAIWGQGTLVTVSS

SEQ ID NO: 791 - protein, 110 aa, Artificial Sequence
  VL2 of A56-24A05
QSALTQPASVSGSPGQSITISCTGTSSDVGGYNYVSWYQQHPGKAPKLMIYEVNKRPSGVSNRFSGSKSGNTAFLTISGLQSEDEADYYCSSYTSSSTFDFGTGTKVTVL

SEQ ID NO: 792 - protein, 25 aa, Artificial Sequence
  H-FR1 of A56-24A05
QVQLVQSGAEVKKTGSSVKVSCKTS

SEQ ID NO: 793 - protein, 17 aa, Artificial Sequence
  H-FR2 of A56-24A05
LHWVRQAPGQALEWLGW

SEQ ID NO: 794 - protein, 38 aa, Artificial Sequence; identical to SEQ ID NO: 46
  H-FR3 of A56-24A05

SEQ ID NO: 795 - protein, 11 aa, Artificial Sequence
  H-FR4 of A56-24A05
WGQGTLVTVSS

SEQ ID NO: 796 - protein, 25 aa, Artificial Sequence
  L-FR1 of A56-24A05
QSALTQPASVSGSPGQSITISCTGT

SEQ ID NO: 797 - protein, 17 aa, Artificial Sequence
  L-FR2 of A56-24A05
VSWYQQHPGKAPKLMIY

SEQ ID NO: 798 - protein, 36 aa, Artificial Sequence
  L-FR3 of A56-24A05
IYEVNKRPSGVSNRFSGSKSGNTAFLTISGLQSEDE

SEQ ID NO: 799 - protein, 10 aa, Artificial Sequence
  L-FR4 of A56-24A05
FGTGTKVTVL

SEQ ID NO: 800 - protein, 8 aa, Artificial Sequence
  H-CDR1 of A56-30H01
GFTFKTYS

SEQ ID NO: 801 - protein, 8 aa, Artificial Sequence
  H-CDR2 of A56-30H01
INNNGDAT

SEQ ID NO: 802 - protein, 28 aa, Artificial Sequence
  H-CDR3 of A56-30H01
ARDLIAHEQPKFSLRYFDWLSSRKGMDV

SEQ ID NO: 803 - protein, 9 aa, Artificial Sequence
  L-CDR1 of A56-30H01
SSDVGGYNY

SEQ ID NO: 804 - protein, 3 aa, Artificial Sequence
  L-CDR2 of A56-30H01
DVT

SEQ ID NO: 805 - protein, 10 aa, Artificial Sequence
  L-CDR3 of A56-30H01
SSYSSSTFYV

SEQ ID NO: 806 - DNA, 804 bp, Artificial Sequence
  SCFV of A56-30H01
caggtgcagctggtgcagtctgggggaggcttggtccagcctggggggtccctgaaactctcctgttcagcctctggattcaccttcaaaacctattctatgcactgggtccgccaggctccggggaagggactggaatatgtttcagctattaataataatggggatgccacatactacgcagactccgtgaagggcagattcaccatctccagagacaattccaaggacacgctgtatcttcaaatgaacagtctgagagccgaggacacggccgtgtattactgtgcgagagatcttatagcccatgaacagccgaaattctccttacgatattttgactggttatcaagcaggaagggtatggacgtctggggccaagggaccacgatcaccgtctcctcaggcctcgggggcctcggaggaggaggtagtggcggaggaggctccggtggatccagcggtgtgggttccaattttatgctgactcagcccgcctccgtgtctgggtcccctggacagtcgatcaccatctcctgcactggaagcagcagcgacgttggtggttataactatgtctcctggtaccaacagcacccaggcaaagccccccaactcatcatttatgatgtcactaagcggccctcaggggtttctaatcgcttctccggctccaagtctggcaactcggcctccctgaccatctctggactccaggctgaggacgaggctgattattactgcagctcatacagcagcagcactttttacgtcttcggaactgggaccaaggtcaccgtccta

SEQ ID NO: 807 - protein, 135 aa, Artificial Sequence
  VH2 of A56-30H01
QVQLVQSGGGLVQPGGSLKLSCSASGFTFKTYSMHWVRQAPGKGLEYVSAINNNGDATYYADSVKGRFTISRDNSKDTLYLQMNSLRAEDTAVYYCARDLIAHEQPKFSLRYFDWLSSRKGMDVWGQGTTITVSS

SEQ ID NO: 808 - protein, 110 aa, Artificial Sequence; identical to SEQ ID NO: 519
  VL2 of A56-30H01

SEQ ID NO: 809 - protein, 25 aa, Artificial Sequence
  H-FR1 of A56-30H01
QVQLVQSGGGLVQPGGSLKLSCSAS

SEQ ID NO: 810 - protein, 17 aa, Artificial Sequence
  H-FR2 of A56-30H01
MHWVRQAPGKGLEYVSA

SEQ ID NO: 811 - protein, 38 aa, Artificial Sequence
  H-FR3 of A56-30H01
YYADSVKGRFTISRDNSKDTLYLQMNSLRAEDTAVYYC

SEQ ID NO: 812 - protein, 11 aa, Artificial Sequence
  H-FR4 of A56-30H01
WGQGTTITVSS

SEQ ID NO: 813 - protein, 25 aa, Artificial Sequence
  L-FR1 of A56-30H01
NFMLTQPASVSGSPGQSITISCTGS

SEQ ID NO: 814 - protein, 17 aa, Artificial Sequence
  L-FR2 of A56-30H01
VSWYQQHPGKAPQLIIY

SEQ ID NO: 815 - protein, 36 aa, Artificial Sequence; identical to SEQ ID NO: 152
  L-FR3 of A56-30H01

SEQ ID NO: 816 - protein, 10 aa, Artificial Sequence
  L-FR4 of A56-30H01
FGTGTKVTVL

SEQ ID NO: 817 - protein, 9 aa, Artificial Sequence
  H-CDR1 of A56-32H08
SGFKFEDHA

SEQ ID NO: 818 - protein, 8 aa, Artificial Sequence
  H-CDR2 of A56-32H08
ISGNGDDT

SEQ ID NO: 819 - protein, 5 aa, Artificial Sequence
  H-CDR3 of A56-32H08
VTRGA

SEQ ID NO: 820 - protein, 6 aa, Artificial Sequence
  L-CDR1 of A56-32H08
QSVGTW

SEQ ID NO: 821 - protein, 3 aa, Artificial Sequence
  L-CDR2 of A56-32H08
AAS

SEQ ID NO: 822 - protein, 8 aa, Artificial Sequence
  L-CDR3 of A56-32H08
QQADSFHS

SEQ ID NO: 823 - DNA, 723 bp, Artificial Sequence
  SCFV of A56-32H08
cagatgcagctggtggagtcagggggaggcgtggtacagcctggggggtccctaagactcgcctgtgtaggctctggattcaagtttgaagatcatgccatacactgggtccgtcaacgtccagggaagggtctggagtgggtcgccgttataagtggcaatggcgatgacacatactatgcagactctgcgaagggccgattcaccatttccagagacaacagcaaaaactccctgtatctgcaaatgaacagtctgagagccgaggacacggccgtgtattactgtgtgactagaggcgctcagggccggggaaccctggtcaccgtctcctcaggcctcgggggcctcggaggaggaggtagtggcggaggaggctccggtggatccagcggtgtgggttccgacatccagatgacccagtctccatcttccgtgtctgcatctgtaggagacagagtcaccatcacttgtcgggcgagtcagagtgttggcacctggttagcctggtatcagcagaaaccagggagggcccctaaactcctgatctctgctgcatccagtttgcaccctggggtcccatcaaggttcagcggcagtggatctgggacagaattcactctcaccatcagcagcctgcagcctgaggatattgcaacttactattgtcaacaggctgacagtttccattctttcggccctgggaccaaagtggatatcaaa

SEQ ID NO: 824 - protein, 112 aa, Artificial Sequence
  VH2 of A56-32H08
QMQLVESGGGVVQPGGSLRLACVGSGFKFEDHAIHWVRQRPGKGLEWVAVISGNGDDTYYADSAKGRFTISRDNSKNSLYLQMNSLRAEDTAVYYCVTRGAQGRGTLVTVSS

SEQ ID NO: 825 - protein, 106 aa, Artificial Sequence
  VL2 of A56-32H08
DIQMTQSPSSVSASVGDRVTITCRASQSVGTWLAWYQQKPGRAPKLLISAASSLHPGVPSRFSGSGSGTEFTLTISSLQPEDIATYYCQQADSFHSFGPGTKVDIK

SEQ ID NO: 826 - protein, 24 aa, Artificial Sequence
  H-FR1 of A56-32H08
QMQLVESGGGVVQPGGSLRLACVG

SEQ ID NO: 827 - protein, 17 aa, Artificial Sequence
  H-FR2 of A56-32H08
IHWVRQRPGKGLEWVAV

SEQ ID NO: 828 - protein, 38 aa, Artificial Sequence; identical to SEQ ID NO: 182
  H-FR3 of A56-32H08

SEQ ID NO: 829 - protein, 11 aa, Artificial Sequence
  H-FR4 of A56-32H08
QGRGTLVTVSS

SEQ ID NO: 830 - protein, 26 aa, Artificial Sequence [sequence omitted]

SEQ ID NO: 831 - protein, 17 aa, Artificial Sequence
  L-FR2 of A56-32H08
LAWYQQKPGRAPKLLIS

SEQ ID NO: 832 - protein, 36 aa, Artificial Sequence
  L-FR3 of A56-32H08
ISAASSLHPGVPSRFSGSGSGTEFTLTISSLQPEDI

SEQ ID NO: 833 - protein, 10 aa, Artificial Sequence
  L-FR4 of A56-32H08
FGPGTKVDIK

SEQ ID NO: 834 - protein, 8 aa, Artificial Sequence
  H-CDR1 of A56-35A06
GDTFRKFT

SEQ ID NO: 835 - protein, 8 aa, Artificial Sequence
  H-CDR2 of A56-35A06
LIPIFGTP

SEQ ID NO: 836 - protein, 17 aa, Artificial Sequence
  H-CDR3 of A56-35A06
VRENYEFLTGATRYFDL

SEQ ID NO: 837 - protein, 9 aa, Artificial Sequence
  L-CDR1 of A56-35A06
SSNLGAPND

SEQ ID NO: 838 - protein, 3 aa, Artificial Sequence
  L-CDR2 of A56-35A06
GST

SEQ ID NO: 839 - protein, 12 aa, Artificial Sequence
  L-CDR3 of A56-35A06
QSYDNRLSGFVV

SEQ ID NO: 840 - DNA, 777 bp, Artificial Sequence
  SCFV of A56-35A06
caggtgcagctggtgcagtctggggctgaggtgaagaagcctgggtcctcggttacggtctcctgcaaggcctctggagacaccttcaggaagtttactttcaactgggtgcgacaggcccctggacaagggcttgagtggatgggagggctcatcccgatctttggtacacctaaatactcacagaagttccaggacagattcacaataaccgcggacgaatcaacgagcacagcctacatggagctacgtcgcctgggatctgaggacacggccgtgtattactgtgtgagagagaattatgagttcttgactggcgccactcgctacttcgatctctggggccgcggcaccctgatcaccgtctcctcaggcctcgggggcctcggaggaggaggtagtggcggaggaggctccggtggatccagcggtgtgggttcccagttcgtgctgactcagccgccctcagtgtctggggccccagggcagggggtcaccatctcatgcactgggagcagttccaatctcggggcacctaatgatgtacactggtaccagcaacgtccaggaacagccccccgactcctcatctatggtagcaccaatcgcccttcaggagtccctgaccgattctctggttccatgtctggcgcctccgcatctctggccatcactgggctcctgcctgaggatgaggctgattattactgccagtcctatgacaacagactgagtggttttgtggttttcggcggagggaccaagctgaccgtccta

SEQ ID NO: 841 - protein, 124 aa, Artificial Sequence
  VH2 of A56-35A06
QVQLVQSGAEVKKPGSSVTVSCKASGDTFRKFTFNWVRQAPGQGLEWMGGLIPIFGTPKYSQKFQDRFTITADESTSTAYMELRRLGSEDTAVYYCVRENYEFLTGATRYFDLWGRGTLITVSS

SEQ ID NO: 842 - protein, 112 aa, Artificial Sequence
  VL2 of A56-35A06
QFVLTQPPSVSGAPGQGVTISCTGSSSNLGAPNDVHWYQQRPGTAPRLLIYGSTNRPSGVPDRFSGSMSGASASLAITGLLPEDEADYYCQSYDNRLSGFVVFGGGTKLTVL

SEQ ID NO: 843 - protein, 25 aa, Artificial Sequence
  H-FR1 of A56-35A06
QVQLVQSGAEVKKPGSSVTVSCKAS

SEQ ID NO: 844 - protein, 17 aa, Artificial Sequence
  H-FR2 of A56-35A06
FNWVRQAPGQGLEWMGG

SEQ ID NO: 845 - protein, 38 aa, Artificial Sequence
  H-FR3 of A56-35A06
KYSQKFQDRFTITADESTSTAYMELRRLGSEDTAVYYC

SEQ ID NO: 846 - protein, 11 aa, Artificial Sequence
  H-FR4 of A56-35A06
WGRGTLITVSS

SEQ ID NO: 847 - protein, 25 aa, Artificial Sequence
  L-FR1 of A56-35A06
QFVLTQPPSVSGAPGQGVTISCTGS

SEQ ID NO: 848 - protein, 17 aa, Artificial Sequence
  L-FR2 of A56-35A06
VHWYQQRPGTAPRLLIY

SEQ ID NO: 849 - protein, 36 aa, Artificial Sequence
  L-FR3 of A56-35A06
IYGSTNRPSGVPDRFSGSMSGASASLAITGLLPEDE

SEQ ID NO: 850 - protein, 10 aa, Artificial Sequence
  L-FR4 of A56-35A06
FGGGTKLTVL

SEQ ID NO: 851 - protein, 8 aa, Artificial Sequence
  H-CDR1 of A56-35G07
GDTFSSYA

SEQ ID NO: 852 - protein, 8 aa, Artificial Sequence
  H-CDR2 of A56-35G07
TIPRLGAT

SEQ ID NO: 853 - protein, 19 aa, Artificial Sequence
  H-CDR3 of A56-35G07
ARYIPLVRGVRQPRDDFEI

SEQ ID NO: 854 - protein, 7 aa, Artificial Sequence
  L-CDR1 of A56-35G07
QSVSSSY

SEQ ID NO: 855 - protein, 3 aa, Artificial Sequence
  L-CDR2 of A56-35G07
GAS

SEQ ID NO: 856 - protein, 11 aa, Artificial Sequence
  L-CDR3 of A56-35G07
QHRKSWPPGAT

SEQ ID NO: 857 - DNA, 777 bp, Artificial Sequence
  SCFV of A56-35G07
cagatgcagctggtgcagtctggggctgaggtgaggaagcctgggtcctcggtgaaggtctcctgcaaggcttctggagacaccttcagcagctatgctgtcagctgggtgcgacaggcccctggactagggcttgaatggatgggaaggaccatccctcgccttggggcaacaagctacgcacagaacttccagggcagagtctcgatcactgcggacaaatccacgaatacagtgtacatggaactgagtgggttgcgatctgaggacacggccgtgtattactgtgcgaggtacattcctctggttcggggagtccgacagccaagagatgattttgaaatttggggcccagggacaatgatcaccgtctcctcaggcctcgggggcctcggaggaggaggtagtggcggaggaggctccggtggatccagcggtgtgggttccgacatccagatgacccagtctccaggcaccctgtctttgtctccaggggaaagagccaccctctcctgcagggccagtcagagtgttagcagcagctacttagcctggtaccagcagaaacctggccaggctcccaggctcctcatctatggtgcatccagcagggccactggcatcccagacaggttcagtggcagtgggtctgggacagacttcactcttaccatcagcagcctcgagcctgaagattttgcagtttattactgtcagcaccgtaagagctggcctccgggggccaccttcggccaagggacacgactagaaatcaaa

SEQ ID NO: 858 - protein, 126 aa, Artificial Sequence
  VH2 of A56-35G07
QMQLVQSGAEVRKPGSSVKVSCKASGDTFSSYAVSWVRQAPGLGLEWMGRTIPRLGATSYAQNFQGRVSITADKSTNTVYMELSGLRSEDTAVYYCARYIPLVRGVRQPRDDFEIWGPGTMITVSS

SEQ ID NO: 859 - protein, 110 aa, Artificial Sequence
  VL2 of A56-35G07
DIQMTQSPGTLSLSPGERATLSCRASQSVSSSYLAWYQQKPGQAPRLLIYGASSRATGIPDRFSGSGSGTDFTLTISSLEPEDFAVYYCQHRKSWPPGATFGQGTRLEIK

SEQ ID NO: 860 - protein, 25 aa, Artificial Sequence
  H-FR1 of A56-35G07
QMQLVQSGAEVRKPGSSVKVSCKAS

SEQ ID NO: 861 - protein, 17 aa, Artificial Sequence
  H-FR2 of A56-35G07
VSWVRQAPGLGLEWMGR

SEQ ID NO: 862 - protein, 38 aa, Artificial Sequence
  H-FR3 of A56-35G07
SYAQNFQGRVSITADKSTNTVYMELSGLRSEDTAVYYC

SEQ ID NO: 863 - protein, 11 aa, Artificial Sequence
  H-FR4 of A56-35G07
WGPGTMITVSS

SEQ ID NO: 864 - protein, 26 aa, Artificial Sequence
  L-FR1 of A56-35G07
DIQMTQSPGTLSLSPGERATLSCRAS

SEQ ID NO: 865 - protein, 17 aa, Artificial Sequence
  L-FR2 of A56-35G07
LAWYQQKPGQAPRLLIY

SEQ ID NO: 866 - protein, 36 aa, Artificial Sequence
  L-FR3 of A56-35G07
IYGASSRATGIPDRFSGSGSGTDFTLTISSLEPEDF

SEQ ID NO: 867 - protein, 10 aa, Artificial Sequence
  L-FR4 of A56-35G07
FGQGTRLEIK

SEQ ID NO: 868 - protein, 8 aa, Artificial Sequence
  H-CDR1 of A56-36B11
GGNFNAYA

SEQ ID NO: 869 - protein, 8 aa, Artificial Sequence
  H-CDR2 of A56-36B11
IIPFFGSP

SEQ ID NO: 870 - protein, 10 aa, Artificial Sequence
  H-CDR3 of A56-36B11
TRSRDYGMDV

SEQ ID NO: 871 - protein, 11 aa, Artificial Sequence
  L-CDR1 of A56-36B11
QSLVDNDGNTY

SEQ ID NO: 872 - protein, 3 aa, Artificial Sequence
  L-CDR2 of A56-36B11
RVS

SEQ ID NO: 873 - protein, 9 aa, Artificial Sequence
  L-CDR3 of A56-36B11
MQTTHWPPL

SEQ ID NO: 874 - DNA, 756 bp, Artificial Sequence
  SCFV of A56-36B11
caggtgcagctggtacagtctggggctgaggtgaggaggcctgggtcctcggttaaggtctcctgcgagacttctggaggcaacttcaacgcctatgcgatcaactgggtgcgacaggcccctggacaggggcttgaatggatgggaggaatcatccctttctttggttcgccaaactacgcacagaggttccagggcagactcacgatcaccgcggacgaatctacgaggacaacctacatggaattgagcagtctgagatctgaggacacggccgtgtattactgcactagatcacgcgactacgggatggacgtctggggccaagggaccacgatcaccgtctcctcaggcctcgggggcctcggaggaggaggtagtggcggaggaggctccggtggatccagcggtgtgggttccgatattgtgatgacccagactccactctccctgcccgtcatccttggacagccggcctccgtctcctgcaggtctagtcaaagcctcgtagacaatgatggaaatacctacttgcattggtttcagcagaggccaggccaatctccaaggcgcctaatttatagggtttctaaccgggactctggggtcccggacagattcagcggcagtgggtcaggcactgatttcacactcaaaatcagcagggtggaggctgaggatgttggggtttattactgcatgcaaactacacactggcctccccttttcggcggagggaccaaggtggatatcaaa

SEQ ID NO: 875 - protein, 117 aa, Artificial Sequence
  VH2 of A56-36B11
QVQLVQSGAEVRRPGSSVKVSCETSGGNFNAYAINWVRQAPGQGLEWMGGIIPFFGSPNYAQRFQGRLTITADESTRTTYMELSSLRSEDTAVYYCTRSRDYGMDVWGQGTTITVSS

SEQ ID NO: 876 - protein, 112 aa, Artificial Sequence
  VL2 of A56-36B11
DIVMTQTPLSLPVILGQPASVSCRSSQSLVDNDGNTYLHWFQQRPGQSPRRLIYRVSNRDSGVPDRFSGSGSGTDFTLKISRVEAEDVGVYYCMQTTHWPPLFGGGTKVDIK

SEQ ID NO: 877 - protein, 25 aa, Artificial Sequence
  H-FR1 of A56-36B11
QVQLVQSGAEVRRPGSSVKVSCETS

SEQ ID NO: 878 - protein, 17 aa, Artificial Sequence
  H-FR2 of A56-36B11
INWVRQAPGQGLEWMGG

SEQ ID NO: 879 - protein, 38 aa, Artificial Sequence
  H-FR3 of A56-36B11
NYAQRFQGRLTITADESTRTTYMELSSLRSEDTAVYYC

SEQ ID NO: 880 - protein, 11 aa, Artificial Sequence
  H-FR4 of A56-36B11
WGQGTTITVSS

SEQ ID NO: 881 - protein, 26 aa, Artificial Sequence
  L-FR1 of A56-36B11
DIVMTQTPLSLPVILGQPASVSCRSS

SEQ ID NO: 882 - protein, 17 aa, Artificial Sequence
  L-FR2 of A56-36B11
LHWFQQRPGQSPRRLIY

SEQ ID NO: 883 - protein, 36 aa, Artificial Sequence
  L-FR3 of A56-36B11
IYRVSNRDSGVPDRFSGSGSGTDFTLKISRVEAEDV

SEQ ID NO: 884 - protein, 10 aa, Artificial Sequence
  L-FR4 of A56-36B11
FGGGTKVDIK

SEQ ID NO: 885 - protein, 8 aa, Artificial Sequence
  H-CDR1 of A56-41C01
GGSISSHY

SEQ ID NO: 886 - protein, 7 aa, Artificial Sequence
  H-CDR2 of A56-41C01
ISNSGNT

SEQ ID NO: 887 - protein, 11 aa, Artificial Sequence
  H-CDR3 of A56-41C01
ASQRSDGSLDY

SEQ ID NO: 888 - protein, 12 aa, Artificial Sequence
  L-CDR1 of A56-41C01
QSLLDSDDGNTY

SEQ ID NO: 889 - protein, 3 aa, Artificial Sequence
  L-CDR2 of A56-41C01
EVS

SEQ ID NO: 890 - protein, 9 aa, Artificial Sequence
  L-CDR3 of A56-41C01
MQRIEFPYT

SEQ ID NO: 891 - DNA, 759 bp, Artificial Sequence
  SCFV of A56-41C01
caggtgcagctgcaggagtcgggcccaggactggtgaagccttcggagaccctgtccctcacctgcactgtctccggtggctccatcagtagtcactactggagctgggtccggcagcccccagggaagagaccggagtggattgggtacatctctaacagtgggaacacgatctacaacccctccctcaagagtcgagtcaccatatcattaaacacgtccaggaaccaattctccctgcagctgaggtctgtgaccgccgtggacacggccgtgtattactgtgcgagtcaaaggagcgacggatcccttgactaccggggccctggaaccctggtcaccgtctcctcaggcctcgggggcctcggaggaggaggtagtggcggaggaggctccggtggatccagcggtgtgggttccgatattgtgatgacccagactccactctccctgcccgtcacccctggagaggcggcctccatctcctgcaggtctagtcagagcctcttggatagtgatgatggaaacacctatttggactggtacctgcagaagccaggccagcctccacagctcctgatctacgaagtttccaatcggttctctggagtgccagataggttcagtggcagcgggtcagggacagacttcacactgaaaatcagcagggtggaggctgaggatgttggagtttattactgcatgcaacgtatagagtttccttatacttttggccaagggaccaaggtggaaatcaaa

SEQ ID NO: 892 - protein, 117 aa, Artificial Sequence
  VH2 of A56-41C01
QVQLQESGPGLVKPSETLSLTCTVSGGSISSHYWSWVRQPPGKRPEWIGYISNSGNTIYNPSLKSRVTISLNTSRNQFSLQLRSVTAVDTAVYYCASQRSDGSLDYRGPGTLVTVSS

SEQ ID NO: 893 - protein, 113 aa, Artificial Sequence
  VL2 of A56-41C01
DIVMTQTPLSLPVTPGEAASISCRSSQSLLDSDDGNTYLDWYLQKPGQPPQLLIYEVSNRFSGVPDRFSGSGSGTDFTLKISRVEAEDVGVYYCMQRIEFPYTFGQGTKVEIK

SEQ ID NO: 894 - protein, 25 aa, Artificial Sequence
  H-FR1 of A56-41C01
QVQLQESGPGLVKPSETLSLTCTVS

SEQ ID NO: 895 - protein, 17 aa, Artificial Sequence
  H-FR2 of A56-41C01
WSWVRQPPGKRPEWIGY

SEQ ID NO: 896 - protein, 38 aa, Artificial Sequence
  H-FR3 of A56-41C01
IYNPSLKSRVTISLNTSRNQFSLQLRSVTAVDTAVYYC

SEQ ID NO: 897 - protein, 11 aa, Artificial Sequence
  H-FR4 of A56-41C01
RGPGTLVTVSS

SEQ ID NO: 898 - protein, 26 aa, Artificial Sequence
  L-FR1 of A56-41C01
DIVMTQTPLSLPVTPGEAASISCRSS

SEQ ID NO: 899 - protein, 17 aa, Artificial Sequence
  L-FR2 of A56-41C01
LDWYLQKPGQPPQLLIY

SEQ ID NO: 900 - protein, 36 aa, Artificial Sequence
  L-FR3 of A56-41C01
IYEVSNRFSGVPDRFSGSGSGTDFTLKISRVEAEDV

SEQ ID NO: 901 - protein, 10 aa, Artificial Sequence
  L-FR4 of A56-41C01
FGQGTKVEIK

SEQ ID NO: 902 - protein, 8 aa, Artificial Sequence
  H-CDR1 of A56-42H07
GDTFSRYA

SEQ ID NO: 903 - protein, 8 aa, Artificial Sequence
  H-CDR2 of A56-42H07
IIPVLGAA

SEQ ID NO: 904 - protein, 16 aa, Artificial Sequence
  H-CDR3 of A56-42H07
ARDLVRGVTPHYGMDV

SEQ ID NO: 905 - protein, 11 aa, Artificial Sequence
  L-CDR1 of A56-42H07
QSLLHSNGYNY

SEQ ID NO: 906 - protein, 3 aa, Artificial Sequence
  L-CDR2 of A56-42H07
LGS

SEQ ID NO: 907 - protein, 9 aa, Artificial Sequence
  L-CDR3 of A56-42H07
MQARQTPLT

SEQ ID NO: 908 - DNA, 774 bp, Artificial Sequence
  SCFV of A56-42H07
caggtgcagctggtgcagtctggggctgaggtgaagaagcctgggtcctcggtgaaggtctcctgcaaggcttctggagacacgttcagcagatatgctatcagctggatccgacaggcccctggacaagggcctgagtggatgggaaggatcatccctgtccttggtgcagcaaattatgcacggaagttccaggacagagtcacgatcacagcggacaaatccacgactacagcctacatggaactgaccagtctgagatctgaggacacggccgtgtattactgtgcgagagatttagttcggggagttactccacactacggtatggacgtctggggccaagggaccacggtcaccgtctcctcaggcctcgggggcctcggaggaggaggtagtggcggaggaggctccggtggatccagcggtgtgggttccgatattgtgatgacccagactccactctccctgcccgtcacccctggagagccggcctccatctcctgcaggtctagtcagagcctcctgcatagtaatggatacaattatttggattggtacctgcagaagccagggcagtcccctcagctcctgatctatttgggttctagtcgggcctccggggtccctgacaggttcagtggcagtggatcaggcacagattttacactgaaaatcagcagggtggaggctgaagatgttggggtttattactgcatgcaagctcgacaaactcctctcactttcggcggagggaccaaggtagagatcaaa

SEQ ID NO: 909 - protein, 123 aa, Artificial Sequence
  VH2 of A56-42H07
QVQLVQSGAEVKKPGSSVKVSCKASGDTFSRYAISWIRQAPGQGPEWMGRIIPVLGAANYARKFQDRVTITADKSTTTAYMELTSLRSEDTAVYYCARDLVRGVTPHYGMDVWGQGTTVTVSS

SEQ ID NO: 910 - protein, 112 aa, Artificial Sequence
  VL2 of A56-42H07
DIVMTQTPLSLPVTPGEPASISCRSSQSLLHSNGYNYLDWYLQKPGQSPQLLIYLGSSRASGVPDRFSGSGSGTDFTLKISRVEAEDVGVYYCMQARQTPLTFGGGTKVEIK

SEQ ID NO: 911 - protein, 25 aa, Artificial Sequence [sequence omitted]

SEQ ID NO: 912 - protein, 17 aa, Artificial Sequence
  H-FR2 of A56-42H07
ISWIRQAPGQGPEWMGR

SEQ ID NO: 913 - protein, 38 aa, Artificial Sequence
  H-FR3 of A56-42H07
NYARKFQDRVTITADKSTTTAYMELTSLRSEDTAVYYC

SEQ ID NO: 914 - protein, 11 aa, Artificial Sequence
  H-FR4 of A56-42H07
WGQGTTVTVSS

SEQ ID NO: 915 - protein, 26 aa, Artificial Sequence
  L-FR1 of A56-42H07
DIVMTQTPLSLPVTPGEPASISCRSS

SEQ ID NO: 916 - protein, 17 aa, Artificial Sequence
  L-FR2 of A56-42H07
LDWYLQKPGQSPQLLIY

SEQ ID NO: 917 - protein, 36 aa, Artificial Sequence
  L-FR3 of A56-42H07
IYLGSSRASGVPDRFSGSGSGTDFTLKISRVEAEDV

SEQ ID NO: 918 - protein, 10 aa, Artificial Sequence
  L-FR4 of A56-42H07
FGGGTKVEIK

SEQ ID NO: 919 - protein, 8 aa, Artificial Sequence
  H-CDR1 of A56-44G01
GFTFSSYA

SEQ ID NO: 920 - protein, 8 aa, Artificial Sequence
  H-CDR2 of A56-44G01
ISYDGSNK

SEQ ID NO: 921 - protein, 17 aa, Artificial Sequence
  H-CDR3 of A56-44G01
AKDLWGRVGALVGALDL

SEQ ID NO: 922 - protein, 6 aa, Artificial Sequence
  L-CDR1 of A56-44G01
NLRTKY

SEQ ID NO: 923 - protein, 3 aa, Artificial Sequence
  L-CDR2 of A56-44G01
QDT

SEQ ID NO: 924 - protein, 9 aa, Artificial Sequence
  L-CDR3 of A56-44G01
QAWDSGNYV

SEQ ID NO: 925 - DNA, 759 bp, Artificial Sequence
  SCFV of A56-44G01
caggtgcagctggtggagtctgggggaggtgtggtccagcctgggaggtccctgagactctcctgtgcagcctctggattcaccttcagtagctatgctatgcactgggtccgccaggctccaggcaaggggctggagtgggtggcagttatatcatatgatggaagtaataaatactacgcagactccgtgaagggccgattcaccatctccagagacaattccaagaacacgctgtatctgcaaatgaacagtctgagagccgaggacacggccgtgtattactgtgcgaaagatctctgggggcgagtgggagccctcgtcggtgctcttgatttgtggggccaagggacaatgatcaccgtctcctcaggcctcgggggcctcggaggaggaggtagtggcggaggaggctccggtggatccagcggtgtgggttcctcctatgagctgacacagggaccctcactgtccgtgtcgccaggacagacagccaacatcatctgctctggagataacttgcgtactaaatatgtttcttggtaccagcagaagccaggccagtcccctatattggtcatctatcaggacaccaggcggccctcaggcatccctgcgcgattctctggctccaactctgggaacacagccactctgaccatcagcgggacccaggctatggatgaggctgactattactgtcaggcgtgggacagcggcaactatgtcttcggaactgggaccaaggttaccgtccta

SEQ ID NO: 926 - protein, 124 aa, Artificial Sequence
  VH2 of A56-44G01
QVQLVESGGGVVQPGRSLRLSCAASGFTFSSYAMHWVRQAPGKGLEWVAVISYDGSNKYYADSVKGRFTISRDNSKNTLYLQMNSLRAEDTAVYYCAKDLWGRVGALVGALDLWGQGTMITVSS

SEQ ID NO: 927 - protein, 106 aa, Artificial Sequence
  VL2 of A56-44G01
SYELTQGPSLSVSPGQTANIICSGDNLRTKYVSWYQQKPGQSPILVIYQDTRRPSGIPARFSGSNSGNTATLTISGTQAMDEADYYCQAWDSGNYVFGTGTKVTVL

SEQ ID NO: 928 - protein, 25 aa, Artificial Sequence
  H-FR1 of A56-44G01
QVQLVESGGGVVQPGRSLRLSCAAS

SEQ ID NO: 929 - protein, 17 aa, Artificial Sequence
  H-FR2 of A56-44G01
MHWVRQAPGKGLEWVAV

SEQ ID NO: 930 - protein, 38 aa, Artificial Sequence; identical to SEQ ID NO: 505
  H-FR3 of A56-44G01

SEQ ID NO: 931 - protein, 11 aa, Artificial Sequence
  H-FR4 of A56-44G01
WGQGTMITVSS

SEQ ID NO: 932 - protein, 25 aa, Artificial Sequence
  L-FR1 of A56-44G01
SYELTQGPSLSVSPGQTANIICSGD

SEQ ID NO: 933 - protein, 17 aa, Artificial Sequence
  L-FR2 of A56-44G01
VSWYQQKPGQSPILVIY

SEQ ID NO: 934 - protein, 36 aa, Artificial Sequence
  L-FR3 of A56-44G01
IYQDTRRPSGIPARFSGSNSGNTATLTISGTQAMDE

SEQ ID NO: 935 - protein, 10 aa, Artificial Sequence
  L-FR4 of A56-44G01
FGTGTKVTVL

SEQ ID NO: 936 - protein, 8 aa, Artificial Sequence
  H-CDR1 of A56-46A07
GFIFSDSP

SEQ ID NO: 937 - protein, 10 aa, Artificial Sequence
  H-CDR2 of A56-46A07
IGTTASTYAT

SEQ ID NO: 938 - protein, 11 aa, Artificial Sequence
  H-CDR3 of A56-46A07
ARDRSGWSRDY

SEQ ID NO: 939 - protein, 6 aa, Artificial Sequence
  L-CDR1 of A56-46A07
QGIGRS

SEQ ID NO: 940 - protein, 3 aa, Artificial Sequence
  L-CDR2 of A56-46A07
AAS

SEQ ID NO: 941 - protein, 9 aa, Artificial Sequence
  L-CDR3 of A56-46A07
QQVYSYPYS

SEQ ID NO: 942 - DNA, 750 bp, Artificial Sequence
  SCFV of A56-46A07
caggtgcagctggtggagtctgggggaggcttggtccagccgggggggtccctgaaactctcctgtgcagcctctgggttcatcttcagtgactctcctatgcactgggtccgccaggcttccgggaaaggcctggagtgggttggccgcattggaaccacagcttccacttacgcgacagtatatgctgcgtcggtgaaaggcaggttcaccatctccagagatgactcaaagaacacggcttatctgcaaatgaacagtctgagagccgaggacacggccgtgtattactgtgcgagagatagaagtggctggtcccgtgactactggggccagggaaccctggtcaccgtctcctcaggcctcgggggcctcggaggaggaggtagtggcggaggaggctccggtggatccagcggtgtgggttccgacatccagatgacccagtctccatcctccctgtctgcatctgtaggagacagagtcaccatcacttgccgggccagtcagggcattggcaggtctttagcgtggtatcagcaaaaacccgggaaagcccctacagtcctgatctatgctgcatccactttgcacagtggggtcccatcaagattcagcggcgctggatctggaacagatttcgctctcaccatcagccgcctgctacctgaagattttgcaacttattactgtcaacaggtttattcttacccgtacagttttggcctggggaccatgctggagatcaaa

SEQ ID NO: 943 - protein, 120 aa, Artificial Sequence
  VH2 of A56-46A07
QVQLVESGGGLVQPGGSLKLSCAASGFIFSDSPMHWVRQASGKGLEWVGRIGTTASTYATVYAASVKGRFTISRDDSKNTAYLQMNSLRAEDTAVYYCARDRSGWSRDYWGQGTLVTVSS

SEQ ID NO: 944 - protein, 107 aa, Artificial Sequence
  VL2 of A56-46A07
DIQMTQSPSSLSASVGDRVTITCRASQGIGRSLAWYQQKPGKAPTVLIYAASTLHSGVPSRFSGAGSGTDFALTISRLLPEDFATYYCQQVYSYPYSFGLGTMLEIK

SEQ ID NO: 945 - protein, 25 aa, Artificial Sequence
  H-FR1 of A56-46A07
QVQLVESGGGLVQPGGSLKLSCAAS

SEQ ID NO: 946 - protein, 17 aa, Artificial Sequence
  H-FR2 of A56-46A07
MHWVRQASGKGLEWVGR

SEQ ID NO: 947 - protein, 38 aa, Artificial Sequence
  H-FR3 of A56-46A07
VYAASVKGRFTISRDDSKNTAYLQMNSLRAEDTAVYYC

SEQ ID NO: 948 - protein, 11 aa, Artificial Sequence
  H-FR4 of A56-46A07
WGQGTLVTVSS

SEQ ID NO: 949 - protein, 26 aa, Artificial Sequence [sequence omitted]

SEQ ID NO: 950 - protein, 17 aa, Artificial Sequence
  L-FR2 of A56-46A07
LAWYQQKPGKAPTVLIY

SEQ ID NO: 951 - protein, 36 aa, Artificial Sequence
  L-FR3 of A56-46A07
TLHSGVPSRFSGAGSGTDFALTISRLLPEDFATYYC

SEQ ID NO: 952 - protein, 10 aa, Artificial Sequence
  L-FR4 of A56-46A07
FGLGTMLEIK

SEQ ID NO: 953 - protein, 8 aa, Artificial Sequence
  H-CDR1 of A56-50A09
GFTFDDYA

SEQ ID NO: 954 - protein, 8 aa, Artificial Sequence
  H-CDR2 of A56-50A09
ISGDGGST

SEQ ID NO: 955 - protein, 16 aa, Artificial Sequence
  H-CDR3 of A56-50A09
ARVFQYYGLPRGAFDI

SEQ ID NO: 956 - protein, 6 aa, Artificial Sequence
  L-CDR1 of A56-50A09
QVINNY

SEQ ID NO: 957 - protein, 3 aa, Artificial Sequence
  L-CDR2 of A56-50A09
AAS

SEQ ID NO: 958 - protein, 9 aa, Artificial Sequence
  L-CDR3 of A56-50A09
LQHKSYPLT

SEQ ID NO: 959 - DNA, 759 bp, Artificial Sequence
  SCFV of A56-50A09
caggtgcagctggtgcagtctgggggaggtgtggtacagcctggggggtccctgagactctcctgtgcagcctctggattcacctttgatgattatgccatgcactgggtccgtcaagctccagggaagggtctggagtgggtctctcttattagtggggatggtggtagcacatactatgcagactctgtgaagggccgattcaccatctccagagacaacagcaaaaactccctgtatctgcaaatgaacagtctaagagccgaggacacggccgtgtattactgtgcgagagtcttccagtactatgggctaccaaggggtgcttttgatatctggggccaagggacaatgatcaccgtctcctcaggcctcgggggcctcggaggaggaggtagtggcggaggaggctccggtggatccagcggtgtgggttccgacatccagatgacccagtctccatctgccatgtctgcatctataggagacagagtcaccatcacttgtcgggcgagtcaggtcattaacaattatttaatctggtttcagcagaaaccagggaaagtccctaagcgcctgatctatgctgcatccagtttgcaaagtggggtcccatcaaggttcagcggcagtggatctgggacagaattcactctcacaatcagcagcctacagcctgaagattttgcaacttattactgtttacagcataagagttaccctctcactttcggccctgggaccaaagtggaaatcaaa

SEQ ID NO: 960 - protein, 123 aa, Artificial Sequence
  VH2 of A56-50A09
QVQLVQSGGGVVQPGGSLRLSCAASGFTFDDYAMHWVRQAPGKGLEWVSLISGDGGSTYYADSVKGRFTISRDNSKNSLYLQMNSLRAEDTAVYYCARVFQYYGLPRGAFDIWGQGTMITVSS

SEQ ID NO: 961 - protein, 107 aa, Artificial Sequence
  VL2 of A56-50A09
DIQMTQSPSAMSASIGDRVTITCRASQVINNYLIWFQQKPGKVPKRLIYAASSLQSGVPSRFSGSGSGTEFTLTISSLQPEDFATYYCLQHKSYPLTFGPGTKVEIK

SEQ ID NO: 962 - protein, 25 aa, Artificial Sequence
  H-FR1 of A56-50A09
QVQLVQSGGGVVQPGGSLRLSCAAS

SEQ ID NO: 963 - protein, 17 aa, Artificial Sequence
  H-FR2 of A56-50A09
MHWVRQAPGKGLEWVSL

SEQ ID NO: 964 - protein, 38 aa, Artificial Sequence
  H-FR3 of A56-50A09
YYADSVKGRFTISRDNSKNSLYLQMNSLRAEDTAVYYC

SEQ ID NO: 965 - protein, 11 aa, Artificial Sequence
  H-FR4 of A56-50A09
WGQGTMITVSS

SEQ ID NO: 966 - protein, 26 aa, Artificial Sequence
  L-FR1 of A56-50A09
DIQMTQSPSAMSASIGDRVTITCRAS

SEQ ID NO: 967 - protein, 17 aa, Artificial Sequence
  L-FR2 of A56-50A09
LIWFQQKPGKVPKRLIY

SEQ ID NO: 968 - protein, 36 aa, Artificial Sequence
  L-FR3 of A56-50A09
IYAASSLQSGVPSRFSGSGSGTEFTLTISSLQPEDF

SEQ ID NO: 969 - protein, 10 aa, Artificial Sequence
  L-FR4 of A56-50A09
FGPGTKVEIK

SEQ ID NO: 970 - protein, 10 aa, Artificial Sequence
  H-CDR1 of A56-50A11
GFSLSNARMG

SEQ ID NO: 971 - protein, 7 aa, Artificial Sequence
  H-CDR2 of A56-50A11
IFSSDEK

SEQ ID NO: 972 - protein, 15 aa, Artificial Sequence
  H-CDR3 of A56-50A11
ARTSRISPTGEAFDI

SEQ ID NO: 973 - protein, 6 aa, Artificial Sequence
  L-CDR1 of A56-50A11
QNIGSI

SEQ ID NO: 974 - protein, 3 aa, Artificial Sequence
  L-CDR2 of A56-50A11
YAS

SEQ ID NO: 975 - protein, 9 aa, Artificial Sequence
  L-CDR3 of A56-50A11
HQSRSLPQT

SEQ ID NO: 976 - DNA, 759 bp, Artificial Sequence
  SCFV of A56-50A11
caggtcaccttgagggagtctggtcctgtgctggtgaaacccacagagaccctcacgctgacctgcaccgtctctggattctcactcagcaatgctagaatgggtgtgggctggatccgtcagcccccagggaaggccctggagtggctcgcccacattttttcgagcgacgaaaaatcttttagggcatctctgaagagcaggctcaccatctccaaggacacctccaaaagccaggtggtccttacaatgaccaacatggatcctgtagacacagccatatattactgtgcacggacatcccgtatatcaccaactggggaagcttttgatatctggggccaagggacagtggtcaccgtctcctcaggcctcgggggcctcggaggaggaggtagtggcggaggaggctccggtggatccagcggtgtgggttccgatattgtgatgacccagactccagactttcggtctgtggctccagcggagacagtcaccatcacctgccgggccagtcagaacattggtagtattttacactggtaccagcagaaaccaaatcagtctccagtcctcctcatcaagtatgcttcccagtccatctcaggggtcccgtcgaggttcagtggcagtggatctgggacagagttcaccctcacgatctacagcctggaagctgaagatgctgcaacgtattactgtcatcagagtaggagtttacctcagacttttggccaggggaccaagctggaggtcaaa

SEQ ID NO: 977 - protein, 123 aa, Artificial Sequence
  VH2 of A56-50A11
QVTLRESGPVLVKPTETLTLTCTVSGFSLSNARMGVGWIRQPPGKALEWLAHIFSSDEKSFRASLKSRLTISKDTSKSQVVLTMTNMDPVDTAIYYCARTSRISPTGEAFDIWGQGTVVTVSS

SEQ ID NO: 978 - protein, 107 aa, Artificial Sequence
  VL2 of A56-50A11
DIVMTQTPDFRSVAPAETVTITCRASQNIGSILHWYQQKPNQSPVLLIKYASQSISGVPSRFSGSGSGTEFTLTIYSLEAEDAATYYCHQSRSLPQTFGQGTKLEVK

SEQ ID NO: 979 - protein, 25 aa, Artificial Sequence
  H-FR1 of A56-50A11
QVTLRESGPVLVKPTETLTLTCTVS

SEQ ID NO: 980 - protein, 17 aa, Artificial Sequence
  H-FR2 of A56-50A11
VGWIRQPPGKALEWLAH

SEQ ID NO: 981 - protein, 38 aa, Artificial Sequence
  H-FR3 of A56-50A11
SFRASLKSRLTISKDTSKSQVVLTMTNMDPVDTAIYYC

SEQ ID NO: 982 - protein, 11 aa, Artificial Sequence
  H-FR4 of A56-50A11
WGQGTVVTVSS

SEQ ID NO: 983 - protein, 26 aa, Artificial Sequence
  L-FR1 of A56-50A11
DIVMTQTPDFRSVAPAETVTITCRAS

SEQ ID NO: 984 - protein, 17 aa, Artificial Sequence
  L-FR2 of A56-50A11
LHWYQQKPNQSPVLLIK

SEQ ID NO: 985 - protein, 36 aa, Artificial Sequence
  L-FR3 of A56-50A11
IKYASQSISGVPSRFSGSGSGTEFTLTIYSLEAEDA

SEQ ID NO: 986 - protein, 10 aa, Artificial Sequence
  L-FR4 of A56-50A11
FGQGTKLEVK

SEQ ID NO: 987 - protein, 8 aa, Artificial Sequence
  H-CDR1 of A56-54C01
GFTFVVFP

SEQ ID NO: 988 - protein, 8 aa, Artificial Sequence
  H-CDR2 of A56-54C01
ISGSGGST

SEQ ID NO: 989 - protein, 14 aa, Artificial Sequence
  H-CDR3 of A56-54C01
AIGGPLTSHNWFDP

SEQ ID NO: 990 - protein, 8 aa, Artificial Sequence
  L-CDR1 of A56-54C01
SGSIGSSY

SEQ ID NO: 991 - protein, 3 aa, Artificial Sequence
  L-CDR2 of A56-54C01
EDA

SEQ ID NO: 992 - protein, 10 aa, Artificial Sequence
  L-CDR3 of A56-54C01
QSYDGSNHFV

SEQ ID NO: 993 - DNA, 765 bp, Artificial Sequence
  SCFV of A56-54C01
caggtgcagctggtagagtcggggggaggcgtggtccagcctggggggtccctgaaactctcctgtgcagcctctggattcaccttcgttgtctttcctatgcgctgggtccgccaggctccagggaaggggctggagtgggtctcagctattagtggtagtggtggtagcacatactactcagactccgtgaagggccggttcaccatctccagagacaattccaagaacaccctgtatctgcaaatgaacagtctgagagccgaggacacggccgtgtattactgtgcgattgggggtcctttgacttcccacaactggttcgacccctggggccagggaaccctggtcaccgtctcctcaggcctcgggggcctcggaggaggaggtagtggcggaggaggctccggtggatccagcggtgtgggttccaattttatgctgactcagccccactctgtgtcggagtctccggggaagacggtaaccatctcctgcacccgcagcagtggcagcattggcagcagctatatacagtggtaccagcagcgcccgggcagtgcccccaccactgtgatgtatgaagatgccgaaagaccctctggcgtccctgatcggttctctggctccatcgacagctcctccaactctgcctccctcaccatctctggactgaagactgaggacgaggctgactactactgtcagtcttatgatggcagcaatcatttcgtgttcggcggagggaccaagctgaccgtccta

SEQ ID NO: 994 - protein, 121 aa, Artificial Sequence
  VH2 of A56-54C01
QVQLVESGGGVVQPGGSLKLSCAASGFTFVVFPMRWVRQAPGKGLEWVSAISGSGGSTYYSDSVKGRFTISRDNSKNTLYLQMNSLRAEDTAVYYCAIGGPLTSHNWFDPWGQGTLVTVSS

SEQ ID NO: 995 - protein, 111 aa, Artificial Sequence
  VL2 of A56-54C01
NFMLTQPHSVSESPGKTVTISCTRSSGSIGSSYIQWYQQRPGSAPTTVMYEDAERPSGVPDRFSGSIDSSSNSASLTISGLKTEDEADYYCQSYDGSNHFVFGGGTKLTVL

SEQ ID NO: 996 - protein, 25 aa, Artificial Sequence
  H-FR1 of A56-54C01
QVQLVESGGGVVQPGGSLKLSCAAS

SEQ ID NO: 997 - protein, 17 aa, Artificial Sequence
  H-FR2 of A56-54C01
MRWVRQAPGKGLEWVSA

SEQ ID NO: 998 - protein, 38 aa, Artificial Sequence
  H-FR3 of A56-54C01
YYSDSVKGRFTISRDNSKNTLYLQMNSLRAEDTAVYYC

SEQ ID NO: 999 - protein, 11 aa, Artificial Sequence
  H-FR4 of A56-54C01
WGQGTLVTVSS

SEQ ID NO: 1000 - protein, 25 aa, Artificial Sequence
  L-FR1 of A56-54C01
NFMLTQPHSVSESPGKTVTISCTRS

SEQ ID NO: 1001 - protein, 17 aa, Artificial Sequence
  L-FR2 of A56-54C01
IQWYQQRPGSAPTTVMY

SEQ ID NO: 1002 - protein, 36 aa, Artificial Sequence
  L-FR3 of A56-54C01
MYEDAERPSGVPDRFSGSIDSSSNSASLTISGLKTE

SEQ ID NO: 1003 - protein, 10 aa, Artificial Sequence
  L-FR4 of A56-54C01
FGGGTKLTVL

SEQ ID NO: 1004 - protein, 8 aa, Artificial Sequence
  H-CDR1 of A56-59A11
GFSLSNYG

SEQ ID NO: 1005 - protein, 8 aa, Artificial Sequence
  H-CDR2 of A56-59A11
ISASSSYK

SEQ ID NO: 1006 - protein, 15 aa, Artificial Sequence
  H-CDR3 of A56-59A11
ARDRYFYGSGSYPPA

SEQ ID NO: 1007 - protein, 11 aa, Artificial Sequence
  L-CDR1 of A56-59A11
QSLLQTNGYNY

SEQ ID NO: 1008 - protein, 3 aa, Artificial Sequence
  L-CDR2 of A56-59A11
LGS

SEQ ID NO: 1009 - protein, 8 aa, Artificial Sequence
  L-CDR3 of A56-59A11
MHSLQTPT

SEQ ID NO: 1010 - DNA, 768 bp, Artificial Sequence
  SCFV of A56-59A11
caggtgcagctggtggagtctgggggaggcgtggtccagcctgggaggtccctgagactctcctgtgcagcgtctggattcagcctcagtaactatggcatgcactgggtccgccaggctccaggcaaggggctggagtgggtatcatatattagtgctagtagtagttacaagaagtacgcagactcagtgaagggccgattcaccatctccagagacaacgccaagaactccctgtatctgcaaatgaacagtctgagagccgaggacacggccgtgtattactgtgcgagagatcgatatttctatggttcggggagttatccccccgccttgggccggggaaccctggtcaccgtctcctcaggcctcgggggcctcggaggaggaggtagtggcggaggaggctccggtggatccagcggtgtgggttccgatattgtgatgacccagactccactctccctgcccgttacccctggagagccggcctccatctcctgcaggtctagtcagagcctcctgcagacgaatggatacaactatttggattggtacctgcagaagccagggcagactccacagctcctgatctatttgggttctaatcgggcctccggggtccctgacaggttcagtggcagtggatcaggcacagattttacactgaaaatcagcagagtggaggctgaggatgttggggtttattactgcatgcattctctacaaactccgactttcggccctgggaccaaagtagaaatcaaa

SEQ ID NO: 1011 - protein, 122 aa, Artificial Sequence
  VH2 of A56-59A11
QVQLVESGGGVVQPGRSLRLSCAASGFSLSNYGMHWVRQAPGKGLEWVSYISASSSYKKYADSVKGRFTISRDNAKNSLYLQMNSLRAEDTAVYYCARDRYFYGSGSYPPALGRGTLVTVSS

SEQ ID NO: 1012 - protein, 111 aa, Artificial Sequence
  VL2 of A56-59A11
DIVMTQTPLSLPVTPGEPASISCRSSQSLLQTNGYNYLDWYLQKPGQTPQLLIYLGSNRASGVPDRFSGSGSGTDFTLKISRVEAEDVGVYYCMHSLQTPTFGPGTKVEIK

SEQ ID NO: 1013 - protein, 25 aa, Artificial Sequence
  H-FR1 of A56-59A11
QVQLVESGGGVVQPGRSLRLSCAAS

SEQ ID NO: 1014 - protein, 17 aa, Artificial Sequence
  H-FR2 of A56-59A11
MHWVRQAPGKGLEWVSY

SEQ ID NO: 1015 - protein, 38 aa, Artificial Sequence
  H-FR3 of A56-59A11
KYADSVKGRFTISRDNAKNSLYLQMNSLRAEDTAVYYC

SEQ ID NO: 1016 - protein, 11 aa, Artificial Sequence
  H-FR4 of A56-59A11
LGRGTLVTVSS

SEQ ID NO: 1017 - protein, 26 aa, Artificial Sequence
  L-FR1 of A56-59A11
DIVMTQTPLSLPVTPGEPASISCRSS

SEQ ID NO: 1018 - protein, 17 aa, Artificial Sequence
  L-FR2 of A56-59A11
LDWYLQKPGQTPQLLIY

SEQ ID NO: 1019 - protein, 36 aa, Artificial Sequence; identical to SEQ ID NO: 16
  L-FR3 of A56-59A11

SEQ ID NO: 1020 - protein, 10 aa, Artificial Sequence
  L-FR4 of A56-59A11
FGPGTKVEIK

SEQ ID NO: 1021 - protein, 8 aa, Artificial Sequence
  H-CDR1 of A56-59E12
GFNFGDYA

SEQ ID NO: 1022 - protein, 10 aa, Artificial Sequence
  H-CDR2 of A56-59E12
TSSKHYGGTI

SEQ ID NO: 1023 - protein, 14 aa, Artificial Sequence
  H-CDR3 of A56-59E12
AKGKWLRFDSPFDS

SEQ ID NO: 1024 - protein, 11 aa, Artificial Sequence
  L-CDR1 of A56-59E12
QSLLHNNGNKF

SEQ ID NO: 1025 - protein, 3 aa, Artificial Sequence
  L-CDR2 of A56-59E12
LGS

SEQ ID NO: 1026 - protein, 9 aa, Artificial Sequence
  L-CDR3 of A56-59E12
MQALRTPWT

SEQ ID NO: 1027 - DNA, 774 bp, Artificial Sequence
  SCFV of A56-59E12
caggtgcagctggtgcagtctgggggaggcttggtaaagccagggcggtcccagagactctcctgtacaggttctggattcaactttggtgattatgccatcagttggatccgccaggctccagggaaggggctggagtgggtcggcttcactagcagcaaacattatggtgggacaatagactacgccgcgtctgtgaaaggcagattcatcatctcaagagatgattcgaaaagcaccgcctatctgcaaatgaacagtctgagagccgaggacacggccgtgtattactgcgcgaaaggaaagtggctacgattcgattcgccatttgactcctggggccagggaaccctggtcaccgtctcctcaggcctcgggggcctcggaggaggaggtagtggcggaggaggctccggtggatccagcggtgtgggttccgatattgtgatgacccagactccactctccctgcccgtcacccttggagagccggcctccatctcctgcaggtctagtcagagcctcctgcataataatggaaacaagtttttcgattggtacctgcagaagccagggcagtctccacagctcctgatctatttgggttctaatcgggcctccggggtccctgacaggttcagtggcagtggatcaggcacagattttgcactgaagatcagtagagtggaggctgaggatgttgggctttattattgcatgcaagctctccgaactccgtggacgttcggccaagggaccaaggtggaaatcaaa

SEQ ID NO: 1028 - protein, 123 aa, Artificial Sequence
  VH2 of A56-59E12
QVQLVQSGGGLVKPGRSQRLSCTGSGFNFGDYAISWIRQAPGKGLEWVGFTSSKHYGGTIDYAASVKGRFIISRDDSKSTAYLQMNSLRAEDTAVYYCAKGKWLRFDSPFDSWGQGTLVTVSS

SEQ ID NO: 1029 - protein, 112 aa, Artificial Sequence
  VL2 of A56-59E12
DIVMTQTPLSLPVTLGEPASISCRSSQSLLHNNGNKFFDWYLQKPGQSPQLLIYLGSNRASGVPDRFSGSGSGTDFALKISRVEAEDVGLYYCMQALRTPWTFGQGTKVEIK

SEQ ID NO: 1030 - protein, 25 aa, Artificial Sequence
  H-FR1 of A56-59E12
QVQLVQSGGGLVKPGRSQRLSCTGS

SEQ ID NO: 1031 - protein, 17 aa, Artificial Sequence
  H-FR2 of A56-59E12
ISWIRQAPGKGLEWVGF

SEQ ID NO: 1032 - protein, 38 aa, Artificial Sequence
  H-FR3 of A56-59E12
DYAASVKGRFIISRDDSKSTAYLQMNSLRAEDTAVYYC

SEQ ID NO: 1033 - protein, 11 aa, Artificial Sequence
  H-FR4 of A56-59E12
WGQGTLVTVSS

SEQ ID NO: 1034 - protein, 26 aa, Artificial Sequence
  L-FR1 of A56-59E12
DIVMTQTPLSLPVTLGEPASISCRSS

SEQ ID NO: 1035 - protein, 17 aa, Artificial Sequence
  L-FR2 of A56-59E12
FDWYLQKPGQSPQLLIY

SEQ ID NO: 1036 - protein, 36 aa, Artificial Sequence
  L-FR3 of A56-59E12
IYLGSNRASGVPDRFSGSGSGTDFALKISRVEAEDV

SEQ ID NO: 1037 - protein, 10 aa, Artificial Sequence
  L-FR4 of A56-59E12
FGQGTKVEIK

SEQ ID NO: 1038 - protein, 310 aa, Artificial Sequence
  amino acid sequence for A56 protein
MTRLPILLLLISLVYATPFPQTSKKIGDDATLSCNRNNTNDYVVMSAWYKEPNSIILLAAKSDVLYFDNYTKDKISYDSPYDDLVTTITIKSLTARDAGTYVCAFFMTSPTNDTDKVDYEEYSTELIVNTDSESTIDIILSGSTHSPETSSEKPEDIDNFNCSSVFEIATPEPITDNVEDHTDTVTYTSDSINTVSASSGESTTDETPEPITDKEEDHTVTDTVSYTTVSTSSGIVTTKSTTDDAYNDNDTVPSTTVGSSTTSISNYKTKDFVEIFGITALIILSAVAIFCITYYICNKRSRKYKTENKP

SEQ ID NO: 1039 - DNA, 930 bp, Artificial Sequence
  nucleotide sequence of A56 protein
atgacacgattaccaatacttttgttactaatatcattagtatacgctacaccttttcctcagacatctaaaaaaataggtgatgatgcaactctatcatgtaatcgaaataatacaaatgactacgttgttatgagtgcttggtataaggagcccaattccattattcttttagctgctaaaagcgacgtcttgtattttgataattataccaaggataaaatatcttacgactctccatacgatgatctagttacaactatcacaattaaatcattgactgctagagatgccggtacttatgtatgtgcattctttatgacatcacctacaaatgacactgataaagtagattatgaagaatactccacagagttgattgtaaatacagatagtgaatcgactatagacataatactatctggatctacacattcaccagaaactagttctgagaaaccagaggatatagataattttaattgctcgtcggtattcgaaatcgcgactccggaaccaattactgataatgtagaagatcatacagacaccgtcacatacactagtgatagcattaatacagtaagtgcatcatctggagaatccacaacagacgagactccggaaccaattactgataaagaagaagatcatacagtcacagacactgtctcatacactacagtaagtacatcatctggaattgtcactactaaatcaaccaccgatgatacgtacaatgataatgatacagtaccaccaactactgtaggcagtagtacaacctctattagcaattataaaaccaaggactttgtagaaatatttggtattaccgcattaattatattgtcggccgtggcaatattctgtattacgtattatatatgtaataaacgttcacgtaaatacaaaacagagaacaagccg

SEQ ID NO: 1040 - protein, 270 aa, Artificial Sequence
  amino acid sequence for A56 protein fragment (BN-A56-S)
MTRLPILLLLISLVYATPFPQTSKKIGDDATLSCNRNNTNDYVVMSAWYKEPNSIILLAAKSDVLYFDNYTKDKISYDSPYDDLVTTITIKSLTARDAGTYVCAFFMTSPTNDTDKVDYEEYSTELIVNTDSESTIDIILSGSTHSPETSSEKPEDIDNFNCSSVFEIATPEPITDNVEDHTDTVTYTSDSINTVSASSGESTTDETPEPITDKEEDHTVTDTVSYTTVSTSSGIVTTKSTTDDAYNDNDTVPSTTVGSSTTSISNYKTK

SEQ ID NO: 1041 - DNA, 810 bp, Artificial Sequence
  nucleotide sequence of A56 protein fragment (BN-A56-S)
atgacacgattaccaatacttttgttactaatatcattagtatacgctacaccttttcctcagacatctaaaaaaataggtgatgatgcaactctatcatgtaatcgaaataatacaaatgactacgttgttatgagtgcttggtataaggagcccaattccattattcttttagctgctaaaagcgacgtcttgtattttgataattataccaaggataaaatatcttacgactctccatacgatgatctagttacaactatcacaattaaatcattgactgctagagatgccggtacttatgtatgtgcattctttatgacatcacctacaaatgacactgataaagtagattatgaagaatactccacagagttgattgtaaatacagatagtgaatcgactatagacataatactatctggatctacacattcaccagaaactagttctgagaaaccagaggatatagataattttaattgctcgtcggtattcgaaatcgcgactccggaaccaattactgataatgtagaagatcatacagacaccgtcacatacactagtgatagcattaatacagtaagtgcatcatctggagaatccacaacagacgagactccggaaccaattactgataaagaagaagatcatacagtcacagacactgtctcatacactacagtaagtacatcatctggaattgtcactactaaatcaaccaccgatgatacgtacaatgataatgatacagtaccaccaactactgtaggcagtagtacaacctctattagcaattataaaaccaag

SEQ ID NO: 1042 - protein, 300 aa, Artificial Sequence
  amino acid sequence for A56 protein fragment (BN-A56-17)
TPFPQTSKKIGDDATLSCNRNNTNDYVVMSAWYKEPNSIILLAAKSDVLYFDNYTKDKISYDSPYDDLVTTITIKSLTARDAGTYVCAFFMTSPTNDTDKVDYEEGGGGGGYSTELIVNTDSESTIDIILSGSTHSPETSSEKPEDIDNFNCSSVFEIATPEPITDNVEDHTDTVTYTSDSINTVSASSGESTTDETPEPITDKEEDHTVTDTVSYTTVSTSSGIVTTKSTTDDAYNDNDTVPSTTVGSSTTSISNYKTKDFVEIFGITALIILSAVAIFCITYYICNKRSRKYKTENKP

SEQ ID NO: 1043 - DNA, 900 bp, Artificial Sequence
  nucleotide sequence of A56 protein fragment (BN-A56-17)
acaccttttcctcagacatctaaaaaaataggtgatgatgcaactctatcatgtaatcgaaataatacaaatgactacgttgttatgagtgcttggtataaggagcccaattccattattcttttagctgctaaaagcgacgtcttgtattttgataattataccaaggataaaatatcttacgactctccatacgatgatctagttacaactatcacaattaaatcattgactgctagagatgccggtacttatgtatgtgcattctttatgacatcacctacaaatgacactgataaagtagattatgaagaaggcggcggcggcggcggctactccacagagttgattgtaaatacagatagtgaatcgactatagacataatactatctggatctacacattcaccagaaactagttctgagaaaccagaggatatagataattttaattgctcgtcggtattcgaaatcgcgactccggaaccaattactgataatgtagaagatcatacagacaccgtcacatacactagtgatagcattaatacagtaagtgcatcatctggagaatccacaacagacgagactccggaaccaattactgataaagaagaagatcatacagtcacagacactgtctcatacactacagtaagtacatcatctggaattgtcactactaaatcaaccaccgatgatacgtacaatgataatgatacagtaccaccaactactgtaggcagtagtacaacctctattagcaattataaaaccaaggactttgtagaaatatttggtattaccgcattaattatattgtcggccgtggcaatattctgtattacgtattatatatgtaataaacgttcacgtaaatacaaaacagagaacaagccg

SEQ ID NO: 1044 - protein, 267 aa, Artificial Sequence
  amino acid sequence for A56 protein fragment (BN-A56-170)
MTRLPILLLLISLVYATPFPQTSKKIGDDATLSCNRNNTNDYVVMSAWYKEPNSIILLAAKSDVLYFDNYTKDKISYDSPYDDLVTTITIKSLTARDAGTYVCAFFMTSPTNDTDKVDYEEGGGGGGPEPITDNVEDHTDTVTYTSDSINTVSASSGESTTDETPEPITDKEEDHTVTDTVSYTTVSTSSGIVTTKSTTDDAYNDNDTVPSTTVGSSTTSISNYKTKDFVEIFGITALIILSAVAIFCITYYICNKRSRKYKTENKP

SEQ ID NO: 1045 - DNA, 801 bp, Artificial Sequence
  nucleotide sequence of A56 protein fragment (BN-A56-170)
atgacacgattaccaatacttttgttactaatatcattagtatacgctacaccttttcctcagacatctaaaaaaataggtgatgatgcaactctatcatgtaatcgaaataatacaaatgactacgttgttatgagtgcttggtataaggagcccaattccattattcttttagctgctaaaagcgacgtcttgtattttgataattataccaaggataaaatatcttacgactctccatacgatgatctagttacaactatcacaattaaatcattgactgctagagatgccggtacttatgtatgtgcattctttatgacatcacctacaaatgacactgataaagtagattatgaagaaggcggcggcggcggcggcccggaaccaattactgataatgtagaagatcatacagacaccgtcacatacactagtgatagcattaatacagtaagtgcatcatctggagaatccacaacagacgagactccggaaccaattactgataaagaagaagatcatacagtcacagacactgtctcatacactacagtaagtacatcatctggaattgtcactactaaatcaaccaccgatgatacgtacaatgataatgatacagtaccaccaactactgtaggcagtagtacaacctctattagcaattataaaaccaaggactttgtagaaatatttggtattaccgcattaattatattgtcggccgtggcaatattctgtattacgtattatatatgtaataaacgttcacgtaaatacaaaacagagaacaagccg

SEQ ID NO: 1046 - protein, 197 aa, Artificial Sequence
  amino acid sequence for A56 protein fragment (BN-A56-240)
MTRLPILLLLISLVYATPFPQTSKKIGDDATLSCNRNNTNDYVVMSAWYKEPNSIILLAAKSDVLYFDNYTKDKISYDSPYDDLVTTITIKSLTARDAGTYVCAFFMTSPTNDTDKVDYEEGGGGGGTTDDAYNDNDTVPSTTVGSSTTSISNYKTKDFVEIFGITALIILSAVAIFCITYYICNKRSRKYKTENKP

SEQ ID NO: 1047 - DNA, 591 bp, Artificial Sequence
  nucleotide sequence of A56 protein fragment (BN-A56-240)
atgacacgattaccaatacttttgttactaatatcattagtatacgctacaccttttcctcagacatctaaaaaaataggtgatgatgcaactctatcatgtaatcgaaataatacaaatgactacgttgttatgagtgcttggtataaggagcccaattccattattcttttagctgctaaaagcgacgtcttgtattttgataattataccaaggataaaatatcttacgactctccatacgatgatctagttacaactatcacaattaaatcattgactgctagagatgccggtacttatgtatgtgcattctttatgacatcacctacaaatgacactgataaagtagattatgaagaaggcggcggcggcggcggcaccaccgatgatacgtacaatgataatgatacagtaccaccaactactgtaggcagtagtacaacctctattagcaattataaaaccaaggactttgtagaaatatttggtattaccgcattaattatattgtcggccgtggcaatattctgtattacgtattatatatgtaataaacgttcacgtaaatacaaaacagagaacaagccg

SEQ ID NO: 1048 - protein, 167 aa, Artificial Sequence
  amino acid sequence for A56 protein fragment (BN-A56-276)
MTRLPILLLLISLVYATPFPQTSKKIGDDATLSCNRNNTNDYVVMSAWYKEPNSIILLAAKSDVLYFDNYTKDKISYDSPYDDLVTTITIKSLTARDAGTYVCAFFMTSPTNDTDKVDYEEGGGGGGDFVEIFGITALIILSAVAIFCITYYICNKRSRKYKTENKP

SEQ ID NO: 1049 - DNA, 501 bp, Artificial Sequence
  nucleotide sequence of A56 protein fragment (BN-A56-276)
atgacacgattaccaatacttttgttactaatatcattagtatacgctacaccttttcctcagacatctaaaaaaataggtgatgatgcaactctatcatgtaatcgaaataatacaaatgactacgttgttatgagtgcttggtataaggagcccaattccattattcttttagctgctaaaagcgacgtcttgtattttgataattataccaaggataaaatatcttacgactctccatacgatgatctagttacaactatcacaattaaatcattgactgctagagatgccggtacttatgtatgtgcattctttatgacatcacctacaaatgacactgataaagtagattatgaagaaggcggcggcggcggcggcgactttgtagaaatatttggtattaccgcattaattatattgtcggccgtggcaatattctgtattacgtattatatatgtaataaacgttcacgtaaatacaaaacagagaacaagccg

SEQ ID NO: 1050 - protein, 205 aa, Artificial Sequence
  amino acid sequence for A56 protein fragment (A56-121)
MTRLPILLLLISLVYAYSTELIVNTDSESTIDIILSGSTHSPETSSEKPEDIDNFNCSSVFEIATPEPITDNVEDHTDTVTYTSDSINTVSASSGESTTDETPEPITDKEEDHTVTDTVSYTTVSTSSGIVTTKSTTDDAYNDNDTVPSTTVGSSTTSISNYKTKDFVEIFGITALIILSAVAIFCITYYICNKRSRKYKTENKP

SEQ ID NO: 1051 - DNA, 615 bp, Artificial Sequence
  nucleotide sequence of A56 protein fragment (A56-121)
atgacacgattaccaatacttttgttactaatatcattagtatacgcttactccacagagttgattgtaaatacagatagtgaatcgactatagacataatactatctggatctacacattcaccagaaactagttctgagaaaccagaggatatagataattttaattgctcgtcggtattcgaaatcgcgactccggaaccaattactgataatgtagaagatcatacagacaccgtcacatacactagtgatagcattaatacagtaagtgcatcatctggagaatccacaacagacgagactccggaaccaattactgataaagaagaagatcatacagtcacagacactgtctcatacactacagtaagtacatcatctggaattgtcactactaaatcaaccaccgatgatacgtacaatgataatgatacagtaccaccaactactgtaggcagtagtacaacctctattagcaattataaaaccaaggactttgtagaaatatttggtattaccgcattaattatattgtcggccgtggcaatattctgtattacgtattatatatgtaataaacgttcacgtaaatacaaaacagagaacaagccg

SEQ ID NO: 1052 - protein, 189 aa, Artificial Sequence
  amino acid sequence for A56 protein fragment (A56-17)
YSTELIVNTDSESTIDIILSGSTHSPETSSEKPEDIDNFNCSSVFEIATPEPITDNVEDHTDTVTYTSDSINTVSASSGESTTDETPEPITDKEEDHTVTDTVSYTTVSTSSGIVTTKSTTDDAYNDNDTVPSTTVGSSTTSISNYKTKDFVEIFGITALIILSAVAIFCITYYICNKRSRKYKTENKP

SEQ ID NO: 1053 - DNA, 567 bp, Artificial Sequence
  nucleotide sequence of A56 protein fragment (A56-17)
tactccacagagttgattgtaaatacagatagtgaatcgactatagacataatactatctggatctacacattcaccagaaactagttctgagaaaccagaggatatagataattttaattgctcgtcggtattcgaaatcgcgactccggaaccaattactgataatgtagaagatcatacagacaccgtcacatacactagtgatagcattaatacagtaagtgcatcatctggagaatccacaacagacgagactccggaaccaattactgataaagaagaagatcatacagtcacagacactgtctcatacactacagtaagtacatcatctggaattgtcactactaaatcaaccaccgatgatacgtacaatgataatgatacagtaccaccaactactgtaggcagtagtacaacctctattagcaattataaaaccaaggactttgtagaaatatttggtattaccgcattaattatattgtcggccgtggcaatattctgtattacgtattatatatgtaataaacgttcacgtaaatacaaaacagagaacaagccg

SEQ ID NO: 1054 - protein, 165 aa, Artificial Sequence
  amino acid sequence for A56 protein fragment (A56-121S)
MTRLPILLLLISLVYAYSTELIVNTDSESTIDIILSGSTHSPETSSEKPEDIDNFNCSSVFEIATPEPITDNVEDHTDTVTYTSDSINTVSASSGESTTDETPEPITDKEEDHTVTDTVSYTTVSTSSGIVTTKSTTDDAYNDNDTVPSTTVGSSTTSISNYKTK

SEQ ID NO: 1055 - DNA, 495 bp, Artificial Sequence
  nucleotide sequence of A56 protein fragment (A56-121S)
atgacacgattaccaatacttttgttactaatatcattagtatacgcttactccacagagttgattgtaaatacagatagtgaatcgactatagacataatactatctggatctacacattcaccagaaactagttctgagaaaccagaggatatagataattttaattgctcgtcggtattcgaaatcgcgactccggaaccaattactgataatgtagaagatcatacagacaccgtcacatacactagtgatagcattaatacagtaagtgcatcatctggagaatccacaacagacgagactccggaaccaattactgataaagaagaagatcatacagtcacagacactgtctcatacactacagtaagtacatcatctggaattgtcactactaaatcaaccaccgatgatacgtacaatgataatgatacagtaccaccaactactgtaggcagtagtacaacctctattagcaattataaaaccaag

SEQ ID NO: 1056 - protein, 156 aa, Artificial Sequence
  amino acid sequence for A56 protein fragment (A56-170)
MTRLPILLLLISLVYAPEPITDNVEDHTDTVTYTSDSINTVSASSGESTTDETPEPITDKEEDHTVTDTVSYTTVSTSSGIVTTKSTTDDAYNDNDTVPSTTVGSSTTSISNYKTKDFVEIFGITALIILSAVAIFCITYYICNKRSRKYKTENKP

SEQ ID NO: 1057 - DNA, 468 bp, Artificial Sequence
  nucleotide sequence of A56 protein fragment (A56-170)
atgacacgattaccaatacttttgttactaatatcattagtatacgctccggaaccaattactgataatgtagaagatcatacagacaccgtcacatacactagtgatagcattaatacagtaagtgcatcatctggagaatccacaacagacgagactccggaaccaattactgataaagaagaagatcatacagtcacagacactgtctcatacactacagtaagtacatcatctggaattgtcactactaaatcaaccaccgatgatacgtacaatgataatgatacagtaccaccaactactgtaggcagtagtacaacctctattagcaattataaaaccaaggactttgtagaaatatttggtattaccgcattaattatattgtcggccgtggcaatattctgtattacgtattatatatgtaataaacgttcacgtaaatacaaaacagagaacaagccg

SEQ ID NO: 1058 - protein, 86 aa, Artificial Sequence
  amino acid sequence for A56 protein fragment (A56-240)
MTRLPILLLLISLVYATTDDAYNDNDTVPSTTVGSSTTSISNYKTKDFVEIFGITALIILSAVAIFCITYYICNKRSRKYKTENKP

SEQ ID NO: 1059 - DNA, 258 bp, Artificial Sequence
  nucleotide sequence of A56 protein fragment (A56-240)
atgacacgattaccaatacttttgttactaatatcattagtatacgctaccaccgatgatacgtacaatgataatgatacagtaccaccaactactgtaggcagtagtacaacctctattagcaattataaaaccaaggactttgtagaaatatttggtattaccgcattaattatattgtcggccgtggcaatattctgtattacgtattatatatgtaataaacgttcacgtaaatacaaaacagagaacaagccg

SEQ ID NO: 1060 - protein, 56 aa, Artificial Sequence
  amino acid sequence for A56 protein fragment (A56-276)
MTRLPILLLLISLVYADFVEIFGITALIILSAVAIFCITYYICNKRSRKYKTENKP

SEQ ID NO: 1061 - DNA, 168 bp, Artificial Sequence
  nucleotide sequence of A56 protein fragment (A56-276)
atgacacgattaccaatacttttgttactaatatcattagtatacgctgactttgtagaaatatttggtattaccgcattaattatattgtcggccgtggcaatattctgtattacgtattatatatgtaataaacgttcacgtaaatacaaaacagagaacaagccg

SEQ ID NO: 1062 - protein, 8 aa, Artificial Sequence
  VH-CDR1 (LakePharma variant3)
GYSFTGYT

SEQ ID NO: 1063 - protein, 8 aa, Artificial Sequence
  H-CDR1 of LakePharma variant4
GYSFTGYT

SEQ ID NO: 1064 - protein, 8 aa, Artificial Sequence
  H-CDR2 of LakePharma variant3,4
INPYNGGT

SEQ ID NO: 1065 - protein, 14 aa, Artificial Sequence
  H-CDR3 of LakePharma variant 3,4
ARSHYRYDYWYFDV

SEQ ID NO: 1066 - protein, 11 aa, Artificial Sequence
  L-CDR1 of LakePharma variant 3,4
QSLVHSNGNTY

SEQ ID NO: 1067 - protein, 3 aa, Artificial Sequence
  L-CDR2 of LakePharma variant 3,4
KVS

SEQ ID NO: 1068 - protein, 10 aa, Artificial Sequence
  L-CDR3 of LakePharma variant 3,4
SQSTHVPPFT

SEQ ID NO: 1069 - protein, 445 aa, Artificial Sequence
  VH of LakePharma variant 3,4
QVQLQQSGPELVKPGASMKLSCKASGYSFTGYTMNWVKQSHGKNLEWIGLINPYNGGTSYNQKFKGKATLTVDKSSSTAYMELLSLTSEDSAVYYCARSHYRYDYWYFDVWGAGTTVTVSSAKTTPPSVYPLAPGSAAQTNSMVTLGCLVKGYFPEPVTVTWNSGSLSSGVHTFPAVLQSDLYTLSSSVTVPSSTWPSETVTCNVAHPASSTKVDKKIVPRDCGCKPCICTVPEVSSVFIFPPKPKDVLTITLTPKVTCVVVDISKDDPEVQFSWFVDDVEVHTAQTQPREEQFNSTFRSVSELPIMHQDWLNGKEFKCRVNSAAFPAPIEKTISKTKGRPKAPQVYTIPPPKEQMAKDKVSLTCMITDFFPEDITVEWQWNGQPAENYKNTQPIMDTDGSYFVYSKLNVQKSNWEAGNTFTCSVLHEGLHNHHTEKSLSHSPGK

SEQ ID NO: 1070 - protein, 445 aa, Artificial Sequence
  VH of LakePharma variant 4
EVQLQQSGPELVKPGASMKLSCKASGYSFTGYTMNWVKQSHGKNLEWIGLINPYNGGTSYNQKFKGKATLTVDKSSSTAYMELLSLTSEDSAVYYCARSHYRYDYWYFDVWGAGTTVTVSSAKTTPPSVYPLAPGSAAQTNSMVTLGCLVKGYFPEPVTVTWNSGSLSSGVHTFPAVLQSDLYTLSSSVTVPSSTWPSETVTCNVAHPASSTKVDKKIVPRDCGCKPCICTVPEVSSVFIFPPKPKDVLTITLTPKVTCVVVDISKDDPEVQFSWFVDDVEVHTAQTQPREEQFNSTFRSVSELPIMHQDWLNGKEFKCRVNSAAFPAPIEKTISKTKGRPKAPQVYTIPPPKEQMAKDKVSLTCMITDFFPEDITVEWQWNGQPAENYKNTQPIMDTDGSYFVYSKLNVQKSNWEAGNTFTCSVLHEGLHNHHTEKSLSHSPGK

SEQ ID NO: 1071 - protein, 220 aa, Artificial Sequence
  VL of LakePharma variant 3, 4
DVVMTQTPLSLPVSLGDQASISCRSSQSLVHSNGNTYLHWYLQKPGQSPKLLIYKVSNRFSGVPDRFSGSGSGTDFTLKISRVEAEDLGVYFCSQSTHVPPFTFGSGTKLEIKRADAAPTVSIFPPSSEQLTSGGASVVCFLNNFYPKDINVKWKIDGSERQNGVLNSWTDQDSKDSTYSMSSTLTLTKDEYERHNSYTCEATHKTSTSPIVKSFNRNEC

SEQ ID NO: 1072 - DNA, 945 bp, Artificial Sequence
  nucleotide sequence of A56 protein
atgacacgattaccaatacttttgttactaatatcattagtatacgctacaccttttcctcagacatctaaaaaaataggtgatgatgcaactctatcatgtaatcgaaataatacaaatgactacgttgttatgagtgcttggtataaggagcccaattctattattcttttagctgctaaaagcgacgtcttgtattttgataattataccaaggataaaatatcttacgactctccatacgatgatctagttacaactatcacaattaaatcattgactgctagagatgccggtacttatgtatgtgcattctttatgacatcgcctacaaatgacactgataaagtagattatgaagaatactccacagagttgattgtaaatacagatagtgaatcgactattgacataatactatctggatctacacattcaccggaaactagttctgagaaaccagaggatatagataattttaattgctcgtcggtattcgaaatcgcgactccggaaccaattactgataatgtagaagatcatacagacaccgtcacatacactagtgatagcattaatacagtaagtgcatcatctggagaatccacaacagacgagactccggaaccaattactgataaagaagaagatcatacagtcacagacactgtctcatacactacagtaagtacatcatctggaattgtcactactaaatcaaccaccgatgatgcggatctttatgatacgtacaatgataatgatacagtaccatcaactactgtaggtagtagtacaacctctattagcaattataaaaccaaggactttgtagaaatatttggtattaccgcattaattatattgtcggccgtggcaatattctgtattacgtattatatatgtaataaacgttcacgtaaatacaaaacagagaacaaagtc

SEQ ID NO: 1073 - protein, 315 aa, Artificial Sequence
  amino acid sequence for A56 protein
MTRLPILLLLISLVYATPFPQTSKKIGDDATLSCNRNNTNDYVVMSAWYKEPNSIILLAAKSDVLYFDNYTKDKISYDSPYDDLVTTITIKSLTARDAGTYVCAFFMTSPTNDTDKVDYEEYSTELIVNTDSESTIDIILSGSTHSPETSSEKPEDIDNFNCSSVFEIATPEPITDNVEDHTDTVTYTSDSINTVSASSGESTTDETPEPITDKEEDHTVTDTVSYTTVSTSSGIVTTKSTTDDADLYDTYNDNDTVPSTTVGSSTTSISNYKTKDFVEIFGITALIILSAVAIFCITYYICNKRSRKYKTENKV

SEQ ID NO: 1074 - DNA, 930 bp, Artificial Sequence
  nucleotide sequence of A56 protein(OTS-412-A56)
atgacacgattaccaatacttttgttactaatatcattagtatacgctacaccttttcctcagacatctaaaaaaataggtgatgatgcaactctatcatgtaatcgaaataatacaaatgactacgttgttatgagtgcttggtataaggagcccaattctattattcttttagctgctaaaagcgacgtcttgtattttgataattataccaaggataaaatatcttacgactctccatacgatgatctagttacaactatcacaattaaatcattgactgctagagatgccggtacttatgtatgtgcattctttatgacatcgcctacaaatgacactgataaagtagattatgaagaatactccacagagttgattgtaaatacagatagtgaatcgactattgacataatactatctggatctacacattcaccggaaactagttctgagaaaccagaggatatagataattttaattgctcgtcggtattcgaaatcgcgactccggaaccaattactgataatgtagaagatcatacagacaccgtcacatacactagtgatagcattaatacagtaagtgcatcatctggagaatccacaacagacgagactccggaaccaattactgataaagaagaagatcatacagtcacagacactgtctcatacactacagtaagtacatcatctggaattgtcactactaaatcaaccaccgatgatgcgtacaatgataatgatacagtaccatcaactactgtaggtagtagtacaacctctattagcaattataaaaccaaggactttgtagaaatatttggtattaccgcattaattatattgtcggccgtggcaatattctgtattacgtattatatatgtaataaacgttcacgtaaatacaaaacagagaacaaagtc

SEQ ID NO: 1075 - protein, 310 aa, Artificial Sequence
  amino acid sequence of A56 protein (OTS-412-A56)
MTRLPILLLLISLVYATPFPQTSKKIGDDATLSCNRNNTNDYVVMSAWYKEPNSIILLAAKSDVLYFDNYTKDKISYDSPYDDLVTTITIKSLTARDAGTYVCAFFMTSPTNDTDKVDYEEYSTELIVNTDSESTIDIILSGSTHSPETSSEKPEDIDNFNCSSVFEIATPEPITDNVEDHTDTVTYTSDSINTVSASSGESTTDETPEPITDKEEDHTVTDTVSYTTVSTSSGIVTTKSTTDDAYNDNDTVPSTTVGSSTTSISNYKTKDFVEIFGITALIILSAVAIFCITYYICNKRSRKYKTENKV

SEQ ID NO: 1076 - DNA, 774 bp, Artificial Sequence
  nucleotide sequence of A56 protein fragment
acaccttttcctcagacatctaaaaaaataggtgatgatgcaactctatcatgtaatcgaaataatacaaatgactacgttgttatgagtgcttggtataaggagcccaattctattattcttttagctgctaaaagcgacgtcttgtattttgataattataccaaggataaaatatcttacgactctccatacgatgatctagttacaactatcacaattaaatcattgactgctagagatgccggtacttatgtatgtgcattctttatgacatcgcctacaaatgacactgataaagtagattatgaagaatactccacagagttgattgtaaatacagatagtgaatcgactattgacataatactatctggatctacacattcaccggaaactagttctgagaaaccagaggatatagataattttaattgctcgtcggtattcgaaatcgcgactccggaaccaattactgataatgtagaagatcatacagacaccgtcacatacactagtgatagcattaatacagtaagtgcatcatctggagaatccacaacagacgagactccggaaccaattactgataaagaagaagatcatacagtcacagacactgtctcatacactacagtaagtacatcatctggaattgtcactactaaatcaaccaccgatgatgcgtacaatgataatgatacagtaccatcaactactgtaggtagtagtacaacctctattagcaattataaaaccaaggactttgtagaa

SEQ ID NO: 1077 - protein, 258 aa, Artificial Sequence
  amino acid sequence of A56 protein fragment
TPFPQTSKKIGDDATLSCNRNNTNDYVVMSAWYKEPNSIILLAAKSDVLYFDNYTKDKISYDSPYDDLVTTITIKSLTARDAGTYVCAFFMTSPTNDTDKVDYEEYSTELIVNTDSESTIDIILSGSTHSPETSSEKPEDIDNFNCSSVFEIATPEPITDNVEDHTDTVTYTSDSINTVSASSGESTTDETPEPITDKEEDHTVTDTVSYTTVSTSSGIVTTKSTTDDAYNDNDTVPSTTVGSSTTSISNYKTKDFVE

SEQ ID NO: 1078 - DNA, 942 bp, Artificial Sequence
  nucleotide sequence of A56 protein (WOTS-418-A56)
atgacacgattaccaatacttttgttactaatatcattagtatacgctacaccttttcctcagacatctaaaaaaataggtgatgatgcaactctatcatgtaatcgaaataatacaaatgactacgttgttatgagtgcttggtataaggagcccaattccattattcttttagctgctaaaagcgacgtcttgtattttgataattataccaaggataaaatatcttacgactctccatacgatgatctagttacaactatcacaattaaatcattgactgctagagatgccggtacttatgtatgtgcattctttatgacatcaactacaaatgacactgataaagtagattatgaagaatactccacagagttgattgtaaatacagatagtgaatcgactatagacataatactatctggatctacacattcaccggaaactagttctaagaaacctgattatatagataattctaattgctcgtcggtattcgaaatcgcgactccggaaccaattactgataatgtagaagatcatacagacaccgtcacatacactagtgatagcattaatacagtaagtgcatcatctggagaatccacaacagacgagactccggaaccaattactgataaagaagatcatacagttacagacactgtctcatacactacagtaagtacatcatctggaattgtcactactaaatcaaccaccgatgatgcggatctttatgatacgtacaatgataatgatacagtaccaccaactactgtaggcggtagtacaacctctattagcaattataaaaccaaggactttgtagaaatatttggtattaccgcattaattatattgtcggccgtggcaattttctgtattacatattatatatataataaacgttcacgtaaatacaaaacagagaacaaagtc

SEQ ID NO: 1079 - protein, 314 aa, Artificial Sequence
  amino acid sequence of A56 protein (WOTS-418-A56)
MTRLPILLLLISLVYATPFPQTSKKIGDDATLSCNRNNTNDYVVMSAWYKEPNSIILLAAKSDVLYFDNYTKDKISYDSPYDDLVTTITIKSLTARDAGTYVCAFFMTSTTNDTDKVDYEEYSTELIVNTDSESTIDIILSGSTHSPETSSKKPDYIDNSNCSSVFEIATPEPITDNVEDHTDTVTYTSDSINTVSASSGESTTDETPEPITDKEDHTVTDTVSYTTVSTSSGIVTTKSTTDDADLYDTYNDNDTVPPTTVGGSTTSISNYKTKDFVEIFGITALIILSAVAIFCITYYIYNKRSRKYKTENKV

SEQ ID NO: 1080 - protein, 21 aa, Artificial Sequence
  amino acid sequence for CD8 signal sequence
MALPVTALLLPLALLLHAARP

SEQ ID NO: 1081 - protein, 249 aa, Artificial Sequence
  amino acid sequence for anti-UTTA scFv (Ab13)
QMQLVESGAEVKKTGSSVKVSCKASGDTLTYRFLHWVRQAPGQAPEWMGWITPFNDNTNYAQKFQDRVTITRDRSMSTAYMELSSLRSEDTAVYYCATGGGNNYYGMEVWGQGTPITVSSGLGGLGGGGSGGGGSGGSSGVGSSYELTQPLSLSVSPGQTASITCSGDKLGDKFTSWYQQQPGQSPVLVIYQDAKRPSGIPERFSGSNSGSTATLTISGTQSMDEADYYCQAWDSSSVVFGGGTKLTVL

SEQ ID NO: 1082 - protein, 261 aa, Artificial Sequence
  amino acid sequence for anti-UTTA scFv (Ab16)
QVQLQQSGPGLVKPSQTLSLTCAISGDSVSSNSAAWNWIRQSPSRGLEWLGRTYYRSKWYNDYAVSVKSRITINPDTSKNQFSLQLNSVTAVDTAVYYCAKSYAGPISYYYYGLDVWGQGTTVTVSSGLGGLGGGGSGGGGSGGSSGVGSQSALTQPASVSGSPGQSVTISCTGTSSDIGRYNLVSWYQQHPGKAPKLMIYGGSKRPSGVSNRFSGSNSDNTASLTISGLRAEDEADYYCSSYASSSTPYVFGTGTKVTVL

SEQ ID NO: 1083 - protein, 249 aa, Artificial Sequence
  amino acid sequence for anti-UTTA scFv (Ab18)
QVQLVESGGGLVQPGKSLRLSCAASGFTFSTYGMTWVRQAPGKGLEWVSGISGGGSSTNYADSVKGRFIISRDNSNNTLYLQMNSLRAEDTAVYYCARWGVMLSFDYWGQGTPVTVSSGLGGLGGGGSGGGGSGGSSGVGSDIQMTQSPSTLPASVGDRVTITCRASYSVSPWLAWYQQKPGKAPKLLIYKASTLESGVPSRFSGSGSGTEFTLTISSLQPDDFATYYCQQFNSYMMYTFGQGTKLEIK

SEQ ID NO: 1084 - protein, 255 aa, Artificial Sequence
  amino acid sequence for anti-UTTA scFv (Ab01)
QMQLVQSGAEVKKPGSSVKVSCKASGGTFSSYAISWVRQAPGQGLEWMGGIIPIFGTANYAQKFQGRVTMTRDTSTSTVYMELSSLKSEDTAVYYCARFVFGSGTYLDSWGQGTLVTVSSGLGGLGGGGSGGGGSGGSSGVGSDIVMTQTPLSLPVTPGESASISCRSSQSLLYSNGNNYLDWYLQKPGQSPQLLIYLGSNRASGVPDRFSGSGSGTDFTLKISRVEAEDVGVYYCMQALQTPLTFGGGTKVDIK

SEQ ID NO: 1085 - protein, 255 aa, Artificial Sequence
  amino acid sequence for anti-UTTA scFv (Ab19)
QVQLVESGAEVRRPGSSVKVSCKTSGVTFSGYVLSWVRQAPGHGLEWMGRIIPLIDVENYAREFQGRMKITADKSTNTVYMELNNLRSEDTAVYYCAKSVVRGLDYYYYGFDVWGQGTTVTVSSGLGGLGGGGSGGGGSGGSSGVGSSYELTQPPSLSVAPGKTARITCGGNNIGSKSVHWYQQKPGQAPRLVTYYDGNRPSGIPERFSGSNSGNTATLIISRVEAGDEADYYCQVWDSSSDQGVFGTGTKVTVL

SEQ ID NO: 1086 - protein, 108 aa, Artificial Sequence
  amino acid sequence for CD8 TM
TTTPAPRPPTPAPTIASQPLSLRPEACRPAAGGAVHTRGTTTPAPRPPTPAPTIASQPLSLRPEACRPAAGGAVHTRGLDFACDIYIWAPLAGTCGVLLLSLVITLYC

SEQ ID NO: 1087 - protein, 42 aa, Artificial Sequence
  amino acid sequence for 4-1BB Signaling Domain
KRGRKKLLYIFKQPFMRPVQTTQEEDGCSCRFPEEEEGGCEL

SEQ ID NO: 1088 - protein, 112 aa, Artificial Sequence
  amino acid sequence for CD3Z Signaling Domain
RVKFSRSADAPAYKQGQNQLYNELNLGRREEYDVLDKRRGRDPEMGGKPRRKNPQEGLYNELQKDKMAEAYSEIGMKGERRRGKGHDGLYQGLSTATKDTYDALHMQALPPR

SEQ ID NO: 1089 - DNA, 63 bp, Artificial Sequence
  nucleotide sequence of CD8 signal sequence
atggctctgcctgtgacagctctgctgctgcctctggctctgcttctgcatgctgctagacct

SEQ ID NO: 1090 - DNA, 747 bp, Artificial Sequence; identical to SEQ ID NO: 228
  nucleotide sequence of anti-UTTA scFv (Ab13)

SEQ ID NO: 1091 - DNA, 783 bp, Artificial Sequence
  nucleotide sequence of anti-UTTA scFv (Ab16)
caggtgcagctgcagcagtcaggtccaggactggtgaagccctcgcagaccctctcactcacctgtgccatctccggggacagtgtctctagcaacagtgctgcttggaactggatcaggcagtccccatcgagaggccttgagtggctgggaaggacatactacaggtccaagtggtataatgattatgcagtatctgtgaaaagtcgaataaccatcaacccagacacatccaagaaccagttctccctgcagctgaactctgtgaccgccgtggacacggccgtgtattactgtgcgaaatcctatgcggggcctatctcttattactactacggtctggacgtctggggccaagggaccacggtcaccgtctcctcaggcctcgggggcctcggaggaggaggtagtggcggaggaggctccggtggatccagcggtgtgggttcccagtctgccctgactcagcctgcctccgtgtctgggtctcctggacagtcggtcaccatctcctgcactggaaccagcagtgacattggtcgttataaccttgtctcctggtaccaacagcacccaggcaaagcccccaaactcatgatttatgggggcagtaagcggccctcaggggtttctaatcgcttctctggctccaactctgacaacacggcctccctgacaatctctgggctccgggctgaggacgaggctgattattactgcagttcatatgcaagcagcagcaccccttatgtcttcggaactgggaccaaggtcaccgtccta

SEQ ID NO: 1092 - DNA, 747 bp, Artificial Sequence; identical to SEQ ID NO: 330
  nucleotide sequence of anti-UTTA scFv (Ab18)

SEQ ID NO: 1093 - DNA, 765 bp, Artificial Sequence; identical to SEQ ID NO: 7
  nucleotide sequence of anti-UTTA scFv (Ab01)

SEQ ID NO: 1094 - DNA, 765 bp, Artificial Sequence; identical to SEQ ID NO: 347
  nucleotide sequence of anti-UTTA scFv (Ab19)

SEQ ID NO: 1095 - DNA, 207 bp, Artificial Sequence
  nucleotide sequence of CD8 TM
accacaacacccgctcctagacctccaacaccagctccaacaatcgccagccagcctctgtctctgaggcctgaagcttgtagacctgctgcaggcggagccgtgcataccagaggactggatttcgcctgcgacatctacatctgggcccctctggctggaacatgtggcgttctgctgctcagcctggtcatcaccctgtactgc

SEQ ID NO: 1096 - DNA, 126 bp, Artificial Sequence
  nucleotide sequence of 4-1BB Signaling Domain
aagcggggcagaaagaagctgctgtacatcttcaagcagcccttcatgcggcccgtgcagacaacccaagaggaagatggctgctcctgcagattccccgaggaagaagaaggcggctgcgagctg

SEQ ID NO: 1097 - DNA, 336 bp, Artificial Sequence
  nucleotide sequence of CD3Z Signaling Domain
agagtgaagttcagcagatccgccgacgctcccgcctataagcagggacagaaccagctgtacaacgagctgaacctggggagaagagaagagtacgacgtgctggacaagcggagaggcagagatcctgagatgggcggcaagcccagacggaagaatcctcaagagggcctgtataatgagctgcagaaagacaagatggccgaggcctactccgagatcggaatgaagggcgagcgcagaagaggcaagggacacgatggactgtaccagggcctgagcaccgccaccaaggatacctatgatgccctgcacatgcaggccctgcctccaaga